European Patent Specification EP 3 484 488 B1, published August 9, 2023. Title: ANTIGEN BINDING MOLECULES AND METHODS OF USE THEREOF. Applicant: KITE PHARMA, INC. The sequence listing filed with the application follows.

SEQUENCE LISTING (500 sequences)

SEQ ID NO: 1 - protein, 18 aa, Artificial Sequence
  Description of Artificial Sequence: Synthetic peptide
  Linker fragment sequence
GSTSGSGKPGSGEGSTKG

SEQ ID NO: 2 - protein, 10 aa, Artificial Sequence
  Description of Artificial Sequence: Synthetic peptide
  Linker fragment sequence; Clone 8 epitope
GSGKPGSGEG

SEQ ID NO: 3 - protein, 8 aa, Artificial Sequence
  Description of Artificial Sequence: Synthetic peptide
  Linker fragment sequence; Clone 16 epitope
GKPGSGEG

SEQ ID NO: 4 - DNA, 408 bp, Artificial Sequence
  Description of Artificial Sequence: Synthetic polynucleotide
  Clone 8 VH DNA
atggagactgggctgcgctggcttctcctggtcgctgtgctcaaaggtgtccagtgtcagtcggtggaggagtccgggggtcgcctggtcacgcctgggacacccctgacactcacctgcacagcctctggattcaccatcagtaaccttgcaataatctgggtccgccaggctccagggaaggggctggaatatatcggagacattgatggtcgtggtgacatatactgtgcgacctgggcgaaaggccgattcaccatctccaaaacctcgaccacactggatctgagattcaccagcccgacaaccgaggacacggccacctacttctgtgccgtagatggtgatggtagtggttggggtgactttaacttttggggcccaggcaccctggtcaccgtctcctca

SEQ ID NO: 5 - protein, 136 aa, Artificial Sequence
  Description of Artificial Sequence: Synthetic polypeptide
  Clone 8 VH AA
METGLRWLLLVAVLKGVQCQSVEESGGRLVTPGTPLTLTCTASGFTISNLAIIWVRQAPGKGLEYIGDIDGRGDIYCATWAKGRFTISKTSTTLDLRFTSPTTEDTATYFCAVDGDGSGWGDFNFWGPGTLVTVSS

SEQ ID NO: 6 - protein, 459 aa, Artificial Sequence
  Description of Artificial Sequence: Synthetic polypeptide
  Clone 8 HC AA
METGLRWLLLVAVLKGVQCQSVEESGGRLVTPGTPLTLTCTASGFTISNLAIIWVRQAPGKGLEYIGDIDGRGDIYCATWAKGRFTISKTSTTLDLRFTSPTTEDTATYFCAVDGDGSGWGDFNFWGPGTLVTVSSGQPKAPSVFPLAPCCGDTPSSTVTLGCLVKGYLPEPVTVTWNSGTLTNGVRTFPSVRQSSGLYSLSSVVSVTSSSQPVTCNVAHPATNTKVDKTVAPSTCSKPTCPPPELLGGPSVFIFPPKPKDTLMISRTPEVTCVVVDVSQDDPEVQFTWYINNEQVRTARPPLREQQFNSTIRVVSTLPIAHQDWLRGKEFKCKVHNKALPAPIEKTISKARGQPLEPKVYTMGPPREELSSRSVSLTCMINGFYPSDISVEWEKNGKAEDNYKTTPAVLDSDGSYFLYSKLSVPTSEWQRGDVFTCSVMHEALHNHYTQKSISRSPGK

SEQ ID NO: 7 - protein, 7 aa, Artificial Sequence
  Description of Artificial Sequence: Synthetic peptide
  Clone 8 VH CDR1 AA
GFTISNL

SEQ ID NO: 8 - protein, 15 aa, Artificial Sequence
  Description of Artificial Sequence: Synthetic peptide
  Clone 8 VH CDR2 AA
DIDGRGDIYCATWAK

SEQ ID NO: 9 - protein, 12 aa, Artificial Sequence
  Description of Artificial Sequence: Synthetic peptide
  Clone 8 VH CDR3 AA
DGDGSGWGDFNF

SEQ ID NO: 10 - DNA, 396 bp, Artificial Sequence
  Description of Artificial Sequence: Synthetic polynucleotide
  Clone 8 VL DNA
atggacacgagggcccccactcagctgctggggctcctgctgctctggctcccaggtgccagatgtgcctatgatatgacccagactccagcctctgtggaggtagctgtgggaggcacagtcagcatcaagtgccaggccagtcagagcattagcactgcattagcctggtatcagcagaaaccaggacagcctcccaagctcctgatctacagggcatccactctggcatctggggtctcatcgcggttcaaaggcagtggatctgggacacagttcactctcaccatcagcggcgtggagtgtgacgatgctgccacttactactgtcaacagggttggagtactgtgaatgttgataatgttttcggcggagggaccgaggtggtggtcaga

SEQ ID NO: 11 - protein, 132 aa, Artificial Sequence
  Description of Artificial Sequence: Synthetic polypeptide
  Clone 8 VL AA
MDTRAPTQLLGLLLLWLPGARCAYDMTQTPASVEVAVGGTVSIKCQASQSISTALAWYQQKPGQPPKLLIYRASTLASGVSSRFKGSGSGTQFTLTISGVECDDAATYYCQQGWSTVNVDNVFGGGTEVVVR

SEQ ID NO: 12 - protein, 235 aa, Artificial Sequence
  Description of Artificial Sequence: Synthetic polypeptide
  Clone 8 LC AA
MDTRAPTQLLGLLLLWLPGARCAYDMTQTPASVEVAVGGTVSIKCQASQSISTALAWYQQKPGQPPKLLIYRASTLASGVSSRFKGSGSGTQFTLTISGVECDDAATYYCQQGWSTVNVDNVFGGGTEVVVRDPVAPTVLIFPPAADQVATGTVTIVCVANKYFPDVTVTWEVDGTTQTTGIENSKTPQNSADCTYNLSSTLTLTSTQYNSHKEYTCKVTQGTTSVVQSFNRGDC

SEQ ID NO: 13 - protein, 11 aa, Artificial Sequence
  Description of Artificial Sequence: Synthetic peptide
  Clone 8 VL CDR1 AA
QASQSISTALA

SEQ ID NO: 14 - protein, 7 aa, Artificial Sequence
  Description of Artificial Sequence: Synthetic peptide
  Clone 8 VL CDR2 AA
RASTLAS

SEQ ID NO: 15 - protein, 12 aa, Artificial Sequence
  Description of Artificial Sequence: Synthetic peptide
  Clone 8 VL CDR3 AA
QQGWSTVNVDNV

SEQ ID NO: 16 - DNA, 402 bp, Artificial Sequence
  Description of Artificial Sequence: Synthetic polynucleotide
  Clone 16 VH DNA
atggagactgggctgcgctggcttctcctggtcgctgtgctcaaaggtgtccagtgtcagtcgctggaggagtccgggggtcgcctggtcacgcctgggacacccctgacactcacctgcacagtctctggatccgacatcagtagctaccacatgggctgggtccgccaggctccagggaaggggctggaatacatcggaatcattgttagtagtggtagcgcatactacgcgacctgggcaaaaggccgattcaccatctccaggacctcgaccacggtggatctgaaaatcaccagtccgacaaccgaggactcggccacctatttctgtgccagaaatcaatatagtggttatggctttagcttctggggcccaggcaccctggtcaccgtctcctca

SEQ ID NO: 17 - protein, 134 aa, Artificial Sequence
  Description of Artificial Sequence: Synthetic polypeptide
  Clone 16 VH AA
METGLRWLLLVAVLKGVQCQSLEESGGRLVTPGTPLTLTCTVSGSDISSYHMGWVRQAPGKGLEYIGIIVSSGSAYYATWAKGRFTISRTSTTVDLKITSPTTEDSATYFCARNQYSGYGFSFWGPGTLVTVSS

SEQ ID NO: 18 - protein, 457 aa, Artificial Sequence
  Description of Artificial Sequence: Synthetic polypeptide
  Clone 16 HC AA
METGLRWLLLVAVLKGVQCQSLEESGGRLVTPGTPLTLTCTVSGSDISSYHMGWVRQAPGKGLEYIGIIVSSGSAYYATWAKGRFTISRTSTTVDLKITSPTTEDSATYFCARNQYSGYGFSFWGPGTLVTVSSGQPKAPSVFPLAPCCGDTPSSTVTLGCLVKGYLPEPVTVTWNSGTLTNGVRTFPSVRQSSGLYSLSSVVSVTSSSQPVTCNVAHPATNTKVDKTVAPSTCSKPTCPPPELLGGPSVFIFPPKPKDTLMISRTPEVTCVVVDVSQDDPEVQFTWYINNEQVRTARPPLREQQFNSTIRVVSTLPIAHQDWLRGKEFKCKVHNKALPAPIEKTISKARGQPLEPKVYTMGPPREELSSRSVSLTCMINGFYPSDISVEWEKNGKAEDNYKTTPAVLDSDGSYFLYSKLSVPTSEWQRGDVFTCSVMHEALHNHYTQKSISRSPGK

SEQ ID NO: 19 - protein, 7 aa, Artificial Sequence
  Description of Artificial Sequence: Synthetic peptide
  Clone 16 VH CDR1 AA
GSDISSY

SEQ ID NO: 20 - protein, 15 aa, Artificial Sequence
  Description of Artificial Sequence: Synthetic peptide
  Clone 16 VH CDR2 AA
IIVSSGSAYYATWAK

SEQ ID NO: 21 - protein, 10 aa, Artificial Sequence
  Description of Artificial Sequence: Synthetic peptide
  Clone 16 VH CDR3 AA
NQYSGYGFSF

SEQ ID NO: 22 - DNA, 399 bp, Artificial Sequence
  Description of Artificial Sequence: Synthetic polynucleotide
  Clone 16 VL DNA
atggacacgagggcccccactcagctgctggggctcctgctgctctggctcccaggtgccacatttgccgtcgtgctgacccagactccatccccagtgtctacagctgtaggaggcacagtcaccatcaattgccagtccagtcacagtgtttattatggcgactggttagcctggtatcagcagaaaccagggcagcctcctaagctcctgatctacagggcatccaatctggcatctggtgtcccatcgcggttcaaaggcagtggatctgggacacagttcactctcaccatcagcggcgtgcagtgtgacgatgctgccacttactactgtctaggcggttatgatgatgatggtgagactgctttcggcggagggaccgaggtggtggtcaaa

SEQ ID NO: 23 - protein, 133 aa, Artificial Sequence
  Description of Artificial Sequence: Synthetic polypeptide
  Clone 16 VL AA
MDTRAPTQLLGLLLLWLPGATFAVVLTQTPSPVSTAVGGTVTINCQSSHSVYYGDWLAWYQQKPGQPPKLLIYRASNLASGVPSRFKGSGSGTQFTLTISGVQCDDAATYYCLGGYDDDGETAFGGGTEVVVK

SEQ ID NO: 24 - protein, 236 aa, Artificial Sequence
  Description of Artificial Sequence: Synthetic polypeptide
  Clone 16 LC AA
MDTRAPTQLLGLLLLWLPGATFAVVLTQTPSPVSTAVGGTVTINCQSSHSVYYGDWLAWYQQKPGQPPKLLIYRASNLASGVPSRFKGSGSGTQFTLTISGVQCDDAATYYCLGGYDDDGETAFGGGTEVVVKDPVAPTVLIFPPAADQVATGTVTIVCVANKYFPDVTVTWEVDGTTQTTGIENSKTPQNSADCTYNLSSTLTLTSTQYNSHKEYTCKVTQGTTSVVQSFNRGDC

SEQ ID NO: 25 - protein, 13 aa, Artificial Sequence
  Description of Artificial Sequence: Synthetic peptide
  Clone 16 VL CDR1 AA
QSSHSVYYGDWLA

SEQ ID NO: 26 - protein, 7 aa, Artificial Sequence
  Description of Artificial Sequence: Synthetic peptide
  Clone 16 VL CDR2 AA
RASNLAS

SEQ ID NO: 27 - protein, 11 aa, Artificial Sequence
  Description of Artificial Sequence: Synthetic peptide
  Clone 16 VL CDR3 AA
LGGYDDDGETA

SEQ ID NO: 28 - protein, 117 aa, Artificial Sequence
  Description of Artificial Sequence: Synthetic polypeptide
  8 4 HC humanized 866
VQLQESGGGVVQPGRSLRLSCAASGFTISNLAIIWVRQAPGKGLEWVADIDGRGDIYCATWAKGRFTISRDNSTLYLQMNSLRADDTAVYYCARDGDGSGWGDFNFWGQGTLVTVSS

SEQ ID NO: 29 - protein, 117 aa, Artificial Sequence
  Description of Artificial Sequence: Synthetic polypeptide
  8 4 HC humanized 673
QSVVESGGVVVQPGGSLRLSCAASGFTISNLAIIWVRQAPGKGPEWVSDIDGRGDIYCATWAKGRFTISRDNSSLYLQMNSLRTEDTAVYYCAKDGDGSGWGDFNFWGQGTMVTVSS

SEQ ID NO: 30 - protein, 117 aa, Artificial Sequence
  Description of Artificial Sequence: Synthetic polypeptide
  8 4 HC humanized 631
QSVEESGGRLVTPGATVKISCKVSGFTISNLAIIWVQQAPGKGLEWMGDIDGRGDIYCATWAQGRVTITADSSTAYMELNGLRYADTAVYYCATDGDGSGWGDFNFWGQGTLVTVSS

SEQ ID NO: 31 - protein, 117 aa, Artificial Sequence
  Description of Artificial Sequence: Synthetic polypeptide
  8 4 HC humanized 1002
QSLEESGGGVVQPGKSLRLSCTASGFTISNLAIIWVRQAPGKGLESVADIDGRGDIYCATWATGRFAISRDNSKLYLHMDNLRAEDTAVYYCARDGDGSGWGDFNFWGQGTTVIVSS

SEQ ID NO: 32 - protein, 117 aa, Artificial Sequence
  Description of Artificial Sequence: Synthetic polypeptide
  8 4 HC humanized 771
QSLEQSGGGLVQPGGSLRLSCAASGFTISNLAIIWVRQAPGKGLEWVSDIDGRGDIYCATWAKGRFTISKSKNTLYLQMNSLRAEDTAVYYCAVDGDGSGWGDFNFWGQGTLVTVSS

SEQ ID NO: 33 - protein, 117 aa, Artificial Sequence
  Description of Artificial Sequence: Synthetic polypeptide
  8 4 HC humanized 849
QSVEESGGDLVKPGGSLRLSCAASGFTISNLAIIWIRQAPGKGLEWLSDIDGRGDIYCATWAKGRFTISRDNASLNLQMNSLRAEDTAVYYCAVDGDGSGWGDFNFWGQGTLVTVSS

SEQ ID NO: 34 - protein, 117 aa, Artificial Sequence
  Description of Artificial Sequence: Synthetic polypeptide
  8 4 HC humanized 706
VLLLESGGGLAQPGGTLRLSCSASGFTISNLAIIWVRQAPGKGLEWVSDIDGRGDIYCATWARGRFIISRDNSTLYLQMNSLRAEDTAVYYCAKDGDGSGWGDFNFWGQGILVTVSS

SEQ ID NO: 35 - protein, 117 aa, Artificial Sequence
  Description of Artificial Sequence: Synthetic polypeptide
  8 4 HC humanized 703
VQLVESGGTLVQPGGSLRLSCSASGFTISNLAIIWVRQAPGKGLEYVSDIDGRGDIYCATWAKGRITISRDNSTLSLQMSTLRTEDTAVYYCVRDGDGSGWGDFNFWGQGTLVTVSS

SEQ ID NO: 36 - protein, 117 aa, Artificial Sequence
  Description of Artificial Sequence: Synthetic polypeptide
  8 4 HC humanized 278
VQLVQSGGGLVKPGGSLRLSCEASGFTISNLAIIWIRQAPGKGLEWVGDIDGRGDIYCATWAKGRFTISRDDSTLYLQVNSLKTEDSAVYYCTTDGDGSGWGDFNFWGQGTLVTVSS

SEQ ID NO: 37 - protein, 117 aa, Artificial Sequence
  Description of Artificial Sequence: Synthetic polypeptide
  8 4 HC humanized 800
QSVLESGPGLVKPSETLSLTCTVSGFTISNLAIIWIRQPPGKGLEWIGDIDGRGDIYCATWAKSRLTISTSKNQFSLRLTSVTAADTAMYYCAVDGDGSGWGDFNFWGQGTLVSVSS

SEQ ID NO: 38 - protein, 117 aa, Artificial Sequence
  Description of Artificial Sequence: Synthetic polypeptide
  8 4 HC humanized 809
VQLVESGGGLVQPGGSLRLSCAASGFTISNLAIIWVRQAPGKGLEWLSDIDGRGDIYCATWARGRFAISNARNSLYLQMNSLRDEDTAVYFCARDGDGSGWGDFNFWGQGTLVTVSS

SEQ ID NO: 39 - protein, 117 aa, Artificial Sequence
  Description of Artificial Sequence: Synthetic polypeptide
  8 4 HC humanized 273
VQLVQSGGGLVQPGGSLRLSCAASGFTISNLAIIWVRQASGKGLEWIGDIDGRGDIYCATWAKGRFTVSRSQNSVFLQMNSLETEDTAVYYCARDGDGSGWGDFNFWGQGTLVTVSS

SEQ ID NO: 40 - protein, 117 aa, Artificial Sequence
  Description of Artificial Sequence: Synthetic polypeptide
  8 4 HC humanized 716
QSVLESGGGWVQPGRSLRLSCSASGFTISNLAIIWVRQAPGKGLEWVSDIDGRGDIYCATWAKGRFTISRDNNSLYLQMNSLRPEDTALYYCAKDGDGSGWGDFNFWGQGVLVTVSS

SEQ ID NO: 41 - protein, 117 aa, Artificial Sequence
  Description of Artificial Sequence: Synthetic polypeptide
  8 4 HC humanized 202
VQLQESGEGLVQPGGSLRLSCAASGFTISNLAIIWVRQAPGKGLEYVSDIDGRGDIYCATWAKGRFTISRDNSTLYLQMGSLRAEDMAVYYCAVDGDGSGWGDFNFWGQGTMVTVSS

SEQ ID NO: 42 - protein, 117 aa, Artificial Sequence
  Description of Artificial Sequence: Synthetic polypeptide
  8 4 HC humanized 21
VQLVESGGGLVQPGGSLRLSCAASGFTISNLAIIWVRQAPGKGLEFVSDIDGRGDIYCATWAKDRFTISRDNSTVYLQMDSLRTEDTAMYFCARDGDGSGWGDFNFWGQGTLVTVSS

SEQ ID NO: 43 - protein, 117 aa, Artificial Sequence
  Description of Artificial Sequence: Synthetic polypeptide
  8 4 HC humanized 173
QSVEESGGRLVTPGGSLRLSCTATGFTISNLAIIWFRQAPGKGLEWVGDIDGRGDIYCATWAKGRFTISRDDNSLYLQMNSLKTEDTAVYYCARDGDGSGWGDFNFWGQGTLVTVSS

SEQ ID NO: 44 - protein, 117 aa, Artificial Sequence
  Description of Artificial Sequence: Synthetic polypeptide
  8 4 HC humanized 23
QSVLESGGDLVQPGGSLRLSCEASGFTISNLAIIWVRQAPGKGLEWVSDIDGRGDIYCATWAKGRFTISKSKHTLFLQMHSLRVEDTAVYYCAKDGDGSGWGDFNFWGQGTTVTVSS

SEQ ID NO: 45 - protein, 117 aa, Artificial Sequence
  Description of Artificial Sequence: Synthetic polypeptide
  8 4 HC humanized 879
QSVEESGGGLVQPGGSLRLSCTASGFTISNLAIIWVRQAPGKGLEWVSDIDGRGDIYCATWAKGRFTISRDSSTLYLQMNNLRVEDTALYYCAHDGDGSGWGDFNFWGRGTQVTVSS

SEQ ID NO: 46 - protein, 110 aa, Artificial Sequence
  Description of Artificial Sequence: Synthetic polypeptide
  8 4 LC humanized 866
DIQMTQSPSSLSASVGDRVTITCQASQSISTALAWYQQKPGKAPKRLIYRASTLASGVPSRFSGSGSGTEFTLTISSLQPEDFATYYCQQGWSTVNVDNVFGQGTKVEIK

SEQ ID NO: 47 - protein, 110 aa, Artificial Sequence
  Description of Artificial Sequence: Synthetic polypeptide
  8 4 LC humanized 340
DIQMTQSPFSLSASVGDRVTITCQASQSISTALAWYQQKPGKAPKLLIYRASTLASGVPSRFSGSGSGTDFTLTISSLQPEDFATYFCQQGWSTVNVDNVFGGGTKLEIK

SEQ ID NO: 48 - protein, 110 aa, Artificial Sequence
  Description of Artificial Sequence: Synthetic polypeptide
  8 4 LC humanized 322
DIQLTQSPSFLSASVGDTVSITCQASQSISTALAWYQQKPGKAPKHLIYRASTLASGVPSRFSGGGSGTDFTLTISSLQPEDFATYYCQQGWSTVNVDNVFGGGTKVEIK

SEQ ID NO: 49 - protein, 110 aa, Artificial Sequence
  Description of Artificial Sequence: Synthetic polypeptide
  8 4 LC humanized 305
DIQLTQSPSSLSASVGDRVTITCQASQSISTALAWFQQKPGKAPKSLIYRASTLASGVPSRFSGSGSGTDFTLTISSLQPEDSATYYCQQGWSTVNVDNVFGGGTKVEIK

SEQ ID NO: 50 - protein, 110 aa, Artificial Sequence
  Description of Artificial Sequence: Synthetic polypeptide
  8 4 LC humanized 303
DIQMTQSPSSLSASVGDRVTITCQASQSISTALAWYQQKPGKAPKLLIYRASTLASGVPSRFSGSGSGTDFTFTISSLQPEDIATYYCQQGWSTVNVDNVFGPGTKVDIK

SEQ ID NO: 51 - protein, 110 aa, Artificial Sequence
  Description of Artificial Sequence: Synthetic polypeptide
  8 4 LC humanized 291
DIQLTQSPSSLSASVGDRVTITCQASQSISTALAWYQQKPGKGPKLLIYRASTLASGVPSRFSGSGSGTDFSLTISSLQPEDLATYYCQQGWSTVNVDNVFGGGTKVEIK

SEQ ID NO: 52 - protein, 110 aa, Artificial Sequence
  Description of Artificial Sequence: Synthetic polypeptide
  8 4 LC humanized 217
DIVMTQSPDSLAVSLGERATINCQASQSISTALAWYQQKPGQPPKLLIYRASTLASGVPDRFSGSGSGTDFTLTISSLQAEDVAVYYCQQGWSTVNVDNVFGQGTKVEIK

SEQ ID NO: 53 - protein, 110 aa, Artificial Sequence
  Description of Artificial Sequence: Synthetic polypeptide
  8 4 LC humanized 197
AYDMTQTPATLSLSPGERATLSCQASQSISTALAWYQQKPGQAPRLLIYRASTLASGIPARFSGSGSGTDFTLTISSLEPEDFAVYYCQQGWSTVNVDNVFGQGTEVVVR

SEQ ID NO: 54 - protein, 110 aa, Artificial Sequence
  Description of Artificial Sequence: Synthetic polypeptide
  8 4 LC humanized 169
EIVLTQSPSFLSAFVGDRITITCQASQSISTALAWYQQKPGKAPKLLIYRASTLASGVPSRFSGSGSGTEFTLTISGLQPEDFASYYCQQGWSTVNVDNVFGGGTKLEIK

SEQ ID NO: 55 - protein, 110 aa, Artificial Sequence
  Description of Artificial Sequence: Synthetic polypeptide
  8 4 LC humanized 17
DIQLTQSPSSLSAAVGDRVTIACQASQSISTALAWYQQKPGKAPKLLIYRASTLASGVPSRFSGSGSGTDFTLSISSLQPGDFATYYCQQGWSTVNVDNVFGGGTKVQMK

SEQ ID NO: 56 - protein, 110 aa, Artificial Sequence
  Description of Artificial Sequence: Synthetic polypeptide
  8 4 LC humanized 13
DIQMTQSPSSLSASVGDSVTITCQASQSISTALAWYQQKPGKAPKLLIYRASTLASGVPSRFSGSGSGTEFTLTINGLQPEDFATYYCQQGWSTVNVDNVFGGGTKLEIK

SEQ ID NO: 57 - protein, 110 aa, Artificial Sequence
  Description of Artificial Sequence: Synthetic polypeptide
  8 4 LC humanized 791
AYELTQTPLSSPVTLGQPASISCQASQSISTALAWLHQRPGQPPRLLIYRASTLASGVPDRFSGSGAGTAFTLKISRVEVEDVGIYYCQQGWSTVNVDNVFGQGTKVEIK

SEQ ID NO: 58 - protein, 110 aa, Artificial Sequence
  Description of Artificial Sequence: Synthetic polypeptide
  8 4 LC humanized 673
AYDMTQTPASVEVSPGERATLSCQASQSISTALAWYQHKPGQAPRLLIYRASTLASGIPARFSGSGSGTEFTLTISSVQSDDFAVYYCQQGWSTVNVDNVFGPGTKVDIK

SEQ ID NO: 59 - protein, 110 aa, Artificial Sequence
  Description of Artificial Sequence: Synthetic polypeptide
  8 4 LC humanized 678
AYELTQSPSSLSASVGDRVTITCQASQSISTALAWFQQKPGKAPKLLIYRASTLASGVPSRFSGSGSGTDFTLTISSLLPTDFATYFCQQGWSTVNVDNVFGQGTQVEVK

SEQ ID NO: 60 - protein, 110 aa, Artificial Sequence
  Description of Artificial Sequence: Synthetic polypeptide
  8 4 LC humanized 631
AYDMTQTPASVEVSVGDRVTITCQASQSISTALAWYQQKPGKAPKLLIYRASTLASGVPSRFGGSGSGTDFTLTISSLQPEDFATYYCQQGWSTVNVDNVFGGGTKVEIK

SEQ ID NO: 61 - protein, 110 aa, Artificial Sequence
  Description of Artificial Sequence: Synthetic polypeptide
  8 4 LC humanized 1002
AYELTQSPSSLSASVGDRVTITCQASQSISTALAWYQQKPGKAPKLLIYRASTLASGVSSRFSGSGSGTDFTLTISSLQPEDFATYYCQQGWSTVNVDNVFGQGTKLEIK

SEQ ID NO: 62 - protein, 110 aa, Artificial Sequence
  Description of Artificial Sequence: Synthetic polypeptide
  8 4 LC humanized 775
AYELTQTPLSSPVTLGQPASISCQASQSISTALAWLQQRPGQPPRLLIYRASTLASGVPDRFSGSGARTDFTLNISRVEAEDAGVYYCQQGWSTVNVDNVFGQGTKLEIK

SEQ ID NO: 63 - protein, 110 aa, Artificial Sequence
  Description of Artificial Sequence: Synthetic polypeptide
  8 4 LC humanized 771
AYELTQSPATLSLSPGERATLSCQASQSISTALAWYQQKPGQAPRLLIHRASTLASGIPARFSGSGSGTDFTLTISSLEPEDFAVYYCQQGWSTVNVDNVFGGGTRVEIK

SEQ ID NO: 64 - protein, 110 aa, Artificial Sequence
  Description of Artificial Sequence: Synthetic polypeptide
  8 4 LC humanized 188
DIQLTQSPSTLSASVGDRITITCQASQSISTALAWYQQKPGKAPKLLIYRASTLASGVPPRFSGSGSGTEFTLTISSLQPDDFATYYCQQGWSTVNVDNVFGQGTKVVVR

SEQ ID NO: 65 - protein, 110 aa, Artificial Sequence
  Description of Artificial Sequence: Synthetic polypeptide
  8 4 LC humanized 717
ELVMTQSPSSLSASVGDRVTITCQASQSISTALAWYQQKPGKAPNLLIYRASTLASGIPSRFSGSGSGTYFTLTINGLQPEDFATYYCQQGWSTVNVDNVFGGGTKVDIK

SEQ ID NO: 66 - protein, 110 aa, Artificial Sequence
  Description of Artificial Sequence: Synthetic polypeptide
  8 4 LC humanized 1048
SYELTQTPPSVSVSPGQTARITCQASQSISTALAWYQQKPGQAPKVLIYRASTLASGIPERFSGSSSGTTVTLTISGVQAEDEADYYCQQGWSTVNVDNVFGGGTKLTVL

SEQ ID NO: 67 - protein, 110 aa, Artificial Sequence
  Description of Artificial Sequence: Synthetic polypeptide
  8 4 LC humanized 849
AYELTQSPLSLSVTPGQPASISCQASQSISTALAWYLQKPGQPPQLLIYRASTLASGVPDRFSGSGSGTDFTLKISRVEAEDVGVYYCQQGWSTVNVDNVFGQGTKVEIK

SEQ ID NO: 68 - protein, 110 aa, Artificial Sequence
  Description of Artificial Sequence: Synthetic polypeptide
  8 4 LC humanized 1016
DIELTQSPSSLSASIGDRVSITCQASQSISTALAWYQQKPGKAPKLLIYRASTLASGVPSRFSGSGSGTDFTLTISSLQPEDFATFYCQQGWSTVNVDNVFGGGTRVEIK

SEQ ID NO: 69 - protein, 110 aa, Artificial Sequence
  Description of Artificial Sequence: Synthetic polypeptide
  8 4 LC humanized 978
EIVLTQSPSSLSASVGDRVTITCQASQSISTALAWYQQKPGKAPKLLIYRASTLASGVPSRFSGSGSGTDFTLTISNLQPEDFATYYCQQGWSTVNVDNVFGGGTKVEIK

SEQ ID NO: 70 - protein, 110 aa, Artificial Sequence
  Description of Artificial Sequence: Synthetic polypeptide
  8 4 LC humanized 706
DIQMTQYPSSLSASVGDRVTIACQASQSISTALAWYQQKPGKPPKLLIYRASTLASGVPSRFSGSGSGTDFTLTISCLQPEDVATYYCQQGWSTVNVDNVFGQGTRVEFK

SEQ ID NO: 71 - protein, 110 aa, Artificial Sequence
  Description of Artificial Sequence: Synthetic polypeptide
  8 4 LC humanized 278
ELVLTQSPSSLSASVGDRVTITCQASQSISTALAWCQQKPGKSPTLLIYRASTLASGVPSRFSGSGSGTGFTLTISGLQPEDFATYYCQQGWSTVNVDNVFGGGTKVEIR

SEQ ID NO: 72 - protein, 110 aa, Artificial Sequence
  Description of Artificial Sequence: Synthetic polypeptide
  8 4 LC humanized 129
EIVMTQSPSSLSASVGDRVTITCQASQSISTALAWYQHKPGKAPRLLIYRASTLASGVPSRFSGSGSGTDFTLTISSLQPDDFATYYCQQGWSTVNVDNVFGQGTKVEVK

SEQ ID NO: 73 - protein, 110 aa, Artificial Sequence
  Description of Artificial Sequence: Synthetic polypeptide
  8 4 LC humanized 1133
AYDMTTQPPSVSVSPGQTASITCQASQSISTALAWYQQKPGQSPVLVIYRASTLASGIPERFSGSNSGNTATLTISGTQAMDEADYYCQQGWSTVNVDNVFGTGTEVVVR

SEQ ID NO: 74 - protein, 110 aa, Artificial Sequence
  Description of Artificial Sequence: Synthetic polypeptide
  8 4 LC humanized 881
AYDMTQSPSSLSASVGDRVTITCQASQSISTALAWYQQKPGKAPNLLIYRASTLASGVPSRFSGSGSGTDFTLTISSLQPEDFATYYCQQGWSTVNVDNVFGGGTKVQIK

SEQ ID NO: 75 - protein, 110 aa, Artificial Sequence
  Description of Artificial Sequence: Synthetic polypeptide
  8 4 LC humanized 882
AYDMTQSPSSLSASVGDRVTITCQASQSISTALAWYQQKPGKAPKLLIYRASTLASGVPSRFSGSGFGTDFTFTISSLQPEDSATYYCQQGWSTVNVDNVFGQGTKLEIK

SEQ ID NO: 76 - protein, 110 aa, Artificial Sequence
  Description of Artificial Sequence: Synthetic polypeptide
  8 4 LC humanized 273
ELVMTQSPSSLSASVGDRVTITCQASQSISTALAWYQQKPGEAPKLLIYRASTLASGVPSRFSGSGSGTDFTLTISGLQSEDFATYYCQQGWSTVNVDNVFGQGTKVEIK

SEQ ID NO: 77 - protein, 110 aa, Artificial Sequence
  Description of Artificial Sequence: Synthetic polypeptide
  8 4 LC humanized 716
ELVMTQSPSSLSASEGDRVTITCQASQSISTALAWYQQKPGRAPKLLIHRASTLASGVPSRFSGSGSGTEFTLTISGLQSEDFATYYCQQGWSTVNVDNVFGGGTTVDVK

SEQ ID NO: 78 - protein, 110 aa, Artificial Sequence
  Description of Artificial Sequence: Synthetic polypeptide
  8 4 LC humanized 677
AYDMTQSPSFLSASVGDRVTITCQASQSISTALAWYQQKPGKAPKLLIYRASTLASGVPSRFSGSGSGTEFTLTISSLQPEDFATYYCQQGWSTVNVDNVFGQGTRLEIK

SEQ ID NO: 79 - protein, 110 aa, Artificial Sequence
  Description of Artificial Sequence: Synthetic polypeptide
  8 4 LC humanized 192
AYDMTQSPSSLSASVGDRVTITCQASQSISTALAWYQQKPGKAPKLLIYRASTLASGVPSRFSGSGSGTDFTLTISSLQAEDFTTYYCQQGWSTVNVDNVFGQGTKVEFK

SEQ ID NO: 80 - protein, 110 aa, Artificial Sequence
  Description of Artificial Sequence: Synthetic polypeptide
  8 4 LC humanized 802
AIRMTQSPSSFSASTGDRVTITCQASQSISTALAWYQQKPGKAPKLLIYRASTLASGVPSRFSGSGSGTDFTLTISCLQSEDFATYYCQQGWSTVNVDNVFGGGTKVEIK

SEQ ID NO: 81 - protein, 110 aa, Artificial Sequence
  Description of Artificial Sequence: Synthetic polypeptide
  8 4 LC humanized 54
AYGMTQSPDSLAVSLGERASINCQASQSISTALAWYQQKPGQPPKLLIYRASTLASGVPDRFSGGGSGTDFTLTISSLQAEDVAVYYCQQGWSTVNVDNVFGGGTKVEIK

SEQ ID NO: 82 - protein, 110 aa, Artificial Sequence
  Description of Artificial Sequence: Synthetic polypeptide
  8 4 LC humanized 173
AIQMTQSPFSLSASVGDRVTITCQASQSISTALAWFQQKPGKAPKSLIYRASTLASGVSSKFSGSGSGTDFTLTISSLQPEDFATYYCQQGWSTVNVDNVFGQGTRLVVR

SEQ ID NO: 83 - protein, 110 aa, Artificial Sequence
  Description of Artificial Sequence: Synthetic polypeptide
  8 4 LC humanized 224
AYDMTQTPASVSLSPGERATLSCQASQSISTALAWYQQKPGQAPRLLIYRASTLASGIPDRFRGSGSATDFTLTISRLEPEDFAVYYCQQGWSTVNVDNVFGGGTEVVVR

SEQ ID NO: 84 - protein, 110 aa, Artificial Sequence
  Description of Artificial Sequence: Synthetic polypeptide
  8 4 LC humanized 657
AYDMTQTPASVEVSVGDRVSITCQASQSISTALAWYQQKPGKAPKLLIYRASTLASGVPSRFSGSGSGTDFTLTITSLQPVDFATYYCQQGWSTVNVDNVFGPGTTVDAK

SEQ ID NO: 85 - protein, 117 aa, Artificial Sequence
  Description of Artificial Sequence: Synthetic polypeptide
  cl_CABBABABA_10_117; 8 4 HC humanized 866; 8 4 HC humanized 340; 8 4 HC humanized 336; 8 4 HC humanized 332; 8 4 HC humanized 322
VQLVESGGGVVQPGRSLRLSCAASGFTISNLAIIWVRQAPGKGLEWVADIDGRGDIYCATWAKGRFTISRDNSTLYLQMNSLRAEDTAVYYCAVDGDGSGWGDFNFWGQGTLVTVSS

SEQ ID NO: 86 - protein, 117 aa, Artificial Sequence
  Description of Artificial Sequence: Synthetic polypeptide
  cl_KABBABABA_13_117; 8 4 HC humanized 315; 8 4 HC humanized 314; 8 4 HC humanized 305; 8 4 HC humanized 303; 8 4 HC humanized 296
VQLVQSGGGVVQPGRSLRLSCAASGFTISNLAIIWVRQAPGKGLEWVADIDGRGDIYCATWAKGRFTISRDNSTLYLQMNSLRAEDTAVYYCAVDGDGSGWGDFNFWGQGTLVTVSS

SEQ ID NO: 87 - protein, 117 aa, Artificial Sequence
  Description of Artificial Sequence: Synthetic polypeptide
  cl_TABBABABA_8_117; 8 4 HC humanized 217; 8 4 HC humanized 197; 8 4 HC humanized 678; 8 4 HC humanized 978; 8 4 HC humanized 635
VQLVESGGGLVKPGGSLRLSCAASGFTISNLAIIWVRQAPGKGLEWVSDIDGRGDIYCATWAKGRFTISRDNASLYLQMNSLRAEDTAVYYCARDGDGSGWGDFNFWGQGTLVTVSS

SEQ ID NO: 88 - protein, 117 aa, Artificial Sequence
  Description of Artificial Sequence: Synthetic polypeptide
  cl_WABBABABA_7_117; 8 4 HC humanized 169; 8 4 HC humanized 122; 8 4 HC humanized 676; 8 4 HC humanized 893; 8 4 HC humanized 57
VQLVESGGGLVQPGGSLRLSCAASGFTISNLAIIWVRQAPGKGLEWVSDIDGRGDIYCATWAKGRFTISRDNSTLYLQMNSLRAEDTAVYYCAKDGDGSGWGDFNFWGQGTLVTVSS

SEQ ID NO: 89 - protein, 117 aa, Artificial Sequence
  Description of Artificial Sequence: Synthetic polypeptide
  cl_ZABBABABA_1_117; 8 4 HC humanized 17
VQLVESGGGLVQPGGSLRLSCAASGFTISNLAIIWVRQAPGRGLVWVSDIDGRGDIYCATWAKGRFTISRDNATLYLQMNNLRAEDTAVYYCARDGDGSGWGDFNFWGQGTLVTVSS

SEQ ID NO: 90 - protein, 117 aa, Artificial Sequence
  Description of Artificial Sequence: Synthetic polypeptide
  cl_CEBBABABA_1_117; 8 4 HC humanized 791
QSVLESGGGLVQPGGSLRLSCAASGFTISNLAIIWVRQAPGKGLEWVSDIDGRGDIYCATWARGRFTISRDNSTLYLQMNSLRAEDTAIYYCAKDGDGSGWGDFNFWGRGTHVTVSS

SEQ ID NO: 91 - protein, 117 aa, Artificial Sequence; identical to SEQ ID NO: 29
  Description of Artificial Sequence: Synthetic polypeptide
  cl_DEBBABABA_1_117; 8 4 HC humanized 673

SEQ ID NO: 92 - protein, 117 aa, Artificial Sequence; identical to SEQ ID NO: 30
  Description of Artificial Sequence: Synthetic polypeptide
  cl_GEBBABABA_1_117; 8 4 HC humanized 631

SEQ ID NO: 93 - protein, 117 aa, Artificial Sequence; identical to SEQ ID NO: 31
  Description of Artificial Sequence: Synthetic polypeptide
  cl_HEBBABABA_1_117; 8 4 HC humanized 1002

SEQ ID NO: 94 - protein, 117 aa, Artificial Sequence
  Description of Artificial Sequence: Synthetic polypeptide
  cl_KEBBABABA_1_117; 8 4 HC humanized 775
QSLEESGGGLVQPGGSLRLSCAASGFTISNLAIIWVRQASGKGLEWVSDIDGRGDIYCATWAKGRFTISRDNSTLYLQMNSLRAEDTAVYSCAVDGDGSGWGDFNFWGQGTLVTVSS

SEQ ID NO: 95 - protein, 117 aa, Artificial Sequence; identical to SEQ ID NO: 32
  Description of Artificial Sequence: Synthetic polypeptide
  cl_LEBBABABA_2_117; 8 4 HC humanized 771; 8 4 HC humanized 772

SEQ ID NO: 96 - protein, 117 aa, Artificial Sequence
  Description of Artificial Sequence: Synthetic polypeptide
  cl_NEBBABABA_1_117; 8 4 HC humanized 188
VQLVESGGGLVQPGGSLRLSCAASGFTISNLAIIWVRQAPGKGLEWASDIDGRGDIYCATWAKGRFTISRDSSTLYLQMNSLRTDDTAVYYCAADGDGSGWGDFNFWGQGTLVTVSS

SEQ ID NO: 97 - protein, 117 aa, Artificial Sequence
  Description of Artificial Sequence: Synthetic polypeptide
  cl_PEBBABABA_9_117; 8 4 HC humanized 186; 8 4 HC humanized 292; 8 4 HC humanized 283; 8 4 HC humanized 204; 8 4 HC humanized 201
VQLVESGGGVVQPGRSLRLSCAASGFTISNLAIIWVRQAPGKGLEWVADIDGRGDIYCATWAKGRFTISRDNSTLYLQMNSLRAEDTAVYYCAKDGDGSGWGDFNFWGQGTLVTVSS

SEQ ID NO: 98 - protein, 117 aa, Artificial Sequence
  Description of Artificial Sequence: Synthetic polypeptide
  cl_QEBBABABA_1_117; 8 4 HC humanized 717
QSVLESGGGWVQPGRSLRLSCAASGFTISNLAIIWVRQAPGKGLEWVADIDGRGDIYCATWAKGRFTISRDNASLYLEMKSLRAEDTAIYYCARDGDGSGWGDFNFWGQGVLVTVSS

SEQ ID NO: 99 - protein, 117 aa, Artificial Sequence
  Description of Artificial Sequence: Synthetic polypeptide
  cl_REBBABABA_2_117; 8 4 HC humanized 1048; 8 4 HC humanized 675
QSVEESGGGLVQPGGSLRLSCAASGFTISNLAIIWVRQAPGKGLEWVSDIDGRGDIYCATWAKGRFTISRDNASLYLQMNSLRAEDTAVYYCARDGDGSGWGDFNFWGQGTLVTVSS

SEQ ID NO: 100 - protein, 117 aa, Artificial Sequence; identical to SEQ ID NO: 33
  Description of Artificial Sequence: Synthetic polypeptide
  cl_SEBBABABA_1_117; 8 4 HC humanized 849

SEQ ID NO: 101 - protein, 117 aa, Artificial Sequence
  Description of Artificial Sequence: Synthetic polypeptide
  cl_TEBBABABA_3_117; 8 4 HC humanized 1016; 8 4 HC humanized 295; 8 4 HC humanized 319
VQLVQSGGGLVKPGGSLRLSCAASGFTISNLAIIWVRQAPGKGLEWVADIDGRGDIYCATWAKGRFTISRDNSTLYLQMNSLRAEDTAVYYCAVDGDGSGWGDFNFWGQGTLVTVSS

SEQ ID NO: 102 - protein, 117 aa, Artificial Sequence
  Description of Artificial Sequence: Synthetic polypeptide
  cl_XEBBABABA_2_117; 8 4 HC humanized 868; 8 4 HC humanized 55
QQLQESGGGLVQPGGSLRLSCSASGFTISNLAIIWVRQAPGKGLEYVSDIDGRGDIYCATWAKGRFTISRDNSTLYLQMSSLRAEDTAVYYCVKDGDGSGWGDFNFWGQGTLVTVSS

SEQ ID NO: 103 - protein, 117 aa, Artificial Sequence
  Description of Artificial Sequence: Synthetic polypeptide
  cl_YEBBABABA_1_117; 8 4 HC humanized 862
VRLVESGGGVVQPGRSLRLSCAASGFTISNLAIIWVRQAPGKGLEWVADIDGRGDIYCATWAKGRFTISRDNSTLHLQMNSLRAEDTAVYYCAKDGDGSGWGDFNFWGKGTTVTVSS

SEQ ID NO: 104 - protein, 117 aa, Artificial Sequence
  Description of Artificial Sequence: Synthetic polypeptide
  cl_ZEBBABABA_1_117; 8 4 HC humanized 715
VQLVESGGGLVQPGGSLRLSCAASGFTISNLAIIWVRQAPGKGLEWVSDIDGRGDIYCATWAKGRFTISRSKNTLYLQMNSLRAEDTAVYYCARDGDGSGWGDFNFWGQGTTVTVSS

SEQ ID NO: 105 - protein, 117 aa, Artificial Sequence; identical to SEQ ID NO: 34
  Description of Artificial Sequence: Synthetic polypeptide
  cl_BIBBABABA_1_117; 8 4 HC humanized 706

SEQ ID NO: 106 - protein, 117 aa, Artificial Sequence; identical to SEQ ID NO: 35
  Description of Artificial Sequence: Synthetic polypeptide
  cl_CIBBABABA_1_117; 8 4 HC humanized 703

SEQ ID NO: 107 - protein, 117 aa, Artificial Sequence
  Description of Artificial Sequence: Synthetic polypeptide
  cl_FIBBABABA_1_117; 8 4 HC humanized 341
VQLVQSGGSLVQPGRSLRLSCAASGFTISNLAIIWVRQAPGKGLEWVADIDGRGDIYCATWAKGRFTTSRDNSTLYLQMNSLRADDTAVYFCAVDGDGSGWGDFNFWGQGTLVTVSS

SEQ ID NO: 108 - protein, 117 aa, Artificial Sequence
  Description of Artificial Sequence: Synthetic polypeptide
  cl_KIBBABABA_1_117; 8 4 HC humanized 301
VQLVESGGDLVQPGESLRLSCAASGFTISNLAIIWVRQAPGKGLEWVSDIDGRGDIYCATWAKGRFTISRDNSTLYLQMNSLRAEDTAVYYCARDGDGSGWGDFNFWGQGTLVTVSS

SEQ ID NO: 109 - protein, 117 aa, Artificial Sequence; identical to SEQ ID NO: 36
  Description of Artificial Sequence: Synthetic polypeptide
  cl_QIBBABABA_1_117; 8 4 HC humanized 278

SEQ ID NO: 110 - protein, 117 aa, Artificial Sequence
  Description of Artificial Sequence: Synthetic polypeptide
  cl_TIBBABABA_1_117; 8 4 HC humanized 129
MQLVESGGGLVQPGRSLRLSCVTSGFTISNLAIIWVRQVPGKGLEWVSDIDGRGDIYCATWAKGRFTISRDNTSLYLQMNSLRPEDTAVYYCAKDGDGSGWGDFNFWGQGTLVTVSS

SEQ ID NO: 111 - protein, 117 aa, Artificial Sequence; identical to SEQ ID NO: 37
  Description of Artificial Sequence: Synthetic polypeptide
  cl_XIBBABABA_1_117; 8 4 HC humanized 800

SEQ ID NO: 112 - protein, 117 aa, Artificial Sequence
  Description of Artificial Sequence: Synthetic polypeptide
  cl_YIBBABABA_7_117; 8 4 HC humanized 1133; 8 4 HC humanized 881; 8 4 HC humanized 677; 8 4 HC humanized 192; 8 4 HC humanized 65
QSVEESGGGVVQPGRSLRLSCAASGFTISNLAIIWVRQAPGKGLEWVADIDGRGDIYCATWAKGRFTISRDNSTLYLQMNSLRAEDTAVYYCARDGDGSGWGDFNFWGQGTTVTVSS

SEQ ID NO: 113 - protein, 117 aa, Artificial Sequence
  Description of Artificial Sequence: Synthetic polypeptide
  cl_FOBBABABA_1_117; 8 4 HC humanized 882
QSVEESGGGLVQPGGSLRLSCAASGFTISNLAIIWVRQPPGKGLEWVGDIDGRGDIYCATWAKGRFTISRSKSTVYLQMNSLKTEDTAVYYCTADGDGSGWGDFNFWGQGMLVTVSS

SEQ ID NO: 114 - protein, 117 aa, Artificial Sequence
  Description of Artificial Sequence: Synthetic polypeptide
  cl_GOBBABABA_1_117; 8 4 HC humanized 660
QSVEESGGGLIQPGGSLRLSCAASGFTISNLAIIWVRQAPGKGLECVSDIDGRGDIYCATWAKGRFTISRDNSTLYLQMTSLRAEDTAVYYCALDGDGSGWGDFNFWGQGTLVTVSS

SEQ ID NO: 115 - protein, 117 aa, Artificial Sequence
  Description of Artificial Sequence: Synthetic polypeptide
  cl_HOBBABABA_2_117; 8 4 HC humanized 1051; 8 4 HC humanized 1050
VQLVESGGGLVKPGGSLRLSCAASGFTISNLAIIWVRQAPGKGLEWVGDIDGRGDIYCATWAKGRFTISRSKNTLYLQMNSLKTEDTAVYYCTVDGDGSGWGDFNFWGQGTLVTVSS

SEQ ID NO: 116 - protein, 117 aa, Artificial Sequence; identical to SEQ ID NO: 38
  Description of Artificial Sequence: Synthetic polypeptide
  cl_MOBBABABA_1_117; 8 4 HC humanized 809

SEQ ID NO: 117 - protein, 117 aa, Artificial Sequence; identical to SEQ ID NO: 39
  Description of Artificial Sequence: Synthetic polypeptide
  cl_VOBBABABA_1_117; 8 4 HC humanized 273

SEQ ID NO: 118 - protein, 117 aa, Artificial Sequence; identical to SEQ ID NO: 40
  Description of Artificial Sequence: Synthetic polypeptide
  cl_WOBBABABA_1_117; 8 4 HC humanized 716

SEQ ID NO: 119 - protein, 117 aa, Artificial Sequence; identical to SEQ ID NO: 41
  Description of Artificial Sequence: Synthetic polypeptide
  cl_ZOBBABABA_1_117; 8 4 HC humanized 202

SEQ ID NO: 120 - protein, 117 aa, Artificial Sequence
  Description of Artificial Sequence: Synthetic polypeptide
  cl_GUBBABABA_1_117; 8 4 HC humanized 54
VQLVESGGGLVQPGGSLRLSCATSGFTISNLAIIWVRQPPGKGLEWVSDIDGRGDIYCATWAKGRFTISRENATLYLQMNSLRAEDTAVYYCAVDGDGSGWGDFNFWGQGTLVTVSS

SEQ ID NO: 121 - protein, 117 aa, Artificial Sequence; identical to SEQ ID NO: 42
  Description of Artificial Sequence: Synthetic polypeptide
  cl_HUBBABABA_1_117; 8 4 HC humanized 21

SEQ ID NO: 122 - protein, 117 aa, Artificial Sequence
  Description of Artificial Sequence: Synthetic polypeptide
  cl_KUBBABABA_1_117; 8 4 HC humanized 788
QSVLESGGGLVQPGGSLRLSCAASGFTISNLAIIWVRQAPGKGLEWVSDIDGRGDIYCATWAKGRFTISRDNSTLFLQISSLRAEDTAVYYCAKDGDGSGWGDFNFWGPGTLVTVSS

SEQ ID NO: 123 - protein, 117 aa, Artificial Sequence
  Description of Artificial Sequence: Synthetic polypeptide
  cl_MUBBABABA_1_117; 8 4 HC humanized 762
VKLLESGGGLVQPGGSLRLSCAASGFTISNLAIIWVRQAPGKGLEWVADIDGRGDIYCATWAKGRFTISRDNSTLYLQMNSLGAEDTAVYYCARDGDGSGWGDFNFWGQGTLVTVSS

SEQ ID NO: 124 - protein, 117 aa, Artificial Sequence; identical to SEQ ID NO: 43
  Description of Artificial Sequence: Synthetic polypeptide
  cl_PUBBABABA_1_117; 8 4 HC humanized 173

SEQ ID NO: 125 - protein, 117 aa, Artificial Sequence
  Description of Artificial Sequence: Synthetic polypeptide
  cl_RUBBABABA_1_117; 8 4 HC humanized 224
QSVEESGGGLVKPGGSLRLSCAASGFTISNLAIIWVRQAPGKGLEWVGDIDGRGDIYCATWAKGRFTISRSKNTLYLQMNSLKTEDTAVYYCATDGDGSGWGDFNFWGQGTLVTVSS

SEQ ID NO: 126 - protein, 117 aa, Artificial Sequence
  Description of Artificial Sequence: Synthetic polypeptide
  cl_VUBBABABA_1_117; 8 4 HC humanized 672
QSVVESGGGLIQPGGSLRLSCAASGFTISNLAIIWVRQAPGKGLEWVSDIDGRGDIYCATWAKGRFTISRDNSTLYLQMNSLRAEDTAVYYCALDGDGSGWGDFNFWGQGTLVTVSS

SEQ ID NO: 127 - protein, 117 aa, Artificial Sequence
  Description of Artificial Sequence: Synthetic polypeptide
  cl_XUBBABABA_1_117; 8 4 HC humanized 267
QSVEQSGGGLVQPGESLRLSCAGSGFTISNLAIIWVRQAPGKGLEWVADIDGRGDIYCATWAKGRFTISRDNASLFLQMNSLRVEDTAVYYCARDGDGSGWGDFNFWGQGTLVTVSS

SEQ ID NO: 128 - protein, 117 aa, Artificial Sequence; identical to SEQ ID NO: 44
  Description of Artificial Sequence: Synthetic polypeptide
  cl_YUBBABABA_1_117; 8 4 HC humanized 23

SEQ ID NO: 129 - protein, 117 aa, Artificial Sequence
  Description of Artificial Sequence: Synthetic polypeptide
  cl_ZUBBABABA_1_117; 8 4 HC humanized 657
QSVEESGGRLVTPGGSLRLSCAASGFTISNLAIIWVRQAPGKGLEWVSDIDGRGDIYCATWAKGRFTISRDNSSLYLQMNSLRTEDSALYYCAIDGDGSGWGDFNFWGQGSLVTVSS

SEQ ID NO: 130 - protein, 117 aa, Artificial Sequence; identical to SEQ ID NO: 45
  Description of Artificial Sequence: Synthetic polypeptide
  cl_BACBABABA_1_117; 8 4 HC humanized 879

SEQ ID NO: 131 - protein, 110 aa, Artificial Sequence; identical to SEQ ID NO: 46
  Description of Artificial Sequence: Synthetic polypeptide
  cl_CACBABABA_1_110; 8 4 LC humanized 866

SEQ ID NO: 132 - protein, 110 aa, Artificial Sequence; identical to SEQ ID NO: 47
  Description of Artificial Sequence: Synthetic polypeptide
  cl_DACBABABA_1_110; 8 4 LC humanized 340

SEQ ID NO: 133 - protein, 110 aa, Artificial Sequence
  Description of Artificial Sequence: Synthetic polypeptide
  cl_FACBABABA_1_110; 8 4 LC humanized 336
DIQLTQSPSSLSASVGDRVTITCQASQSISTALAWYQQKPGKAPKLLIYRASTLASGVPSRFSGSGSGTDFTLTISSLQPEDFATYYCQQGWSTVNVDNVFGQGTKLEIK

SEQ ID NO: 134 - protein, 110 aa, Artificial Sequence
  Description of Artificial Sequence: Synthetic polypeptide
  cl_GACBABABA_1_110; 8 4 LC humanized 332
DIQMTQSPSSLSASVGDRVTITCQASQSISTALAWYQQKPGKAPKLLVYRASTLASGVPSRFSGSGSGTDFTLTISSLQPEDFATYYCQQGWSTVNVDNVFGQGTKVEIK

SEQ ID NO: 135 - protein, 110 aa, Artificial Sequence; identical to SEQ ID NO: 48
  Description of Artificial Sequence: Synthetic polypeptide
  cl_HACBABABA_1_110; 8 4 LC humanized 322

SEQ ID NO: 136 - protein, 110 aa, Artificial Sequence
  Description of Artificial Sequence: Synthetic polypeptide
  cl_KACBABABA_1_110; 8 4 LC humanized 315
DIQLTQSPSSLSASVGDRVTITCQASQSISTALAWYQQKPGKAPKLLIYRASTLASGVPSRFSGSGSGTGFTLTISSLQPEDFATYYCQQGWSTVNVDNVFGGGTKVEIK

SEQ ID NO: 137 - protein, 110 aa, Artificial Sequence
  Description of Artificial Sequence: Synthetic polypeptide
  cl_LACBABABA_1_110; 8 4 LC humanized 314
DIQMTQSPSSLSASVGDRVTITCQASQSISTALAWYQQKPGKAPNLLIYRASTLASGVPSRFSGSGSGTDFTLTISSLQPEDFATYYCQQGWSTVNVDNVFGQGTKVEIK

SEQ ID NO: 138 - protein, 110 aa, Artificial Sequence; identical to SEQ ID NO: 49
  Description of Artificial Sequence: Synthetic polypeptide
  cl_MACBABABA_1_110; 8 4 LC humanized 305

SEQ ID NO: 139 - protein, 110 aa, Artificial Sequence; identical to SEQ ID NO: 50
  Description of Artificial Sequence: Synthetic polypeptide
  cl_NACBABABA_1_110; 8 4 LC humanized 303

SEQ ID NO: 140 - protein, 110 aa, Artificial Sequence
  Description of Artificial Sequence: Synthetic polypeptide
  cl_PACBABABA_1_110; 8 4 LC humanized 296
DIQMTQSPSSLSASVGDRVTITCQASQSISTALAWYQQKPGKAPKLLIYRASTLASGVPSTFSGSGSGTDFTLTISSLQPEDFATYYCQQGWSTVNVDNVFGQGTKVEIK

SEQ ID NO: 141 - protein, 110 aa, Artificial Sequence
  Description of Artificial Sequence: Synthetic polypeptide
  cl_QACBABABA_1_110; 8 4 LC humanized 294
DIQMTQSPSSLSASVGDRVTITCQASQSISTALAWYQQKPGKAPKLLIYRASTLASGVPSRFSGSGSGTDFTLTISSLQPEDFATYYCQQGWSTVNVDNVFGGGTKVEIK

SEQ ID NO: 142 - protein, 110 aa, Artificial Sequence; identical to SEQ ID NO: 51
  Description of Artificial Sequence: Synthetic polypeptide
  cl_RACBABABA_1_110; 8 4 LC humanized 291

SEQ ID NO: 143 - protein, 110 aa, Artificial Sequence
  Description of Artificial Sequence: Synthetic polypeptide
  cl_SACBABABA_1_110; 8 4 LC humanized 284
DIQMTQSPSSLSASVGDRVTITCQASQSISTALAWYQQKPGKAPKSLIYRASTLASGVPSKFSGSGSGTEFTLTISSLQPDDFATYYCQQGWSTVNVDNVFGQGTRLEIK

SEQ ID NO: 144 - protein, 110 aa, Artificial Sequence; identical to SEQ ID NO: 52
  Description of Artificial Sequence: Synthetic polypeptide
  cl_TACBABABA_1_110; 8 4 LC humanized 217

SEQ ID NO: 145 - protein, 110 aa, Artificial Sequence; identical to SEQ ID NO: 53
  Description of Artificial Sequence: Synthetic polypeptide
  cl_VACBABABA_1_110; 8 4 LC humanized 197

SEQ ID NO: 146 - protein, 110 aa, Artificial Sequence; identical to SEQ ID NO: 54
  Description of Artificial Sequence: Synthetic polypeptide
  cl_WACBABABA_1_110; 8 4 LC humanized 169

SEQ ID NO: 147 - protein, 110 aa, Artificial Sequence
  Description of Artificial Sequence: Synthetic polypeptide
  cl_XACBABABA_1_110; 8 4 LC humanized 122
DVVMTQSPASLSASVGDRVTIICQASQSISTALAWYQQKPGKAPKLLIYRASTLASGVPSRFSGSGSRTDFTFTISSLQPEDIATYYCQQGWSTVNVDNVFGPGTKVDIK

SEQ ID NO: 148 - protein, 110 aa, Artificial Sequence; identical to SEQ ID NO: 46
  Description of Artificial Sequence: Synthetic polypeptide
  cl_YACBABABA_1_110; 8 4 LC humanized 44

SEQ ID NO: 149 - protein, 110 aa, Artificial Sequence; identical to SEQ ID NO: 55
  Description of Artificial Sequence: Synthetic polypeptide
  cl_ZACBABABA_1_110; 8 4 LC humanized 17

SEQ ID NO: 150 - protein, 110 aa, Artificial Sequence; identical to SEQ ID NO: 56
  Description of Artificial Sequence: Synthetic polypeptide
  cl_BECBABABA_1_110; 8 4 LC humanized 13

SEQ ID NO: 151 - protein, 110 aa, Artificial Sequence; identical to SEQ ID NO: 57
  Description of Artificial Sequence: Synthetic polypeptide
  cl_CECBABABA_1_110; 8 4 LC humanized 791

SEQ ID NO: 152 - protein, 110 aa, Artificial Sequence; identical to SEQ ID NO: 58
  Description of Artificial Sequence: Synthetic polypeptide
  cl_DECBABABA_1_110; 8 4 LC humanized 673

SEQ ID NO: 153 - protein, 110 aa, Artificial Sequence; identical to SEQ ID NO: 59
  Description of Artificial Sequence: Synthetic polypeptide
  cl_FECBABABA_1_110; 8 4 LC humanized 678

SEQ ID NO: 154 - protein, 110 aa, Artificial Sequence; identical to SEQ ID NO: 60
  Description of Artificial Sequence: Synthetic polypeptide
  cl_GECBABABA_1_110; 8 4 LC humanized 631

SEQ ID NO: 155 - protein, 110 aa, Artificial Sequence; identical to SEQ ID NO: 61
  Description of Artificial Sequence: Synthetic polypeptide
  cl_HECBABABA_1_110; 8 4 LC humanized 1002

SEQ ID NO: 156 - protein, 110 aa, Artificial Sequence; identical to SEQ ID NO: 62
  Description of Artificial Sequence: Synthetic polypeptide
  cl_KECBABABA_1_110; 8 4 LC humanized 775

SEQ ID NO: 157 - protein, 110 aa, Artificial Sequence; identical to SEQ ID NO: 63
  Description of Artificial Sequence: Synthetic polypeptide
  cl_LECBABABA_2_110; 8 4 LC humanized 771; 8 4 LC humanized 772

SEQ ID NO: 158 - protein, 110 aa, Artificial Sequence
  Description of Artificial Sequence: Synthetic polypeptide
  cl_MECBABABA_1_110; 8 4 LC humanized 676
AYDMTQSPATLSLSPGERATLSCQASQSISTALAWYQQKPGQAPRLLIYRASTLASGIPARFSGSGSGTDFTLTISSLEPEDFAVYYCQQGWSTVNVDNVFGGGTKVEIK

SEQ ID NO: 159 - protein, 110 aa, Artificial Sequence; identical to SEQ ID NO: 64
  Description of Artificial Sequence: Synthetic polypeptide
  cl_NECBABABA_1_110; 8 4 LC humanized 188

SEQ ID NO: 160 - protein, 110 aa, Artificial Sequence
  Description of Artificial Sequence: Synthetic polypeptide
  cl_PECBABABA_1_110; 8 4 LC humanized 186
DIQLTQSPSTLSASVGDRVTITCQASQSISTALAWYQQKPGKAPKLLIYRASTLASGVPSRFSGSGSGTEFTLTISSLQPDDFATYYCQQGWSTVNVDNVFGQGTKVVVR

SEQ ID NO: 161 - protein, 110 aa, Artificial Sequence; identical to SEQ ID NO: 65
  Description of Artificial Sequence: Synthetic polypeptide
  cl_QECBABABA_1_110; 8 4 LC humanized 717

SEQ ID NO: 162 - protein, 110 aa, Artificial Sequence; identical to SEQ ID NO: 66
  Description of Artificial Sequence: Synthetic polypeptide
  cl_RECBABABA_1_110; 8 4 LC humanized 1048

SEQ ID NO: 163 - protein, 110 aa, Artificial Sequence; identical to SEQ ID NO: 67
  Description of Artificial Sequence: Synthetic polypeptide
  cl_SECBABABA_1_110; 8 4 LC humanized 849

SEQ ID NO: 164 - protein, 110 aa, Artificial Sequence; identical to SEQ ID NO: 68
  Description of Artificial Sequence: Synthetic polypeptide
  cl_TECBABABA_1_110; 8 4 LC humanized 1016

SEQ ID NO: 165 - protein, 110 aa, Artificial Sequence; identical to SEQ ID NO: 69
  Description of Artificial Sequence: Synthetic polypeptide
  cl_VECBABABA_1_110; 8 4 LC humanized 978

SEQ ID NO: 166 - protein, 110 aa, Artificial Sequence
  Description of Artificial Sequence: Synthetic polypeptide
  cl_WECBABABA_1_110; 8 4 LC humanized 893
DIEMTQSPSSLSASVGDRVTITCQASQSISTALAWYQQKPGKAPKRLIQRASTLASGVPSRFSGSGSGTEFTLTISSLQPEDFATYHCQQGWSTVNVDNVFGGGTKVEIK

SEQ ID NO: 167 - protein, 110 aa, Artificial Sequence
  Description of Artificial Sequence: Synthetic polypeptide
  cl_XECBABABA_1_110; 8 4 LC humanized 868
DIVMTQSPDSLAVSLGERATINCQASQSISTALAWYQQKPGQPPKLLIYRASTLASGVPDRFSGSGSGTDFTLTISSLQAEDVAVYYCQQGWSTVNVDNVFGQGTKLEIK

SEQ ID NO: 168 - protein, 110 aa, Artificial Sequence
  Description of Artificial Sequence: Synthetic polypeptide
  cl_YECBABABA_1_110; 8 4 LC humanized 862
DIQMTQSPSSLSASVGDRVTITCQASQSISTALAWYQQKPGKAPKLLIYRASTLASGVPSRFSGSGSGTDFTLTISSLQPEDFATYYCQQGWSTVNVDNVFGQGTKVEIK

SEQ ID NO: 169 - protein, 110 aa, Artificial Sequence
  Description of Artificial Sequence: Synthetic polypeptide
  cl_ZECBABABA_1_110; 8 4 LC humanized 715
DIQMTQSPSSLSASVGDRVTITCQASQSISTALAWYQQKPGKAPKFLIYRASTLASGVPSRFSGSGSGTDFTLTISSLQPEDFATYYCQQGWSTVNVDNVFGQGTKVEIK

SEQ ID NO: 170 - protein, 110 aa, Artificial Sequence; identical to SEQ ID NO: 70
  Description of Artificial Sequence: Synthetic polypeptide
  cl_BICBABABA_1_110; 8 4 LC humanized 706

SEQ ID NO: 171 - protein, 110 aa, Artificial Sequence
  Description of Artificial Sequence: Synthetic polypeptide
  cl_CICBABABA_1_110; 8 4 LC humanized 703
DIVMTQSPDSLAVSLGERATINCQASQSISTALAWYQQKAGQPPKLLIYRASTLASGVPDRFSGSGSGTDFTLTISSLQAEDVAVYYCQQGWSTVNVDNVFGGGTKVEIK

SEQ ID NO: 172 - protein, 110 aa, Artificial Sequence
  Description of Artificial Sequence: Synthetic polypeptide
  cl_DICBABABA_1_110; 8 4 LC humanized 635
DIQMTQSPSSLSASVGDRVTITCQASQSISTALAWYQQKPGKVPKLLIYRASTLASGVPSRFSGSGSGTDFTLTISSLQPEDVATYYCQQGWSTVNVDNVFGQGTKLEIK

SEQ ID NO: 173 - protein, 110 aa, Artificial Sequence
  Description of Artificial Sequence: Synthetic polypeptide
  cl_FICBABABA_1_110; 8 4 LC humanized 341
DIQMTQSPSSLSASVGDRVTITCQASQSISTALAWYQQKPGKAPKLLIYRASTLASGVPSRFSGSGSGTDFTLTISSLQPEDFATYYCQQGWSTVNVDNVFGGGTKLEIK

SEQ ID NO: 174 - protein, 110 aa, Artificial Sequence
  Description of Artificial Sequence: Synthetic polypeptide
  cl_GICBABABA_1_110; 8 4 LC humanized 328
DIQMTQSPSSLSASVGDRVTITCQASQSISTALAWYQQKPGKAPKLLIYRASTLASGVPSRFSGSGSGTDFTLTISSLQPEDFATYYCQQGWSTVNVDNVFGRGTKVEIK

SEQ ID NO: 175 - protein, 110 aa, Artificial Sequence
  Description of Artificial Sequence: Synthetic polypeptide
  cl_HICBABABA_1_110; 8 4 LC humanized 324
DIQMTQSPSSLSASVGDRVTITCQASQSISTALAWYQQKPGNAPKSLIYRASTLASGVPSKFSGSGSGTDFTLTISSLQPEDFATYYCQQGWSTVNVDNVFGGGTKVEIK

SEQ ID NO: 176 - protein, 110 aa, Artificial Sequence
  Description of Artificial Sequence: Synthetic polypeptide
  cl_KICBABABA_1_110; 8 4 LC humanized 301
DIQMTQSPDSLAVSLGERATINCQASQSISTALAWYQQKPGQPPKLLIYRASTLASGVPDRFSGSGSGTDFTLTISSLQAEDVAVYYCQQGWSTVNVDNVFGQGTKLEIK

SEQ ID NO: 177 - protein, 110 aa, Artificial Sequence
  Description of Artificial Sequence: Synthetic polypeptide
  cl_LICBABABA_1_110; 8 4 LC humanized 295
DIQMTQSPSSLSASVGDRVTITCQASQSISTALAWYQQKPGKAPKLLIYRASTLASGVPSRFSGSGSGTDFTLTISSLQPEDFATYYCQQGWSTVNVDNVFGQGTRLEIK

SEQ ID NO: 178 - protein, 110 aa, Artificial Sequence
  Description of Artificial Sequence: Synthetic polypeptide
  cl_MICBABABA_1_110; 8 4 LC humanized 292
DIQMTQSPSSLSASVGDRVTITCQASQSISTALAWYQQKPGKAPNLLIYRASTLASGVPSRFSGSVSGTDFTLTISSLQPEDFATYYCQQGWSTVNVDNVFGGGTKVEIK

SEQ ID NO: 179 - protein, 110 aa, Artificial Sequence
  Description of Artificial Sequence: Synthetic polypeptide
  cl_NICBABABA_1_110; 8 4 LC humanized 283
DIQLTQSPSSVSASVGDRVTITCQASQSISTALAWYQQKPGKAPKLLIYRASTLASGVPSRFSGSGSGTDFTLTISSLQPEDFATYYCQQGWSTVNVDNVFGQGTRLEIK

SEQ ID NO: 180 - protein, 110 aa, Artificial Sequence
  Description of Artificial Sequence: Synthetic polypeptide
  cl_PICBABABA_1_110; 8 4 LC humanized 282
DIQMTQSPSSVSASVGDRVTITCQASQSISTALAWYQQKLGKAPKLLIYRASTLASGVPSRFSGSGSGTDFTLTISSLQPEDFATYYCQQGWSTVNVDNVFGGGTKVEIK

SEQ ID NO: 181 - protein, 110 aa, Artificial Sequence; identical to SEQ ID NO: 71
  Description of Artificial Sequence: Synthetic polypeptide
  cl_QICBABABA_1_110; 8 4 LC humanized 278

SEQ ID NO: 182 - protein, 110 aa, Artificial Sequence
  Description of Artificial Sequence: Synthetic polypeptide
  cl_RICBABABA_1_110; 8 4 LC humanized 204
DIQLTQSPSSLSASVGDRVTITCQASQSISTALAWYQQKPGKAPKLLIYRASTLASGVPSRFSGSGSGTDFTLTISSLQPEDFATYYCQQGWSTVNVDNVFGQGTKVEIK

SEQ ID NO: 183 - protein, 110 aa, Artificial Sequence
  Description of Artificial Sequence: Synthetic polypeptide
  cl_SICBABABA_1_110; 8 4 LC humanized 201
DIRVTQSPSSLSASVGDRVTITCQASQSISTALAWYQQKPGKAPKLLIYRASTLASGVPSRFSGSGSGTDFTFTISSLQPEDIATYYCQQGWSTVNVDNVFGGGTKVDIK

SEQ ID NO: 184 - protein, 110 aa, Artificial Sequence; identical to SEQ ID NO: 72
  Description of Artificial Sequence: Synthetic polypeptide
  cl_TICBABABA_1_110; 8 4 LC humanized 129

SEQ ID NO: 185 - protein, 110 aa, Artificial Sequence
  Description of Artificial Sequence: Synthetic polypeptide
  cl_VICBABABA_1_110; 8 4 LC humanized 108
DVVMTQSPSSVSASVGDRVTITCQASQSISTALAWYQQKPGKAPKLLIYRASTLASGVPSRFSGSGSGTDFTLTITSLQPEDFATYYCQQGWSTVNVDNVFGGGTKVEIK

SEQ ID NO: 186 - protein, 110 aa, Artificial Sequence
  Description of Artificial Sequence: Synthetic polypeptide
  cl_WICBABABA_1_110; 8 4 LC humanized 57
DIQMTQSPSSLSASVGDRVTITCQASQSISTALAWYQQKPGKAPKRLIYRASTLASGVPSRFSGSGSGTEFTLTISSLQPEDFATYYCQQGWSTVNVDNVFGQGTRLEIK

SEQ ID NO: 187 - protein, 110 aa, Artificial Sequence
  Description of Artificial Sequence: Synthetic polypeptide
  cl_XICBABABA_1_110; 8 4 LC humanized 800
AYELTQTPPSLSVTPGQPASISCQASQSISTALAWYLQKPGQPPQLLIYRASTLASGVPDRFSGSGSGTDFTLKISRVEAEDVGVYYCQQGWSTVNVDNVFGQGTKVEIK

SEQ ID NO: 188 - protein, 110 aa, Artificial Sequence; identical to SEQ ID NO: 73
  Description of Artificial Sequence: Synthetic polypeptide
  cl_YICBABABA_1_110; 8 4 LC humanized 1133

SEQ ID NO: 189 - protein, 110 aa, Artificial Sequence
  Description of Artificial Sequence: Synthetic polypeptide
  cl_ZICBABABA_1_110; 8 4 LC humanized 621
AYELTQSPSSLSASVGDRVTITCQASQSISTALAWYQQKPGKAPKLLIYRASTLASGVPSRFSGSGSGTDFTLTISSLQPEDFATYYCQQGWSTVNVDNVFGQGTKVEIK

SEQ ID NO: 190 - protein, 110 aa, Artificial Sequence; identical to SEQ ID NO: 74
  Description of Artificial Sequence: Synthetic polypeptide
  cl_COCBABABA_1_110; 8 4 LC humanized 881

SEQ ID NO: 191 - protein, 110 aa, Artificial Sequence
  Description of Artificial Sequence: Synthetic polypeptide
  cl_DOCBABABA_1_110; 8 4 LC humanized 55
AYDMTQTPASVEVSPGERATLSCQASQSISTALAWYQQKPGQAPRLLIYRASTLASGIPARFSGSGSGTEFTLTISSLQSEDFAVYYCQQGWSTVNVDNVFGQGTEVVVR

SEQ ID NO: 192 - protein, 110 aa, Artificial Sequence; identical to SEQ ID NO: 75
  Description of Artificial Sequence: Synthetic polypeptide
  cl_FOCBABABA_1_110; 8 4 LC humanized 882

SEQ ID NO: 193 - protein, 110 aa, Artificial Sequence
  Description of Artificial Sequence: Synthetic polypeptide
  cl_GOCBABABA_1_110; 8 4 LC humanized 660
AYVMTQSPATLSLSPGERATLSCQASQSISTALAWYQQRPGQAPRLLIYRASTLASGIPARFSGSGSGTDFTLTISSLEPEDFAVYYCQQGWSTVNVDNVFGGGTKVEIK

SEQ ID NO: 194 - protein, 110 aa, Artificial Sequence
  Description of Artificial Sequence: Synthetic polypeptide
  cl_HOCBABABA_1_110; 8 4 LC humanized 1051
SYELTQTPPSVSVSPGQTARITCQASQSISTALAWYQQKPGQAPVLVIYRASTLASGIPERFSGSSSGTTVTLTISGVQAEDEADYYCQQGWSTVNVDNVFGTGTKVTVL

SEQ ID NO: 195 - protein, 110 aa, Artificial Sequence; identical to SEQ ID NO: 194
  Description of Artificial Sequence: Synthetic polypeptide
  cl_KOCBABABA_1_110; 8 4 LC humanized 1050

SEQ ID NO: 196 - protein, 110 aa, Artificial Sequence; identical to SEQ ID NO: 141
  Description of Artificial Sequence: Synthetic polypeptide
  cl_LOCBABABA_1_110; 8 4 LC humanized 860

SEQ ID NO: 197 - protein, 110 aa, Artificial Sequence
  Description of Artificial Sequence: Synthetic polypeptide
  cl_MOCBABABA_1_110; 8 4 LC humanized 809
DIQMTQSPSSVSASVRDRVTITCQASQSISTALAWYQQKPGKAPKLLIYRASTLASGVPSRFSGSGSGTDFTLTISSLQPEDFATYYCQQGWSTVNVDNVFGPGTKVDIK

SEQ ID NO: 198 - protein, 110 aa, Artificial Sequence; identical to SEQ ID NO: 168
  Description of Artificial Sequence: Synthetic polypeptide
  cl_NOCBABABA_1_110; 8 4 LC humanized 346

SEQ ID NO: 199 - protein, 110 aa, Artificial Sequence
  Description of Artificial Sequence: Synthetic polypeptide
  cl_POCBABABA_1_110; 8 4 LC humanized 345
DIQMTQSPSSLSASVGDRVTITCQASQSISTALAWYQQKPGKAPKLLIYRASTLASGVPSRFSGSGSGTDFTFTISSLQPDDFATYYCQQGWSTVNVDNVFGGGTKVEIK

SEQ ID NO: 200 - protein, 110 aa, Artificial Sequence
  Description of Artificial Sequence: Synthetic polypeptide
  cl_QOCBABABA_1_110; 8 4 LC humanized 334
DIQMTQSPSFVSASVGDRVTITCQASQSISTALAWYQQKPGKAPKLLIYRASTLASGVPSRFSGSGSGTDFTLTISSLQPEDFATYYCQQGWSTVNVDNVFGGGTKVEIK

SEQ ID NO: 201 - protein, 110 aa, Artificial Sequence; identical to SEQ ID NO: 168
  Description of Artificial Sequence: Synthetic polypeptide
  cl_ROCBABABA_1_110; 8 4 LC humanized 319

SEQ ID NO: 202 - protein, 110 aa, Artificial Sequence; identical to SEQ ID NO: 141
  Description of Artificial Sequence: Synthetic polypeptide
  cl_SOCBABABA_1_110; 8 4 LC humanized 308

SEQ ID NO: 203 - protein, 110 aa, Artificial Sequence
  Description of Artificial Sequence: Synthetic polypeptide
  cl_TOCBABABA_1_110; 8 4 LC humanized 281
DIQLTQSPSSVSASVGDRVTITCQASQSISTALAWYQQKPGKAPKLLIYRASTLASGVPSRFSGSGSGTDFTLTISSLQPEDFATYYCQQGWSTVNVDNVFGGGTKVDIK

SEQ ID NO: 204 - protein, 110 aa, Artificial Sequence; identical to SEQ ID NO: 76
  Description of Artificial Sequence: Synthetic polypeptide
  cl_VOCBABABA_1_110; 8 4 LC humanized 273

SEQ ID NO: 205 - protein, 110 aa, Artificial Sequence; identical to SEQ ID NO: 77
  Description of Artificial Sequence: Synthetic polypeptide
  cl_WOCBABABA_1_110; 8 4 LC humanized 716

SEQ ID NO: 206 - protein, 110 aa, Artificial Sequence; identical to SEQ ID NO: 78
  Description of Artificial Sequence: Synthetic polypeptide
  cl_XOCBABABA_1_110; 8 4 LC humanized 677

SEQ ID NO: 207 - protein, 110 aa, Artificial Sequence; identical to SEQ ID NO: 79
  Description of Artificial Sequence: Synthetic polypeptide
  cl_YOCBABABA_1_110; 8 4 LC humanized 192

SEQ ID NO: 208 - protein, 110 aa, Artificial Sequence
  Description of Artificial Sequence: Synthetic polypeptide
  cl_ZOCBABABA_1_110; 8 4 LC humanized 202
DIRMTQSPSSLSASVGDRVTITCQASQSISTALAWYQQKPGKVPKLLIYRASTLASGVPSRFSGSGSGTDFTLTISSLQPEDVATYYCQQGWSTVNVDNVFGPGTKVVVR

SEQ ID NO: 209 - protein, 110 aa, Artificial Sequence; identical to SEQ ID NO: 80
  Description of Artificial Sequence: Synthetic polypeptide
  cl_BUCBABABA_1_110; 8 4 LC humanized 802

SEQ ID NO: 210 - protein, 110 aa, Artificial Sequence
  Description of Artificial Sequence: Synthetic polypeptide
  cl_CUCBABABA_1_110; 8 4 LC humanized 347
DIQMTQSPSSLSASVGDRVSITCQASQSISTALAWYQQKPGKAPKRLIYRASTLASGVPSRFSGSGSGTEFTLTISSLQPDDFATYYCQQGWSTVNVDNVFGGGTKVEIK

SEQ ID NO: 211 - protein, 110 aa, Artificial Sequence
  Description of Artificial Sequence: Synthetic polypeptide
  cl_DUCBABABA_1_110; 8 4 LC humanized 339
DIQLTQSPSSLSASVGDRVTITCQASQSISTALAWYQQKPGKAPKLLIYRASTLASGVPSRFSGSGSGTEFTLTISSLQPDDFATYYCQQGWSTVNVDNVFGGGTKVEIK

SEQ ID NO: 212 - protein, 110 aa, Artificial Sequence
  Description of Artificial Sequence: Synthetic polypeptide
  cl_FUCBABABA_1_110; 8 4 LC humanized 168
DIVMTQSPSTLSASVGDRVTITCQASQSISTALAWYQQKPGKAPKLLIYRASTLASGVPSRFSGSGSGTEFTLTISGLQPEDFATYYCQQGWSTVNVDNVFGGGTKLEIK

SEQ ID NO: 213 - protein, 110 aa, Artificial Sequence; identical to SEQ ID NO: 81
  Description of Artificial Sequence: Synthetic polypeptide
  cl_GUCBABABA_1_110; 8 4 LC humanized 54

SEQ ID NO: 214 - protein, 110 aa, Artificial Sequence
  Description of Artificial Sequence: Synthetic polypeptide
  cl_HUCBABABA_1_110; 8 4 LC humanized 21
DIQMTQSPSSLSASVGDRVTITCQASQSISTALAWYQQKPGKAPKVLIYRASTLASGVPSRFSGSGSGTDFTLTISSLQPEDFATYYCQQGWSTVNVDNVFGPGTKVEVR

SEQ ID NO: 215 - protein, 110 aa, Artificial Sequence
  Description of Artificial Sequence: Synthetic polypeptide
  cl_KUCBABABA_1_110; 8 4 LC humanized 788
AYELTQTPLSSPVTLGQPASISCQASQSISTALAWLQQRPGQPPRLLIYRASTLASGVPDRFSGSGAGTDFTLKISRVEAEDVGIYYCQQGWSTVNVDNVFGQGTKVEIK

SEQ ID NO: 216 - protein, 110 aa, Artificial Sequence
  Description of Artificial Sequence: Synthetic polypeptide
  cl_LUCBABABA_1_110; 8 4 LC humanized 675
AYDMTQSPSSLSASVGDRVTITCQASQSISTALAWYQQKPGKAPKLLIYRASTLASGVPSRFSGSGSGTEFTLTITSLQPEDFATYYCQQGWSTVNVDNVFGPGTKLEIK

SEQ ID NO: 217 - protein, 110 aa, Artificial Sequence
  Description of Artificial Sequence: Synthetic polypeptide
  cl_MUCBABABA_1_110; 8 4 LC humanized 762
AYELTQSPDSLAVSLGERATINCQASQSISTALAWYQQKPGQPPKLLIYRASTLASGVPDRFSGSGSGTDFTLTISSLQAEDVAVYYCQQGWSTVNVDNVFGGGTKVEIK

SEQ ID NO: 218 - protein, 110 aa, Artificial Sequence
  Description of Artificial Sequence: Synthetic polypeptide
  cl_NUCBABABA_1_110; 8 4 LC humanized 818
AYDMTQTPSSVSASVGDRVTITCQASQSISTALAWYQQKPGKAPKLLIYRASTLASGVPSRFSGSGSGTDFTLTISSLQPEDFATYYCQQGWSTVNVDNVFGQGTKVEIK

SEQ ID NO: 219 - protein, 110 aa, Artificial Sequence; identical to SEQ ID NO: 82
  Description of Artificial Sequence: Synthetic polypeptide
  cl_PUCBABABA_1_110; 8 4 LC humanized 173

SEQ ID NO: 220 - protein, 110 aa, Artificial Sequence
  Description of Artificial Sequence: Synthetic polypeptide
  cl_QUCBABABA_1_110; 8 4 LC humanized 65
DIQMTQSPSTLSASVGDRVTITCQASQSISTALAWYQQKPGKAPKLLIYRASTLASGVPSRFSGSGSGTEFTLTISSLQPDDFATYYCQQGWSTVNVDNVFGQGTKVEIK

SEQ ID NO: 221 - protein, 110 aa, Artificial Sequence; identical to SEQ ID NO: 83
  Description of Artificial Sequence: Synthetic polypeptide
  cl_RUCBABABA_1_110; 8 4 LC humanized 224

SEQ ID NO: 222 - protein, 110 aa, Artificial Sequence
  Description of Artificial Sequence: Synthetic polypeptide
  cl_SUCBABABA_1_110; 8 4 LC humanized 230
AYDMTQTPASVSASVGDRVTITCQASQSISTALAWYQQKPGKAPKVLIYRASTLASGVPSRFSGSGSGTDFTLTISTLQPEDFATYYCQQGWSTVNVDNVFGQGTKLEIK

SEQ ID NO: 223 - protein, 110 aa, Artificial Sequence
  Description of Artificial Sequence: Synthetic polypeptide
  cl_TUCBABABA_1_110; 8 4 LC humanized 880
AYDMTQSPSSLSASVGDRVNITCQASQSISTALAWYQQKPGKAPKLLIYRASTLASGVPSRFSGSGSGTDFTLTISSLQPEDFATYYCQQGWSTVNVDNVFGPGTKVDIK

SEQ ID NO: 224 - protein, 110 aa, Artificial Sequence
  Description of Artificial Sequence: Synthetic polypeptide
  cl_VUCBABABA_1_110; 8 4 LC humanized 672
AYDMTQSPSSLSASVGDRVTITCQASQSISTALAWYQQKPGKAPKLLIYRASTLASGVPSRFSGSGSGTDFTLTISSLQPEDFATYYCQQGWSTVNVDNVFGQGTKLEIK

SEQ ID NO: 225 - protein, 110 aa, Artificial Sequence
  Description of Artificial Sequence: Synthetic polypeptide
  cl_WUCBABABA_1_110; 8 4 LC humanized 299
DIQMTQSPSSVSASVGDRVTITCQASQSISTALAWYQQKPGKAPKLLIYRASTLASGVPSRFSGSGSGTEFTLTISSLQPDDFATYYCQQGWSTVNVDNVFGGGTKVEIK

SEQ ID NO: 226 - protein, 110 aa, Artificial Sequence
  Description of Artificial Sequence: Synthetic polypeptide
  cl_XUCBABABA_1_110; 8 4 LC humanized 267
AYDMTQSPSTLAASVGDRVTITCQASQSISTALAWYQQKPGKAPKLLIYRASTLASGVPSRFSGSGSGTEFTLTISSLQPDDFATYYCQQGWSTVNVDNVFGQGTKVEVK

SEQ ID NO: 227 - protein, 110 aa, Artificial Sequence
  Description of Artificial Sequence: Synthetic polypeptide
  cl_YUCBABABA_1_110; 8 4 LC humanized 23
AYELTQSPSSLSASVGDRVTITCQASQSISTALAWYQQKPGKAPKLLIYRASTLASGVPSRFSGSGSGTDFTLTISSLQPEDFATYYCQQGWSTVNVDNVFGPGTKVDIK

SEQ ID NO: 228 - protein, 110 aa, Artificial Sequence; identical to SEQ ID NO: 84
  Description of Artificial Sequence: Synthetic polypeptide
  cl_ZUCBABABA_1_110; 8 4 LC humanized 657

SEQ ID NO: 229 - protein, 110 aa, Artificial Sequence
  Description of Artificial Sequence: Synthetic polypeptide
  cl_BADBABABA_1_110; 8 4 LC humanized 879
AYDMTQSPSSLSASVGDRVTITCQASQSISTALAWYQQKPGKAPKLLIYRASTLASGVPSRFSGSGSGTDFTLTISSLQPEDFATYFCQQGWSTVNVDNVFGGGTKVEIK

SEQ ID NO: 230 - protein, 117 aa, Artificial Sequence
  Description of Artificial Sequence: Synthetic polypeptide
  cl_CABBABABA_15_117; 8 4 HC humanized 356; 8 4 HC humanized 340; 8 4 HC humanized 335; 8 4 HC humanized 303; 8 4 HC humanized 287
VQLVESGGGVVQPGGSLRLSCAASGFTISNLAIIWVRQAPGKGLEWVSDIDGRGDIYCATWAKGRFTISRDNSSLYLQMNSLRAEDTAVYYCARDGDGSGWGDFNFWGPGTLVTVSS

SEQ ID NO: 231 - protein, 117 aa, Artificial Sequence
  Description of Artificial Sequence: Synthetic polypeptide
  cl_LABBABABA_85_117; 8 4 HC humanized 2049; 8 4 HC humanized 2033; 8 4 HC humanized 1360; 8 4 HC humanized 1344; 8 4 HC humanized 777
VQLVESGGGLVQPGGSLRLSCAASGFTISNLAIIWVRQAPGKGLEWVSDIDGRGDIYCATWAKGRFTISRDNSTLYLQMNSLRAEDTAVYYCARDGDGSGWGDFNFWGPGTLVTVSS

SEQ ID NO: 232 - protein, 110 aa, Artificial Sequence
  Description of Artificial Sequence: Synthetic polypeptide
  cl_CACBABABA_76_110; 8 4 LC humanized 356; 8 4 LC humanized 340; 8 4 LC humanized 335; 8 4 LC humanized 303; 8 4 LC humanized 287
AYDMTQSPSSLSASVGDRVTITCQASQSISTALAWYQQKPGKAPKLLIYRASTLASGVPSRFSGSGSGTDFTLTISSLQPEDFATYYCQQGWSTVNVDNVFGGGTEVVVR

SEQ ID NO: 233 - protein, 110 aa, Artificial Sequence
  Description of Artificial Sequence: Synthetic polypeptide
  cl_LACBABABA_2_110; 8 4 LC humanized 2049; 8 4 LC humanized 2033
AYDMTQSPDSLAVSLGERATINCQASQSISTALAWYQQKPGQPPKLLIYRASTLASGVPDRFSGSGSGTDFTLTISSLQAEDVAVYYCQQGWSTVNVDNVFGGGTEVVVR

SEQ ID NO: 234 - protein, 110 aa, Artificial Sequence
  Description of Artificial Sequence: Synthetic polypeptide
  cl_NACBABABA_2_110; 8 4 LC humanized 1360; 8 4 LC humanized 1344
AYDMTQTPLSLSVTPGQPASISCQASQSISTALAWYLQKPGQPPQLLIYRASTLASGVPDRFSGSGSGTDFTLKISRVEAEDVGVYYCQQGWSTVNVDNVFGGGTEVVVR

SEQ ID NO: 235 - protein, 110 aa, Artificial Sequence
  Description of Artificial Sequence: Synthetic polypeptide
  cl_CECBABABA_5_110; 8 4 LC humanized 2207; 8 4 LC humanized 2206; 8 4 LC humanized 2197; 8 4 LC humanized 2208; 8 4 LC humanized 2192
AYDMTQSPAFLSVTPGEKVTITCQASQSISTALAWYQQKPDQAPKLLIKRASTLASGVPSRFSGSGSGTDFTFTISSLEAEDAATYYCQQGWSTVNVDNVFGGGTEVVVR

SEQ ID NO: 236 - protein, 110 aa, Artificial Sequence
  Description of Artificial Sequence: Synthetic polypeptide
  cl_DICBABABA_15_110; 8 4 LC humanized 2263; 8 4 LC humanized 2262; 8 4 LC humanized 2258; 8 4 LC humanized 2257; 8 4 LC humanized 2256
AYDMTQSPASLAVSPGQRATITCQASQSISTALAWYQQKPGQPPKLLIYRASTLASGVPARFSGSGSGTDFTLTINPVEANDTANYYCQQGWSTVNVDNVFGGGTEVVVR

SEQ ID NO: 237 - protein, 117 aa, Artificial Sequence
  Description of Artificial Sequence: Synthetic polypeptide
  cl_CABBABABA_2_117; 8 4 HC humanized 356; 8 4 HC humanized 303
VQLVESRGVLVQPGGSLRLSCAASGFTISNLAIIWVRQAPGKGLEWVSDIDGRGDIYCATWAKGRFTISRDNSTLHLQMNSLRAEDTAVYYCKKDGDGSGWGDFNFWGPGTLVTVSS

SEQ ID NO: 238 - protein, 117 aa, Artificial Sequence
  Description of Artificial Sequence: Synthetic polypeptide
  cl_DABBABABA_17_117; 8 4 HC humanized 340; 8 4 HC humanized 335; 8 4 HC humanized 287; 8 4 HC humanized 282; 8 4 HC humanized 2207
VQLVESGGGLVQPGGSLRLSCAASGFTISNLAIIWVRQAPGKGLEWVSDIDGRGDIYCATWAKGRFTISRDNASLYLQMNSLRAEDTAVYYCARDGDGSGWGDFNFWGPGTLVTVSS

SEQ ID NO: 239 - protein, 117 aa, Artificial Sequence
  Description of Artificial Sequence: Synthetic polypeptide
  cl_LABBABABA_37_117; 8 4 HC humanized 2049; 8 4 HC humanized 2033; 8 4 HC humanized 1360; 8 4 HC humanized 1344; 8 4 HC humanized 777
VQLVESGGGLVQPGGSLRLSCAASGFTISNLAIIWVRQAPGKGLEWVGDIDGRGDIYCATWAKGRFTISRSKNTLYLQMNSLKTEDTAVYYCTRDGDGSGWGDFNFWGPGTLVTVSS

SEQ ID NO: 240 - protein, 117 aa, Artificial Sequence; identical to SEQ ID NO: 231
  Description of Artificial Sequence: Synthetic polypeptide
  cl_DEBBABABA_22_117; 8 4 HC humanized 2206; 8 4 HC humanized 988; 8 4 HC humanized 987; 8 4 HC humanized 935; 8 4 HC humanized 934

SEQ ID NO: 241 - protein, 117 aa, Artificial Sequence
  Description of Artificial Sequence: Synthetic polypeptide
  cl_FEBBABABA_16_117; 8 4 HC humanized 2197; 8 4 HC humanized 978; 8 4 HC humanized 925; 8 4 HC humanized 660; 8 4 HC humanized 395
VQLLESGGGLVQPGGSLRLSCAASGFTISNLAIIWVRQAPGKGLEWVSDIDGRGDIYCATWAKGRFTISRDNSTLYLQMNSLRAEDTAVYYCAKDGDGSGWGDFNFWGPGTLVTVSS

SEQ ID NO: 242 - protein, 117 aa, Artificial Sequence
  Description of Artificial Sequence: Synthetic polypeptide
  cl_HIBBABABA_3_117; 8 4 HC humanized 2257; 8 4 HC humanized 349; 8 4 HC humanized 296
VQLVESGGGLVQPGRSLRLSCTASGFTISNLAIIWFRQAPGKGLEWVGDIDGRGDIYCATWAKGRFTISRSKSIAYLQMNSLKTEDTAVYYCTRDGDGSGWGDFNFWGPGTLVTVSS

SEQ ID NO: 243 - protein, 117 aa, Artificial Sequence
  Description of Artificial Sequence: Synthetic polypeptide
  cl_LIBBABABA_3_117; 8 4 HC humanized 2254; 8 4 HC humanized 346; 8 4 HC humanized 293
VQLVESGGVVVQPGGSLRLSCAASGFTISNLAIIWVRQAPGKGLEWVSDIDGRGDIYCATWAKGRFTISRDNSSLYLQMNSLRTEDTALYYCAKDGDGSGWGDFNFWGPGTLVTVSS

SEQ ID NO: 244 - protein, 110 aa, Artificial Sequence
  Description of Artificial Sequence: Synthetic polypeptide
  cl_CACBABABA_1_110; 8 4 LC humanized 356
AYDMTQSPSSVSASVGDRVTITCQASQSISTALAWYQQKPGKAPKLLIYRASTLASGVPSRFSGSGSGTDFTLTISSLQPEDFATYYCQQGWSTVNVDNVFGGGTEVVVR

SEQ ID NO: 245 - protein, 110 aa, Artificial Sequence; identical to SEQ ID NO: 233
  Description of Artificial Sequence: Synthetic polypeptide
  cl_LACBABABA_2_110; 8 4 LC humanized 2049; 8 4 LC humanized 2033

SEQ ID NO: 246 - protein, 110 aa, Artificial Sequence; identical to SEQ ID NO: 234
  Description of Artificial Sequence: Synthetic polypeptide
  cl_NACBABABA_2_110; 8 4 LC humanized 1360; 8 4 LC humanized 1344

SEQ ID NO: 247 - protein, 110 aa, Artificial Sequence
  Description of Artificial Sequence: Synthetic polypeptide
  cl_QACBABABA_1_110; 8 4 LC humanized 777
AYDMTQSPSSLSASVGDRVTITCQASQSISTALAWYQQKPGKAPKLLIYRASTLASGVPSRFSGSGSGTDFTFTISSLQPEDIATYYCQQGWSTVNVDNVFGGGTEVVVR

SEQ ID NO: 248 - protein, 110 aa, Artificial Sequence
  Description of Artificial Sequence: Synthetic polypeptide
  cl_VACBABABA_1_110; 8 4 LC humanized 565
AYDMTQSPSSLSASVGDRVTITCQASQSISTALAWYQQKPGKAPKRLIYRASTLASGVPSRFSGSGSGTEFTLTISSLQPEDFATYYCQQGWSTVNVDNVFGGGTEVVVR

SEQ ID NO: 249 - protein, 110 aa, Artificial Sequence
  Description of Artificial Sequence: Synthetic polypeptide
  cl_XACBABABA_2_110; 8 4 LC humanized 247; 8 4 LC humanized 231
AYDMTQSPSFLSASVGDRVTITCQASQSISTALAWYQQKPGKAPKLLIYRASTLASGVPSRFSGSGSGTEFTLTISSLQPEDFATYYCQQGWSTVNVDNVFGGGTEVVVR

SEQ ID NO: 250 - protein, 110 aa, Artificial Sequence
  Description of Artificial Sequence: Synthetic polypeptide
  cl_ZACBABABA_2_110; 8 4 LC humanized 141; 8 4 LC humanized 125
AYDMTQSPSSFSASTGDRVTITCQASQSISTALAWYQQKPGKAPKLLIYRASTLASGVPSRFSGSGSGTDFTLTISCLQSEDFATYYCQQGWSTVNVDNVFGGGTEVVVR

SEQ ID NO: 251 - protein, 110 aa, Artificial Sequence; identical to SEQ ID NO: 235
  Description of Artificial Sequence: Synthetic polypeptide
  cl_CECBABABA_1_110; 8 4 LC humanized 2207

SEQ ID NO: 252 - protein, 110 aa, Artificial Sequence; identical to SEQ ID NO: 232
  Description of Artificial Sequence: Synthetic polypeptide
  cl_GECBABABA_1_110; 8 4 LC humanized 988

SEQ ID NO: 253 - protein, 110 aa, Artificial Sequence
  Description of Artificial Sequence: Synthetic polypeptide
  cl_PECBABABA_1_110; 8 4 LC humanized 670
AYDMTQSPSSLSASVGDRVTITCQASQSISTALAWYQQKPGKVPKLLIYRASTLASGVPSRFSGSGSGTDFTLTISSLQPEDVATYYCQQGWSTVNVDNVFGGGTEVVVR

SEQ ID NO: 254 - protein, 110 aa, Artificial Sequence
  Description of Artificial Sequence: Synthetic polypeptide
  cl_ZECBABABA_1_110; 8 4 LC humanized 34
AYDMTQSPSTLSASVGDRVTITCQASQSISTALAWYQQKPGKAPKLLIYRASTLASGVPSRFSGSGSGTEFTLTISSLQPDDFATYYCQQGWSTVNVDNVFGGGTEVVVR

SEQ ID NO: 255 - protein, 110 aa, Artificial Sequence; identical to SEQ ID NO: 236
  Description of Artificial Sequence: Synthetic polypeptide
  cl_DICBABABA_15_110; 8 4 LC humanized 2263; 8 4 LC humanized 2262; 8 4 LC humanized 2258; 8 4 LC humanized 2257; 8 4 LC humanized 2256

SEQ ID NO: 256 - protein, 115 aa, Artificial Sequence
  Description of Artificial Sequence: Synthetic polypeptide
  cl_CABBABABA_1_115; 16 6 HC humanized 586
VQLQESGGGVVQPGTSLRLSCVVSGSDISSYHMGWVRQAPGKGLEWLAIIVSSGSAYYATWAKGRFTVSRSKSTLFLKMNSLRADDTAVYYCARNQYSGYGFSFWGQGTLVTVSS

SEQ ID NO: 257 - protein, 115 aa, Artificial Sequence
  Description of Artificial Sequence: Synthetic polypeptide
  cl_DABBABABA_2_115; 16 6 HC humanized 411; 16 6 HC humanized 213
LQLQESGPRLVKPSETLSLTCTVSGSDISSYHMGWIRQPPGKGLEWIGIIVSSGSAYYATWAKSRLTISTSKNQFSLRLSSVTAADSAVYYCARNQYSGYGFSFWGQGTLVTVSS

SEQ ID NO: 258 - protein, 115 aa, Artificial Sequence
  Description of Artificial Sequence: Synthetic polypeptide
  cl_FABBABABA_1_115; 16 6 HC humanized 372
VQLVESGGGLVQPGGSLRLSCAASGSDISSYHMGWVRQAPGKGLEAVAIIVSSGSAYYATWAKGRFTISRDSSTLFLQLNSLRVEDSGIYYCAKNQYSGYGFSFWGQGTLVTVSS

SEQ ID NO: 259 - protein, 115 aa, Artificial Sequence
  Description of Artificial Sequence: Synthetic polypeptide
  cl_GABBABABA_7_115; 16 6 HC humanized 1996; 16 6 HC humanized 230; 16 6 HC humanized 2056; 16 6 HC humanized 672; 16 6 HC humanized 657
QSLEESGGRLVTPGGSLRLSCAASGSDISSYHMGWVRQAPGKGLEWVSIIVSSGSAYYATWAKGRFTISRDNSTLYLQMNSLRAEDTAVYYCARNQYSGYGFSFWGQGTLVTVSS

SEQ ID NO: 260 - protein, 115 aa, Artificial Sequence
  Description of Artificial Sequence: Synthetic polypeptide
  cl_HABBABABA_2_115; 16 6 HC humanized 1907; 16 6 HC humanized 716
QSLLESGGGWVQPGRSLRLSCSASGSDISSYHMGWVRQAPGKGLEWVGIIVSSGSAYYATWAKGRFTISRDNNSLYLQMNSLRPEDTALYYCAKNQYSGYGFSFWGQGVLVTVSS

SEQ ID NO: 261 - protein, 115 aa, Artificial Sequence
  Description of Artificial Sequence: Synthetic polypeptide
  cl_LABBABABA_3_115; 16 6 HC humanized 1945; 16 6 HC humanized 1451; 16 6 HC humanized 65
QSLEESGGGLVKPGESLRLSCAASGSDISSYHMGWVRQAPGKGLEWVGIIVSSGSAYYATWAKGRFTISRDDSTVYLEMNSLKTEDTAVYYCATNQYSGYGFSFWGQGTLVTVSS

SEQ ID NO: 262 - protein, 115 aa, Artificial Sequence
  Description of Artificial Sequence: Synthetic polypeptide
  cl_NABBABABA_1_115; 16 6 HC humanized 1004
QSLLESGPRLVKPSETLSLTCSVSGSDISSYHMGWVRQPPGQGLEWIGIIVSSGSAYYATWARSRVSISTSQNQVSLKLTSVTAADTAVYYCARNQYSGYGFSFWGQGILVTVSS

SEQ ID NO: 263 - protein, 115 aa, Artificial Sequence
  Description of Artificial Sequence: Synthetic polypeptide
  cl_PABBABABA_13_115; 16 6 HC humanized 1971; 16 6 HC humanized 305; 16 6 HC humanized 1877; 16 6 HC humanized 860; 16 6 HC humanized 283
VQLVESGGGVVQPGRSLRLSCAASGSDISSYHMGWVRQAPGKGLEWVAIIVSSGSAYYATWAKGRFTISRDNSTLYLQMNSLRAEDTAVYYCAKNQYSGYGFSFWGQGTLVTVSS

SEQ ID NO: 264 - protein, 115 aa, Artificial Sequence
  Description of Artificial Sequence: Synthetic polypeptide
  cl_QABBABABA_22_115; 16 6 HC humanized 802; 16 6 HC humanized 587; 16 6 HC humanized 1012; 16 6 HC humanized 988; 16 6 HC humanized 129
VQLVESGGGLVQPGGSLRLSCAASGSDISSYHMGWVRQAPGKGLEWVSIIVSSGSAYYATWAKGRFTISRDNSTLYLQMNSLRAEDTAVYYCARNQYSGYGFSFWGQGTLVTVSS

SEQ ID NO: 265 - protein, 115 aa, Artificial Sequence
  Description of Artificial Sequence: Synthetic polypeptide
  cl_RABBABABA_1_115; 16 6 HC humanized 609
VQLVESGGGLVQPGGSLRLSCTTSGSDISSYHMGWVRQVPGKGLEWVSIIVSSGSAYYATWAKGRFTISRDNSTSYLQMTSLTPEDTAVYYCAKNQYSGYGFSFWGQGTVVSVSS

SEQ ID NO: 266 - protein, 115 aa, Artificial Sequence
  Description of Artificial Sequence: Synthetic polypeptide
  cl_YABBABABA_4_115; 16 6 HC humanized 910; 16 6 HC humanized 218; 16 6 HC humanized 912; 16 6 HC humanized 917
VQLQESGPGLVKPSQTLSLTCTVSGSDISSYHMGWIRQPPGKGLEWIGIIVSSGSAYYATWAKSRVTISTSKNQLSLKLTSVTAADTAVYYCARNQYSGYGFSFWGQGTTVTVSS

SEQ ID NO: 267 - protein, 115 aa, Artificial Sequence
  Description of Artificial Sequence: Synthetic polypeptide
  cl_GEBBABABA_1_115; 16 6 HC humanized 136
VQLQQSGPGLVKTSETLPLTCTVSGSDISSYHMGWIRQPPGKGLEYIGIIVSSGSAYYATWAKNRVTISTSKNQFSLKLSSVTAADTALYYCARNQYSGYGFSFWGQGTLVTVSS

SEQ ID NO: 268 - protein, 115 aa, Artificial Sequence
  Description of Artificial Sequence: Synthetic polypeptide
  cl_KEBBABABA_1_115; 16 6 HC humanized 109
VQLVESGPGLVKPSQTLSLTCTVSGSDISSYHMGWIRQPPGKGLEYIGIIVSSGSAYYATWAKSRLTMSVDTSNYQLKLSSVTAADTAVYYCARNQYSGYGFSFWGQGTTVTVSS

SEQ ID NO: 269 - protein, 115 aa, Artificial Sequence
  Description of Artificial Sequence: Synthetic polypeptide
  cl_LEBBABABA_1_115; 16 6 HC humanized 103
VQLQQSGPGLVKPSGTLSLTCDVSGSDISSYHMGWVRQPPGKGLEWIGIIVSSGSAYYATWAKSRVTISKSKNQFSLRLTSVTAADTAVYYCARNQYSGYGFSFWGQGTLVTVSS

SEQ ID NO: 270 - protein, 115 aa, Artificial Sequence
  Description of Artificial Sequence: Synthetic polypeptide
  cl_NEBBABABA_6_115; 16 6 HC humanized 902; 16 6 HC humanized 1982; 16 6 HC humanized 734; 16 6 HC humanized 920; 16 6 HC humanized 149
VQLVESGPGLVKPSQTLSLTCTVSGSDISSYHMGWIRQPPGKGLEWIGIIVSSGSAYYATWAKSRVTISTSKNQFSLKLSSVTAADTAVYYCARNQYSGYGFSFWGQGTLVTVSS

SEQ ID NO: 271 - protein, 115 aa, Artificial Sequence
  Description of Artificial Sequence: Synthetic polypeptide
  cl_PEBBABABA_1_115; 16 6 HC humanized 851
VQLVQSGGGVVQPGGSLRVSCAASGSDISSYHMGWVRQAPGKGLEWMAIIVSSGSAYYATWAKGRFTISRDNSTVSLQMSSLRAEDTAVYYCAKNQYSGYGFSFWGRGTLVTVSS

SEQ ID NO: 272 - protein, 115 aa, Artificial Sequence
  Description of Artificial Sequence: Synthetic polypeptide
  cl_SEBBABABA_1_115; 16 6 HC humanized 926
VQLVESGPGLVKPSQTLSLTCTVSGSDISSYHMGWIRQHSGKTLEWIGIIVSSGSAYYATWAESRVTISADTSKISLKLSSVTAADTAVYYCARNQYSGYGFSFWGQGTTVTVSS

SEQ ID NO: 273 - protein, 115 aa, Artificial Sequence
  Description of Artificial Sequence: Synthetic polypeptide
  cl_VEBBABABA_1_115; 16 6 HC humanized 904
VQLVESGPGLVKPSQTLSLTCNVSGSDISSYHMGWIRQSPGKGLEWIGIIVSSGSAYYATWARSRVTISADTSKVSLELSPMTAADTAVYYCARNQYSGYGFSFWGQGTTVTVSS

SEQ ID NO: 274 - protein, 115 aa, Artificial Sequence
  Description of Artificial Sequence: Synthetic polypeptide
  cl_WEBBABABA_1_115; 16 6 HC humanized 903
VQLQESGPGLVKPSQTLSLTCTVSGSDISSYHMGWIRQPPGTGLEWIGIIVSSGSAYYATWAKSRVTISGDTSKFSLMLRSVTAADTAVYYCARNQYSGYGFSFWGQGTMVTVSS

SEQ ID NO: 275 - protein, 115 aa, Artificial Sequence
  Description of Artificial Sequence: Synthetic polypeptide
  cl_YEBBABABA_1_115; 16 6 HC humanized 946
VQLVESGGGLIKPGGSLRLSCEVPGSDISSYHMGWVRQGPGRGLEWVGIIVSSGSAYYATWARGRFTISRSKSTVYLEMNALKTEDTGIYYCVTNQYSGYGFSFWGQGTMVTVSS

SEQ ID NO: 276 - protein, 115 aa, Artificial Sequence
  Description of Artificial Sequence: Synthetic polypeptide
  cl_ZEBBABABA_1_115; 16 6 HC humanized 882
QSLEESGGGLVQPGGSLRLSCAASGSDISSYHMGWVRQPPGKGLEWVGIIVSSGSAYYATWAKGRFTISRSKSTVYLQMNSLKTEDTAVYYCTANQYSGYGFSFWGQGMLVTVSS

SEQ ID NO: 277 - protein, 115 aa, Artificial Sequence
  Description of Artificial Sequence: Synthetic polypeptide
  cl_CIBBABABA_1_115; 16 6 HC humanized 2041
QSLVQSGTEVRKPGASVKVSCKASGSDISSYHMGWVRQAPGQGLEWMGIIVSSGSAYYATWAQGRVTMSDTSTTVYMELSSLTSEDTAIYYCARNQYSGYGFSFWGPGTLVTVSS

SEQ ID NO: 278 - protein, 115 aa, Artificial Sequence
  Description of Artificial Sequence: Synthetic polypeptide
  cl_KIBBABABA_1_115; 16 6 HC humanized 1944
QSLEESGGRLVTPGTPLTLTCTVSGSDISSYHMGWVRQPPGKGLEWIGIIVSSGSAYYATWAKNRVTISTSKNQFSLRLNSVTAADTAVYYCARNQYSGYGFSFWGQGTLVTVSS

SEQ ID NO: 279 - protein, 115 aa, Artificial Sequence
  Description of Artificial Sequence: Synthetic polypeptide
  cl_LIBBABABA_4_115; 16 6 HC humanized 1895; 16 6 HC humanized 1992; 16 6 HC humanized 1995; 16 6 HC humanized 1949
QSLEESGGRLVTPGTPLTLTCTVSGSDISSYHMGWVRQAPGKGLVWVSIIVSSGSAYYATWAKGRFTISRDNATLYLQMNSLRAEDTAVYYCARNQYSGYGFSFWGPGTLVTVSS

SEQ ID NO: 280 - protein, 115 aa, Artificial Sequence
  Description of Artificial Sequence: Synthetic polypeptide
  cl_SIBBABABA_2_115; 16 6 HC humanized 993; 16 6 HC humanized 994
VQLVESGGGLIQPGRPLRLSCSGSGSDISSYHMGWVRQAPGKGLEWVGIIVSSGSAYYATWAKGRFTISRDDSVVHLQMNSLRSEDTAVYYCTRNQYSGYGFSFWGQGTMVTVSS

SEQ ID NO: 281 - protein, 115 aa, Artificial Sequence
  Description of Artificial Sequence: Synthetic polypeptide
  cl_TIBBABABA_2_115; 16 6 HC humanized 956; 16 6 HC humanized 965
VQLQESGPGLVKPSQTLSLTCTVSGSDISSYHMGWIRQHPGKGLEWIGIIVSSGSAYYATWAESRLTISADTSNIQLRLSSVTAADTAVYFCARNQYSGYGFSFWGQGTTVTVSS

SEQ ID NO: 282 - protein, 115 aa, Artificial Sequence
  Description of Artificial Sequence: Synthetic polypeptide
  cl_WIBBABABA_1_115; 16 6 HC humanized 278
VQLVQSGGGLVKPGGSLRLSCEASGSDISSYHMGWIRQAPGKGLEWVGIIVSSGSAYYATWAKGRFTISRDDSTLYLQVNSLKTEDSAVYYCTTNQYSGYGFSFWGQGTLVTVSS

SEQ ID NO: 283 - protein, 115 aa, Artificial Sequence
  Description of Artificial Sequence: Synthetic polypeptide
  cl_GOBBABABA_1_115; 16 6 HC humanized 1894
QSLEESGGRLVTPGTPLTLTCTVSGSDISSYHMGWVRQAPGKGLEWVSIIVSSGSAYYATWAKGRFTISRDNASLYLQMNSLRAEDTAVYYCARNQYSGYGFSFFSDYWLVTVSS

SEQ ID NO: 284 - protein, 115 aa, Artificial Sequence
  Description of Artificial Sequence: Synthetic polypeptide
  cl_MOBBABABA_3_115; 16 6 HC humanized 1917; 16 6 HC humanized 677; 16 6 HC humanized 267
QSLEESGGGVVQPGRSLRLSCAASGSDISSYHMGWVRQAPGKGLEWVAIIVSSGSAYYATWAKRRFTISRDNSTLYLQMNSLRAEDTAVYYCARNQYSGYGFSFWGQGTLVTVSS

SEQ ID NO: 285 - protein, 115 aa, Artificial Sequence
  Description of Artificial Sequence: Synthetic polypeptide
  cl_POBBABABA_1_115; 16 6 HC humanized 2038
QSLEESGGRLVTPGTPLTLTCTVSGSDISSYHMGWVRQAPGKGLEWVAIIVSSGSAYYATWAKGRFTISRDNASLYLQMNSLRAEDTAVYYCARNQYSGYGFSFPTSGYYYMDVS

SEQ ID NO: 286 - protein, 115 aa, Artificial Sequence
  Description of Artificial Sequence: Synthetic polypeptide
  cl_QOBBABABA_1_115; 16 6 HC humanized 23
QSLLESGGDLVQPGGSLRLSCEASGSDISSYHMGWVRQAPGKGLEWVSIIVSSGSAYYATWAKGRFTISRDKSTLFLQMHSLRVEDTAVYYCAKNQYSGYGFSFWGQGTTVTVSS

SEQ ID NO: 287 - protein, 115 aa, Artificial Sequence
  Description of Artificial Sequence: Synthetic polypeptide
  cl_VOBBABABA_1_115; 16 6 HC humanized 1013
VQLVQSGGGVVQPGRSLRLSCEVSGSDISSYHMGWVRQAPGKGLEWVAIIVSSGSAYYATWAKGRFTISRSNNTLYLQMNSLTAEDTALYFCARNQYSGYGFSFWGKGTTVTVSS

SEQ ID NO: 288 - protein, 115 aa, Artificial Sequence
  Description of Artificial Sequence: Synthetic polypeptide
  cl_YOBBABABA_1_115; 16 6 HC humanized 113
LQLQESGPGLVKPSQTLSLTCSVSGSDISSYHMGWIRQHPGKGLEWIGIIVSSGSAYYATWAKSRITISTSKNQFSLKLTSVTAADTALYYCARNQYSGYGFSFWGRGTLVTVSS

SEQ ID NO: 289 - protein, 115 aa, Artificial Sequence
  Description of Artificial Sequence: Synthetic polypeptide
  cl_HUBBABABA_1_115; 16 6 HC humanized 12
VQLVQSGGGVVQPGGSLRLSCAASGSDISSYHMGWVRQAPGKGLEWVAIIVSSGSAYYATWAQGRVTISRDNSTVHLQITSLKSEDTAVYYCAKNQYSGYGFSFWGQGTLVTVSS

SEQ ID NO: 290 - protein, 115 aa, Artificial Sequence
  Description of Artificial Sequence: Synthetic polypeptide
  cl_LUBBABABA_1_115; 16 6 HC humanized 273
VQLVQSGGGLVQPGGSLRLSCAASGSDISSYHMGWVRQASGKGLEWIGIIVSSGSAYYATWAKGRFTVSRSQNSVFLQMNSLETEDTAVYYCARNQYSGYGFSFWGQGTLVTVSS

SEQ ID NO: 291 - protein, 115 aa, Artificial Sequence
  Description of Artificial Sequence: Synthetic polypeptide
  cl_NUBBABABA_1_115; 16 6 HC humanized 879
QSLEESGGGLVQPGGSLRLSCTASGSDISSYHMGWVRQAPGKGLEWVSIIVSSGSAYYATWAKGRFTISRDSSTLYLQMNNLRVEDTALYYCAHNQYSGYGFSFWGRGTQVTVSS

SEQ ID NO: 292 - protein, 115 aa, Artificial Sequence
  Description of Artificial Sequence: Synthetic polypeptide
  cl_TUBBABABA_1_115; 16 6 HC humanized 1934
QSLEESGGRLVTPGTPLTLTCTVSGSDISSYHMGWVRQAPGKGLEWVSIIVSSGSAYYATWAKGRFTISRDNASLYLQMNSLRAEDTAVYYCARNQYSGYGFSFGIFDYWVTVSS

SEQ ID NO: 293 - protein, 115 aa, Artificial Sequence
  Description of Artificial Sequence: Synthetic polypeptide
  cl_VUBBABABA_1_115; 16 6 HC humanized 200
VQLQESGPGLVKPSETLSLTCSVSGSDISSYHMGWIRQPAGKGLEWIGIIVSSGSAYYATWARSRVTMSMSKNHFSLKLRSVTAADTAVYFCARNQYSGYGFSFWGQGTLVTVSS

SEQ ID NO: 294 - protein, 115 aa, Artificial Sequence
  Description of Artificial Sequence: Synthetic polypeptide
  cl_WUBBABABA_1_115; 16 6 HC humanized 1977
QSLEESGGRLVTPGTPLTLTCTVSGSDISSYHMGWVRQAPGKGLEWVAIIVSSGSAYYATWAKGRFTISRSKNTLYLQMNSLRAEDTAVYYCARNQYSGYGFSFTCPYFDYWVSS

SEQ ID NO: 295 - protein, 115 aa, Artificial Sequence
  Description of Artificial Sequence: Synthetic polypeptide
  cl_XUBBABABA_1_115; 16 6 HC humanized 2027
QSLEESGGRLVTPGTPLTLTCTVSGSDISSYHMGWVRQAPGKGLEWVAIIVSSGSAYYATWAEGRFTISRDNSTLYLQMYSLRTEDTAVYYCARNQYSGYGFSFYYYGMGVWVSS

SEQ ID NO: 296 - protein, 115 aa, Artificial Sequence
  Description of Artificial Sequence: Synthetic polypeptide
  cl_YUBBABABA_1_115; 16 6 HC humanized 1958
VHLVESGGGVVQPGRSLRLSCAASGSDISSYHMGWVRQAPGKGLEWVAIIVSSGSAYYATWAEGRFTISRDNSKLYLQMNSLRAEDSATYYCARNQYSGYGFSFFGPPYYYYYMS

SEQ ID NO: 297 - protein, 115 aa, Artificial Sequence
  Description of Artificial Sequence: Synthetic polypeptide
  cl_BACBABABA_1_115; 16 6 HC humanized 1905
QSLEESGGRLVTPGTPLTLTCTVSGSDISSYHMGWVRQAPGKGLEWVSIIVSSGSAYYATWAKGRFTISRDNSTLYLQMNSLRAEDTALYYCARNQYSGYGFSFVRGGYFYHMDS

SEQ ID NO: 298 - protein, 110 aa, Artificial Sequence
  Description of Artificial Sequence: Synthetic polypeptide
  cl_CACBABABA_1_110; 16 6 LC humanized 586
IVLTQTPSSLSASVGDRITITCQSSHSVYYGDWLAWYQQKPGKAPKLLIYRASNLASGVPSRFSGSRSGTDFTFTISSLRPEDIATYYCLGGYDDDGETAFGGGTKVEIK

SEQ ID NO: 299 - protein, 110 aa, Artificial Sequence
  Description of Artificial Sequence: Synthetic polypeptide
  cl_DACBABABA_27_110; 16 6 LC humanized 411; 16 6 LC humanized 1004; 16 6 LC humanized 587; 16 6 LC humanized 305; 16 6 LC humanized 988
IVLTQSPSSLSASVGDRVTITCQSSHSVYYGDWLAWYQQKPGKAPKLLIYRASNLASGVPSRFSGSGSGTDFTLTISSLQPEDFATYYCLGGYDDDGETAFGGGTKVEIK

SEQ ID NO: 300 - protein, 110 aa, Artificial Sequence
  Description of Artificial Sequence: Synthetic polypeptide
  cl_FACBABABA_15_110; 16 6 LC humanized 372; 16 6 LC humanized 1877; 16 6 LC humanized 1012; 16 6 LC humanized 860; 16 6 LC humanized 283
IQLTQSPSSLSASVGDRVTITCQSSHSVYYGDWLAWYQQKPGKAPKLLIYRASNLASGVPSRFSGSGSGTEFTLTISSLQPDDFATYYCLGGYDDDGETAFGQGTKVEIK

SEQ ID NO: 301 - protein, 110 aa, Artificial Sequence
  Description of Artificial Sequence: Synthetic polypeptide
  cl_GACBABABA_1_110; 16 6 LC humanized 1996
VVLTQTPSPVSTAVGGTVTLSCQSSHSVYYGDWLAWYQQKPGQAPRLLIYRASNLASGIPDRFSGSGSGTDFTLTISRLEPEDFAVYYCLGGYDDDGETAKGPGTEVVVK

SEQ ID NO: 302 - protein, 110 aa, Artificial Sequence
  Description of Artificial Sequence: Synthetic polypeptide
  cl_HACBABABA_2_110; 16 6 LC humanized 1907; 16 6 LC humanized 716
LVMTQSPSSLSASEGDRVTITCQSSHSVYYGDWLAWYQQKPGRAPKLLIHRASNLASGVPSRFSGSGSGTEFTLTISGLQSEDFATYYCLGGYDDDGETAFGGGTTVDVK

SEQ ID NO: 303 - protein, 110 aa, Artificial Sequence
  Description of Artificial Sequence: Synthetic polypeptide
  cl_LACBABABA_2_110; 16 6 LC humanized 1945; 16 6 LC humanized 1451
VELTQPPSPVSAAPGQKVTISCQSSHSVYYGDWLAWYQQLPGTAPKLLIYRASNLASGIPDRFSGSKSGTSATLGITGLQTGDEADYYCLGGYDDDGETAFGGGTRLTVL

SEQ ID NO: 304 - protein, 110 aa, Artificial Sequence
  Description of Artificial Sequence: Synthetic polypeptide
  cl_PACBABABA_10_110; 16 6 LC humanized 1971; 16 6 LC humanized 2041; 16 6 LC humanized 2038; 16 6 LC humanized 2008; 16 6 LC humanized 1992
VVLTQTPSPVSTAVGGTVTITCQSSHSVYYGDWLAWYQQKPGKAPKLLIYRASNLASGVPSRFSGSGSGTDFTLTISSLQPEDFATYYCLGGYDDDGETAFGGGTEVVVK

SEQ ID NO: 305 - protein, 110 aa, Artificial Sequence
  Description of Artificial Sequence: Synthetic polypeptide
  cl_QACBABABA_5_110; 16 6 LC humanized 802; 16 6 LC humanized 609; 16 6 LC humanized 851; 16 6 LC humanized 908; 16 6 LC humanized 108
VVMTQSPSSLSASVGDRVTITCQSSHSVYYGDWLAWYQQKPGKAPKLLIYRASNLASGVPSRFSGSGSGTDFTLTISSLQPEDFATYYCLGGYDDDGETAFGGGTKVEIK

SEQ ID NO: 306 - protein, 110 aa, Artificial Sequence
  Description of Artificial Sequence: Synthetic polypeptide
  cl_CECBABABA_7_110; 16 6 LC humanized 253; 16 6 LC humanized 103; 16 6 LC humanized 882; 16 6 LC humanized 1982; 16 6 LC humanized 734
IVLTQSPSSLSASVGDRVTITCQSSHSVYYGDWLAWYQQKPGKAPKLLIYRASNLASGVPSRFSGSGSGTEFTLTISSLQPEDSATYYCLGGYDDDGETAFGQGTKVEIK

SEQ ID NO: 307 - protein, 110 aa, Artificial Sequence
  Description of Artificial Sequence: Synthetic polypeptide
  cl_KECBABABA_2_110; 16 6 LC humanized 109; 16 6 LC humanized 334
IQLTQSPSFVSASVGDRITITCQSSHSVYYGDWLAWYQQKPGKAPKLLIYRASNLASGVPSRFSGSRSGTDFTLTISSLQPEDFATYYCLGGYDDDGETAFGQGTKVEIK

SEQ ID NO: 308 - protein, 110 aa, Artificial Sequence
  Description of Artificial Sequence: Synthetic polypeptide
  cl_RECBABABA_2_110; 16 6 LC humanized 17; 16 6 LC humanized 21
IQLTQSPSSLSAAVGDRVTIACQSSHSVYYGDWLAWYQQKPGKAPKLLIYRASNLASGVPSRFSGSGSGTDFTLSISSLQPEDFATYYCLGGYDDDGETAFGGGTKVQMK

SEQ ID NO: 309 - protein, 110 aa, Artificial Sequence
  Description of Artificial Sequence: Synthetic polypeptide
  cl_DICBABABA_1_110; 16 6 LC humanized 202
IRMTQSPSSLSASVGDRVTITCQSSHSVYYGDWLAWYQQKPGKVPKLLIYRASNLASGVPSRFSGSGSGTDFTLTISSLQPEDVATYYCLGGYDDDGETAFGPGTKVVVK

SEQ ID NO: 310 - protein, 110 aa, Artificial Sequence
  Description of Artificial Sequence: Synthetic polypeptide
  cl_FICBABABA_14_110; 16 6 LC humanized 192; 16 6 LC humanized 956; 16 6 LC humanized 230; 16 6 LC humanized 880; 16 6 LC humanized 2056
VVLTQSPSSLSASVGDRVTITCQSSHSVYYGDWLAWYQQKPGKAPKLLIYRASNLASGVPSRFSGSGSGTDFTLTISSLQPEDFATYYCLGGYDDDGETAFGQGTKVEIK

SEQ ID NO: 311 - protein, 110 aa, Artificial Sequence
  Description of Artificial Sequence: Synthetic polypeptide
  cl_NICBABABA_2_110; 16 6 LC humanized 1938; 16 6 LC humanized 762
VELTQSPDSLAVSLGERATINCQSSHSVYYGDWLAWYQQKPGQPPKLLIYRASNLASGVPDRFSGSGSGTDFTLTISSLQAEDVAVYYCLGGYDDDGETAFGGGTKVEIK

SEQ ID NO: 312 - protein, 110 aa, Artificial Sequence
  Description of Artificial Sequence: Synthetic polypeptide
  cl_WICBABABA_1_110; 16 6 LC humanized 278
LVLTQSPSSLSASVGDRVTITCQSSHSVYYGDWLAWCQQKPGKSPTLLIYRASNLASGVPSRFSGSGSGTGFTLTISGLQPEDFATYYCLGGYDDDGETAFGGGTKVEIR

SEQ ID NO: 313 - protein, 110 aa, Artificial Sequence
  Description of Artificial Sequence: Synthetic polypeptide
  cl_YICBABABA_1_110; 16 6 LC humanized 169
IVLTQSPSFLSAFVGDRITITCQSSHSVYYGDWLAWYQQKPGKAPKLLIYRASNLASGVPSRFSGSGSGTEFTLTISGLQPEDFASYYCLGGYDDDGETAFGGGTKLEIK

SEQ ID NO: 314 - protein, 110 aa, Artificial Sequence
  Description of Artificial Sequence: Synthetic polypeptide
  cl_GOCBABABA_1_110; 16 6 LC humanized 1894
VVLTQTPSPVSTAVGDRVTITCQSSHSVYYGDWLAWYRQKPGKVPKLLIYRASNLASGVPSRFSGSGSGTDFTLTISSLQPEDVATYYGLGGYDDDGETAFGGGTEVVVK

SEQ ID NO: 315 - protein, 110 aa, Artificial Sequence
  Description of Artificial Sequence: Synthetic polypeptide
  cl_LOCBABABA_1_110; 16 6 LC humanized 657
VVLTQTPSPVSTSVGDRVSITCQSSHSVYYGDWLAWYQQKPGKAPKLLIYRASNLASGVPSRFSGSGSGTDFTLTITSLQPVDFATYYCLGGYDDDGETAFGPGTTVDAK

SEQ ID NO: 316 - protein, 110 aa, Artificial Sequence
  Description of Artificial Sequence: Synthetic polypeptide
  cl_YOCBABABA_1_110; 16 6 LC humanized 113
IVLTQSPSSVSASVGDRVTITCQSSHSVYYGDWLAWYQLKPGKAPKLLINRASNLASGVPSRFSGSGSGTDFTLTISGLQPEDFATYYCLGGYDDDGETAFGPGTTVDIK

SEQ ID NO: 317 - protein, 110 aa, Artificial Sequence
  Description of Artificial Sequence: Synthetic polypeptide
  cl_MUCBABABA_3_110; 16 6 LC humanized 2032; 16 6 LC humanized 200; 16 6 LC humanized 1905
VVLTQTPSPVSTAVGGTGTINCQSSHSVYYGDWLAWYQQKPGQPPKLLIYRASNLASGVPDRFSGSGSGTDFTLTISSLQAEDVAVYYCLGGYDDDGETAFGGGTKVVVK

SEQ ID NO: 318 - protein, 110 aa, Artificial Sequence
  Description of Artificial Sequence: Synthetic polypeptide
  cl_RUCBABABA_1_110; 16 6 LC humanized 1995
  MOD_RES (45)..(45): Any amino acid
VVLTQTPSPVSTAVGGTVTINCQSSHSVYYGDWLAWYQQKPGQPXKLLIYRASNLASGVPDRFSGSGSGTDFTLTISSLQAEDVAVYYCLGGYDDDGETAFGQGTEVVVK

SEQ ID NO: 319 - protein, 115 aa, Artificial Sequence; identical to SEQ ID NO: 256
  Description of Artificial Sequence: Synthetic polypeptide
  cl_CABBABABA_1_115; 16 6 HC humanized 586

SEQ ID NO: 320 - protein, 115 aa, Artificial Sequence
  Description of Artificial Sequence: Synthetic polypeptide
  cl_DABBABABA_1_115; 16 6 HC humanized 411
LQLQESGPRLVKPSETLSLTCTVSGSDISSYHMGWIRQSPGKGLEWIGIIVSSGSAYYATWAKSRLTMSTSKNQFSLRLSSVTAADSAVYYCARNQYSGYGFSFWGQGTLVTVSS

SEQ ID NO: 321 - protein, 115 aa, Artificial Sequence; identical to SEQ ID NO: 258
  Description of Artificial Sequence: Synthetic polypeptide
  cl_FABBABABA_1_115; 16 6 HC humanized 372

SEQ ID NO: 322 - protein, 115 aa, Artificial Sequence
  Description of Artificial Sequence: Synthetic polypeptide
  cl_GABBABABA_1_115; 16 6 HC humanized 1996
QSLEESGGRLVTPGGSLRLSCAASGSDISSYHMGWVRQAPGKGLEWVGIIVSSGSAYYATWAKGRFTISRDNSTLYLQMNSLRVEDTARYYCARNQYSGYGFSFWGQGTLVTVSS

SEQ ID NO: 323 - protein, 115 aa, Artificial Sequence; identical to SEQ ID NO: 260
  Description of Artificial Sequence: Synthetic polypeptide
  cl_HABBABABA_2_115; 16 6 HC humanized 1907; 16 6 HC humanized 716

SEQ ID NO: 324 - protein, 115 aa, Artificial Sequence; identical to SEQ ID NO: 261
  Description of Artificial Sequence: Synthetic polypeptide
  cl_LABBABABA_2_115; 16 6 HC humanized 1945; 16 6 HC humanized 1451

SEQ ID NO: 325 - protein, 115 aa, Artificial Sequence; identical to SEQ ID NO: 262
  Description of Artificial Sequence: Synthetic polypeptide
  cl_NABBABABA_1_115; 16 6 HC humanized 1004

SEQ ID NO: 326 - protein, 115 aa, Artificial Sequence
  Description of Artificial Sequence: Synthetic polypeptide
  cl_PABBABABA_1_115; 16 6 HC humanized 1971
VQLVESGGGVVQPGRSLRLSCAASGSDISSYHMGWVRQAPGKGLEWLAIIVSSGSAYYATWAKGRFTISRDNSSLYLQLSSLRNEDTAVYYCAKNQYSGYGFSFWGPGTLVTVSS

SEQ ID NO: 327 - protein, 115 aa, Artificial Sequence
  Description of Artificial Sequence: Synthetic polypeptide
  cl_QABBABABA_2_115; 16 6 HC humanized 802; 16 6 HC humanized 988
VQLVESGGGLIQPGGSLRLSCAASGSDISSYHMGWVRQAPGKGLEWVSIIVSSGSAYYATWAKGRFTISRDNASLYLQMNSLRAEDTAVYYCARNQYSGYGFSFWGQGTLVTVSS

SEQ ID NO: 328 - protein, 115 aa, Artificial Sequence; identical to SEQ ID NO: 265
  Description of Artificial Sequence: Synthetic polypeptide
  cl_RABBABABA_1_115; 16 6 HC humanized 609

SEQ ID NO: 329 - protein, 115 aa, Artificial Sequence
  Description of Artificial Sequence: Synthetic polypeptide
  cl_SABBABABA_1_115; 16 6 HC humanized 587
VQLVESGGGLVKPGGSLRLSCVVSGSDISSYHMGWVRQAPGKGLEWLSIIVSSGSAYYATWAKGRFTISRDNASLFLQMNSLRADDTALYFCARNQYSGYGFSFWGQGTLVTVSS

SEQ ID NO: 330 - protein, 115 aa, Artificial Sequence; identical to SEQ ID NO: 263
  Description of Artificial Sequence: Synthetic polypeptide
  cl_TABBABABA_6_115; 16 6 HC humanized 305; 16 6 HC humanized 283; 16 6 HC humanized 334; 16 6 HC humanized 281; 16 6 HC humanized 339

SEQ ID NO: 331 - protein, 115 aa, Artificial Sequence
  Description of Artificial Sequence: Synthetic polypeptide
  cl_VABBABABA_4_115; 16 6 HC humanized 1877; 16 6 HC humanized 860; 16 6 HC humanized 204; 16 6 HC humanized 818
VQLVESGGGVVQPGRSLRLSCAASGSDISSYHMGWVRQAPGKGLEWVAIIVSSGSAYYATWAKGRFTISRDNSTLYLQMNSLRAEDTAVYYCARNQYSGYGFSFWGQGTLVTVSS

SEQ ID NO: 332 - protein, 115 aa, Artificial Sequence
  Description of Artificial Sequence: Synthetic polypeptide
  cl_WABBABABA_1_115; 16 6 HC humanized 1012
VQLQEWGGGVVQPGRSLRLSCAASGSDISSYHMGWVRQAPGKGLEWVAIIVSSGSAYYATWAKGRFTISRDNSTLYLQMNSLRAEDTAVYYCARNQYSGYGFSFWGQGTLVTVSS

SEQ ID NO: 333 - protein, 115 aa, Artificial Sequence
  Description of Artificial Sequence: Synthetic polypeptide
  cl_YABBABABA_1_115; 16 6 HC humanized 910
VQLQESGPGLVKPSQTLSLTCTVSGSDISSYHMGWIRQPPGKGLEWIGIIVSSGSAYYATWAQSRVLISTSKSQLSLKLTSVTAADTAVYYCARNQYSGYGFSFWGQGTTVTVSS

SEQ ID NO: 334 - protein, 115 aa, Artificial Sequence
  Description of Artificial Sequence: Synthetic polypeptide
  cl_CEBBABABA_1_115; 16 6 HC humanized 253
VQLVESGGGLVQPGRSLRLSCATSGSDISSYHMGWVRQAPGKGLEWVGIIVSSGSAYYATWAKGRFTISRDNASLYLQMSSLRAEDTALYYCAKNQYSGYGFSFWGQGTLVTVSS

SEQ ID NO: 335 - protein, 115 aa, Artificial Sequence
  Description of Artificial Sequence: Synthetic polypeptide
  cl_DEBBABABA_1_115; 16 6 HC humanized 218
VQLQESGPGLVKPSETLSLTCTVSGSDISSYHMGWIRQPPGKGLEWIGIIVSSGSAYYATWAKSRVTISTSKNQFSLKLSSVTAADTAVYYCARNQYSGYGFSFWGQGTTVTVSS

SEQ ID NO: 336 - protein, 115 aa, Artificial Sequence
  Description of Artificial Sequence: Synthetic polypeptide
  cl_FEBBABABA_1_115; 16 6 HC humanized 213
LQLQESGPGLVKPSETLSLTCTVSGSDISSYHMGWIRQPPGKGLEWIGIIVSSGSAYYATWAKSRVTISTSKNQFSLKLSSVTAADTAVYYCASNQYSGYGFSFWGQGTLVTVSS

SEQ ID NO: 337 - protein, 115 aa, Artificial Sequence; identical to SEQ ID NO: 267
  Description of Artificial Sequence: Synthetic polypeptide
  cl_GEBBABABA_1_115; 16 6 HC humanized 136

SEQ ID NO: 338 - protein, 115 aa, Artificial Sequence
  Description of Artificial Sequence: Synthetic polypeptide
  cl_HEBBABABA_1_115; 16 6 HC humanized 129
MQLVESGGGLVQPGRSLRLSCVTSGSDISSYHMGWVRQVPGKGLEWVGIIVSSGSAYYATWAKGRFTISRDNTSLYLQMNSLRPEDTAVYYCAKNQYSGYGFSFWGQGTLVTVSS

SEQ ID NO: 339 - protein, 115 aa, Artificial Sequence; identical to SEQ ID NO: 268
  Description of Artificial Sequence: Synthetic polypeptide
  cl_KEBBABABA_1_115; 16 6 HC humanized 109

SEQ ID NO: 340 - protein, 115 aa, Artificial Sequence; identical to SEQ ID NO: 269
  Description of Artificial Sequence: Synthetic polypeptide
  cl_LEBBABABA_1_115; 16 6 HC humanized 103

SEQ ID NO: 341 - protein, 115 aa, Artificial Sequence
  Description of Artificial Sequence: Synthetic polypeptide
  cl_MEBBABABA_1_115; 16 6 HC humanized 954
VQLVESGGGVVQPGRSLRLSCAASGSDISSYHMGWVRQAPGKGLEWVAIIVSSGSAYYATWAKGRFTISRDNSTLYLQMNSLRAEDTAVYYCAKNQYSGYGFSFWGQGTTVTVSS

SEQ ID NO: 342 - protein, 115 aa, Artificial Sequence
  Description of Artificial Sequence: Synthetic polypeptide
  cl_NEBBABABA_1_115; 16 6 HC humanized 902
VQLVESGPGLVKPSQTLSLTCTVSGSDISSYHMGWLRQPPGRGLEWIGIIVSSGSAYYATWAKSRVTLSTSKNQFSLKLNSVTAADTAVYYCARNQYSGYGFSFWGQGTLVTVSS

SEQ ID NO: 343 - protein, 115 aa, Artificial Sequence; identical to SEQ ID NO: 271
  Description of Artificial Sequence: Synthetic polypeptide
  cl_PEBBABABA_1_115; 16 6 HC humanized 851

SEQ ID NO: 344 - protein, 115 aa, Artificial Sequence
  Description of Artificial Sequence: Synthetic polypeptide
  cl_REBBABABA_1_115; 16 6 HC humanized 17
VQLVESGGGLVQPGGSLRLSCAASGSDISSYHMGWVRQAPGRGLVWVSIIVSSGSAYYATWAKGRFTISRDNATLYLQMNNLRAEDTAVYYCARNQYSGYGFSFWGQGTLVTVSS

SEQ ID NO: 345 - protein, 115 aa, Artificial Sequence; identical to SEQ ID NO: 272
  Description of Artificial Sequence: Synthetic polypeptide
  cl_SEBBABABA_1_115; 16 6 HC humanized 926

SEQ ID NO: 346 - protein, 115 aa, Artificial Sequence
  Description of Artificial Sequence: Synthetic polypeptide
  cl_TEBBABABA_1_115; 16 6 HC humanized 908
VQLVESGGGLVEPGGSLRLSCAASGSDISSYHMGWIRQAPGKGLEWLSIIVSSGSAYYATWAKGRFTISRDNASLYLQMNSLRAEDTAVYYCVRNQYSGYGFSFWGQGTMVTVSS

SEQ ID NO: 347 - protein, 115 aa, Artificial Sequence; identical to SEQ ID NO: 273
  Description of Artificial Sequence: Synthetic polypeptide
  cl_VEBBABABA_1_115; 16 6 HC humanized 904

SEQ ID NO: 348 - protein, 115 aa, Artificial Sequence; identical to SEQ ID NO: 274
  Description of Artificial Sequence: Synthetic polypeptide
  cl_WEBBABABA_1_115; 16 6 HC humanized 903

SEQ ID NO: 349 - protein, 115 aa, Artificial Sequence
  Description of Artificial Sequence: Synthetic polypeptide
  cl_XEBBABABA_1_115; 16 6 HC humanized 108
VQLVESGGGLVKPGGSLRLSCAASGSDISSYHMGWIRQAPGKGLEWVSIIVSSGSAYYATWAKGRFTISRDNASLFLQMNSLRAEDTAVYYCAKNQYSGYGFSFWGQGTLITVSS

SEQ ID NO: 350 - protein, 115 aa, Artificial Sequence; identical to SEQ ID NO: 275
  Description of Artificial Sequence: Synthetic polypeptide
  cl_YEBBABABA_1_115; 16 6 HC humanized 946

SEQ ID NO: 351 - protein, 115 aa, Artificial Sequence; identical to SEQ ID NO: 276
  Description of Artificial Sequence: Synthetic polypeptide
  cl_ZEBBABABA_1_115; 16 6 HC humanized 882

SEQ ID NO: 352 - protein, 115 aa, Artificial Sequence
  Description of Artificial Sequence: Synthetic polypeptide
  cl_BIBBABABA_1_115; 16 6 HC humanized 186
VQLVESGGGVVQPGRSLRLSCAASGSDISSYHMGWVRQAPGKGLESVAIIVSSGSAYYATWAKGRFTISRDNSTLYLQMNSLRAEDTAVYYCARNQYSGYGFSFWGQGTLVTVSS

SEQ ID NO: 353 - protein, 115 aa, Artificial Sequence; identical to SEQ ID NO: 277
  Description of Artificial Sequence: Synthetic polypeptide
  cl_CIBBABABA_1_115; 16 6 HC humanized 2041

SEQ ID NO: 354 - protein, 115 aa, Artificial Sequence
  Description of Artificial Sequence: Synthetic polypeptide
  cl_DIBBABABA_1_115; 16 6 HC humanized 202
VQLQESGEGLVQPGGSLRLSCAASGSDISSYHMGWVRQAPGKGLEYVSIIVSSGSAYYATWAKGRFTISRDNSTLYLQMGSLRAEDMAVYYCARNQYSGYGFSFWGQGTMVTVSS

SEQ ID NO: 355 - protein, 115 aa, Artificial Sequence
  Description of Artificial Sequence: Synthetic polypeptide
  cl_FIBBABABA_2_115; 16 6 HC humanized 192; 16 6 HC humanized 880
QHLEESGGGVVQPGRSLRLSCAASGSDISSYHMGWVRQAPGKGLEWVAIIVSSGSAYYATWAKGRFTISRDNSTLYLQMNSLRAEDTAVYYCARNQYSGYGFSFWGQGTTVTVSS

SEQ ID NO: 356 - protein, 115 aa, Artificial Sequence
  Description of Artificial Sequence: Synthetic polypeptide
  cl_GIBBABABA_2_115; 16 6 HC humanized 1982; 16 6 HC humanized 734
QSLLESGPGLVKPSQTLSLTCTVSGSDISSYHMGWIRQPPGKGLEWIGIIVSSGSAYYATWAKSRVTMSTSKNHFSLRLSSVTAADTAVYYCARNQYSGYGFSFWGQGTLVTVSS

SEQ ID NO: 357 - protein, 115 aa, Artificial Sequence; identical to SEQ ID NO: 278
  Description of Artificial Sequence: Synthetic polypeptide
  cl_KIBBABABA_1_115; 16 6 HC humanized 1944

SEQ ID NO: 358 - protein, 115 aa, Artificial Sequence
  Description of Artificial Sequence: Synthetic polypeptide
  cl_LIBBABABA_1_115; 16 6 HC humanized 1895
QSLEESGGRLVTPGTPLTLTCTVSGSDISSYHMGWVRQAPGKGLVWVSIIVSSGSAYYATWAKGRFTISRDNATLYLQMNSLRAEDTAVYYCARNQYSGYGFSFWGKGTTVTVSS

SEQ ID NO: 359 - protein, 115 aa, Artificial Sequence
  Description of Artificial Sequence: Synthetic polypeptide
  cl_MIBBABABA_1_115; 16 6 HC humanized 65
QSLEESGGGLVQPGRSLRLSCAASGSDISSYHMGWVRQAPGKGLEWVGIIVSSGSAYYATWAKGRFTISRDNASLYLQMNSLRAEDTALYYCAKNQYSGYGFSFWGQGTLVTVSS

SEQ ID NO: 360 - protein, 115 aa, Artificial Sequence
  Description of Artificial Sequence: Synthetic polypeptide
  cl_NIBBABABA_2_115; 16 6 HC humanized 1938; 16 6 HC humanized 762
VKLLESGGGLVQPGGSLRLSCAASGSDISSYHMGWVRQAPGKGLEWVAIIVSSGSAYYATWAKGRFTISRDNSTLYLQMNSLGAEDTAVYYCARNQYSGYGFSFWGQGTLVTVSS

SEQ ID NO: 361 - protein, 115 aa, Artificial Sequence
  Description of Artificial Sequence: Synthetic polypeptide
  cl_QIBBABABA_2_115; 16 6 HC humanized 2031; 16 6 HC humanized 621
VQLVESGGGLVKPGGSLRLSCAASGSDISSYHMGWVRQAPGKGLEWVSIIVSSGSAYYATWAKGRFTISRDNSTLYLQMNNLRAEDTAVYYCARNQYSGYGFSFWGQGTLVTVLS

SEQ ID NO: 362 - protein, 115 aa, Artificial Sequence
  Description of Artificial Sequence: Synthetic polypeptide
  cl_SIBBABABA_1_115; 16 6 HC humanized 993
VQLVESGGGLIQPGRPLRLSCSGSGSDISSYHMGWVRQAPGKGLEWVGIIVSSGSAYYATWAKGRFTISRDDSVVHLQMNSLKSEDTAVYYCTRNQYSGYGFSFWGQGTTVTVSS

SEQ ID NO: 363 - protein, 115 aa, Artificial Sequence
  Description of Artificial Sequence: Synthetic polypeptide
  cl_TIBBABABA_1_115; 16 6 HC humanized 956
VQLQESGPGLVKPSQTLSLTCTVSGSDISSYHMGWFRQHPGKGLEWIGIIVSSGSAYYATWAESRLTISEDTSNIQLRLTSVTAADTAVYFCARNQYSGYGFSFWGQGTTVTVSS

SEQ ID NO: 364 - protein, 115 aa, Artificial Sequence
  Description of Artificial Sequence: Synthetic polypeptide
  cl_VIBBABABA_1_115; 16 6 HC humanized 920
VQLVESGPGLVKPSQTLSLTCTVSGSDISSYHMGWIRQFPGKGLEWIGIIVSSGSAYYATWAKSRFTISTSKNQFSLKVDSVTAADTAVYYCARNQYSGYGFSFWGQGTTVTVSS

SEQ ID NO: 365 - protein, 115 aa, Artificial Sequence; identical to SEQ ID NO: 282
  Description of Artificial Sequence: Synthetic polypeptide
  cl_WIBBABABA_1_115; 16 6 HC humanized 278

SEQ ID NO: 366 - protein, 115 aa, Artificial Sequence
  Description of Artificial Sequence: Synthetic polypeptide
  cl_YIBBABABA_2_115; 16 6 HC humanized 169; 16 6 HC humanized 168
VQLVESGGGLVQPGGSLRLSCAASGSDISSYHMGWVRQAPGKGLEWVSIIVSSGSAYYATWAKGRFTISRDNSTLYLQMDSLRAEDTAIYYCAKNQYSGYGFSFWGQGTLVTVSS

SEQ ID NO: 367 - protein, 115 aa, Artificial Sequence
  Description of Artificial Sequence: Synthetic polypeptide
  cl_ZIBBABABA_1_115; 16 6 HC humanized 994
VQLVESGGGLIQPGRSLRLSCSGSGSDISSYHMGWVRQAPGKGLEWVGIIVSSGSAYYATWAKGRFTISRDDSVVYLQMNSLRSEDTAVYYCTRNQYSGYGFSFWGQGTMVTVSS

SEQ ID NO: 368 - protein, 115 aa, Artificial Sequence
  Description of Artificial Sequence: Synthetic polypeptide
  cl_BOBBABABA_2_115; 16 6 HC humanized 975; 16 6 HC humanized 978
VQLVESGGGVVRPGGSLRLSCAASGSDISSYHMGWVRQAPGKGLEWVGIIVSSGSAYYATWAKGRFTISRDNASLYLEMNSLRAEDTALYFCARNQYSGYGFSFWGQGTMVTVSS

SEQ ID NO: 369 - protein, 115 aa, Artificial Sequence
  Description of Artificial Sequence: Synthetic polypeptide
  cl_DOBBABABA_1_115; 16 6 HC humanized 230
QSLEESGGGLVQPGGSLRLSCAASGSDISSYHMGWVRQAPGKGLEWVSIIVSSGSAYYATWAKGRFTISRDNSTLYLQMNSLRAEDTAVYYCAKNQYSGYGFSFWGQGTTVTVSS

SEQ ID NO: 370 - protein, 115 aa, Artificial Sequence; identical to SEQ ID NO: 283
  Description of Artificial Sequence: Synthetic polypeptide
  cl_GOBBABABA_1_115; 16 6 HC humanized 1894

SEQ ID NO: 371 - protein, 115 aa, Artificial Sequence
  Description of Artificial Sequence: Synthetic polypeptide
  cl_HOBBABABA_2_115; 16 6 HC humanized 2056; 16 6 HC humanized 672
QSLVESGGGLIQPGGSLRLSCAASGSDISSYHMGWVRQAPGKGLEWVSIIVSSGSAYYATWAKGRFTISRDNSTLYLQMNSLRAEDTAVYYCARNQYSGYGFSFWGQGTLVTVSS

SEQ ID NO: 372 - protein, 115 aa, Artificial Sequence
  Description of Artificial Sequence: Synthetic polypeptide
  cl_LOBBABABA_1_115; 16 6 HC humanized 657
QSLEESGGRLVTPGGSLRLSCAASGSDISSYHMGWVRQAPGKGLEWVSIIVSSGSAYYATWAKGRFTISRDNSSLYLQMNSLRTEDSALYYCALNQYSGYGFSFWGQGSLVTVSS

SEQ ID NO: 373 - protein, 115 aa, Artificial Sequence; identical to SEQ ID NO: 284
  Description of Artificial Sequence: Synthetic polypeptide
  cl_MOBBABABA_2_115; 16 6 HC humanized 1917; 16 6 HC humanized 677

SEQ ID NO: 374 - protein, 115 aa, Artificial Sequence; identical to SEQ ID NO: 285
  Description of Artificial Sequence: Synthetic polypeptide
  cl_POBBABABA_1_115; 16 6 HC humanized 2038

SEQ ID NO: 375 - protein, 115 aa, Artificial Sequence; identical to SEQ ID NO: 286
  Description of Artificial Sequence: Synthetic polypeptide
  cl_QOBBABABA_1_115; 16 6 HC humanized 23

SEQ ID NO: 376 - protein, 115 aa, Artificial Sequence
  Description of Artificial Sequence: Synthetic polypeptide
  cl_ROBBABABA_1_115; 16 6 HC humanized 21
VQLVESGGGLVQPGGSLRLSCAASGSDISSYHMGWVRQAPGKGLEFVSIIVSSGSAYYATWAKDRFTISRDNSTVYLQMDSLRTEDTAMYFCARNQYSGYGFSFWGQGTLVTVSS

SEQ ID NO: 377 - protein, 115 aa, Artificial Sequence
  Description of Artificial Sequence: Synthetic polypeptide
  cl_SOBBABABA_1_115; 16 6 HC humanized 469
VQLVESGGGLVQPGGSLRLSCAASGSDISSYHMGWVRQAPGKGLEWVAIIVSSGSAYYATWAKGRFTISRDNTSLFLHMSSLRGEDTAIYYCARNQYSGYGFSFWGQGTLVTVSS

SEQ ID NO: 378 - protein, 115 aa, Artificial Sequence
  Description of Artificial Sequence: Synthetic polypeptide
  cl_TOBBABABA_1_115; 16 6 HC humanized 2008
QSLEESGGRLVTPGTSLRLSCAVSGSDISSYHMGWVRQAPGKGLEWVSIIVSSGSAYYATWAKGRFTISRDNSTVYLQMNSLRAEDTAVFYCARNQYSGYGFSFWGQGTLVTVSS

SEQ ID NO: 379 - protein, 115 aa, Artificial Sequence; identical to SEQ ID NO: 287
  Description of Artificial Sequence: Synthetic polypeptide
  cl_VOBBABABA_1_115; 16 6 HC humanized 1013

SEQ ID NO: 380 - protein, 115 aa, Artificial Sequence
  Description of Artificial Sequence: Synthetic polypeptide
  cl_XOBBABABA_1_115; 16 6 HC humanized 149
VQLVQSGPGLVKPSRTLSLTCTVSGSDISSYHMGWIRQPPGKGLEWIGIIVSSGSAYYATWAQNRLTISTSKNQFSLKLASVTAADTAVYFCARNQYSGYGFSFWGQGTLVTVSS

SEQ ID NO: 381 - protein, 115 aa, Artificial Sequence; identical to SEQ ID NO: 288
  Description of Artificial Sequence: Synthetic polypeptide
  cl_YOBBABABA_1_115; 16 6 HC humanized 113

SEQ ID NO: 382 - protein, 115 aa, Artificial Sequence
  Description of Artificial Sequence: Synthetic polypeptide
  cl_BUBBABABA_1_115; 16 6 HC humanized 965
VQLQESGPGLVKPSQTLSLTCTVSGSDISSYHMGWIRQHPGKGLEWIGIIVSSGSAYYATWAKSRVTISADTSKISLKLSSVTAADTAVYYCARNQYSGYGFSFWGQGTTVTVSS

SEQ ID NO: 383 - protein, 115 aa, Artificial Sequence
  Description of Artificial Sequence: Synthetic polypeptide
  cl_CUBBABABA_1_115; 16 6 HC humanized 912
VQLQESGPGLVKPSQTLSLTCTVSGSDISSYHMGWIRQPPGKGLEWIGIIVSSGSAYYATWAKSRVLISTSKNQVSLKLSSVTAADTAVYYCARNQYSGYGFSFWGQGTTVTVSS

SEQ ID NO: 384 - protein, 115 aa, Artificial Sequence; identical to SEQ ID NO: 289
  Description of Artificial Sequence: Synthetic polypeptide
  cl_HUBBABABA_1_115; 16 6 HC humanized 12

SEQ ID NO: 385 - protein, 115 aa, Artificial Sequence
  Description of Artificial Sequence: Synthetic polypeptide
  cl_KUBBABABA_1_115; 16 6 HC humanized 924
VQLVESGPGLVKPSQTLSLTCTVSGSDISSYHMGWFRQPPGKGLEWIGIIVSSGSAYYATWAKSRVTISTSKNQVSLKLSPVTGADTAVYFCARNQYSGYGFSFWGQGTLVTVSS

SEQ ID NO: 386 - protein, 115 aa, Artificial Sequence; identical to SEQ ID NO: 290
  Description of Artificial Sequence: Synthetic polypeptide
  cl_LUBBABABA_1_115; 16 6 HC humanized 273

SEQ ID NO: 387 - protein, 115 aa, Artificial Sequence
  Description of Artificial Sequence: Synthetic polypeptide
  cl_MUBBABABA_1_115; 16 6 HC humanized 2032
QSLEESGGRLVTPGGSLRLSCAGSGSDISSYHMGWVRQAPGKGLEWVSIIVSSGSAYYATWAEGRFTISRDNATLYLQMNSLRVEDTAVYYCATNQYSGYGFSFWGQGTLVTVSS

SEQ ID NO: 388 - protein, 115 aa, Artificial Sequence; identical to SEQ ID NO: 291
  Description of Artificial Sequence: Synthetic polypeptide
  cl_NUBBABABA_1_115; 16 6 HC humanized 879

SEQ ID NO: 389 - protein, 115 aa, Artificial Sequence
  Description of Artificial Sequence: Synthetic polypeptide
  cl_PUBBABABA_1_115; 16 6 HC humanized 267
QSLEQSGGGLVQPGESLRLSCAGSGSDISSYHMGWVRQAPGKGLEWVAIIVSSGSAYYATWAKGRFTISRDNASLFLQMNSLRVEDTAVYYCARNQYSGYGFSFWGQGTLVTVSS

SEQ ID NO: 390 - protein, 115 aa, Artificial Sequence
  Description of Artificial Sequence: Synthetic polypeptide
  cl_QUBBABABA_1_115; 16 6 HC humanized 1992
QSLEESGGRLVTPGTPLTLTCTVSGSDISSYHMGWVRQAPGKGLVWVSIIVSSGSAYYATWAKGRFTISRDNATLYLQMNSLRVEDTAVYYCARNQYSGYGFSFWGPGTLVTVSS

SEQ ID NO: 391 - protein, 115 aa, Artificial Sequence
  Description of Artificial Sequence: Synthetic polypeptide
  cl_RUBBABABA_1_115; 16 6 HC humanized 1995
QSLEESGGRLVTPGTPLTLTCTVSGSDISSYHMGWVRQAPGKGLEWVSIIVSSGSAYYATWAKGRFTISRDNSTLYLQMNSLRAEDTAVYYCAKNQYSGYGFSFWGPGTLVTVSS

SEQ ID NO: 392 - protein, 115 aa, Artificial Sequence
  Description of Artificial Sequence: Synthetic polypeptide
  cl_SUBBABABA_1_115; 16 6 HC humanized 917
VQLQESGPGLVKPSQTLSLTCTVSGSDISSYHMGWIRQPPGKGLEWIGIIVSSGSAYYATWARSRITISETSKNLSLKLTSVTAADTAVYYCARNQYSGYGFSFWGQGTTVTVSS

SEQ ID NO: 393 - protein, 115 aa, Artificial Sequence; identical to SEQ ID NO: 292
  Description of Artificial Sequence: Synthetic polypeptide
  cl_TUBBABABA_1_115; 16 6 HC humanized 1934

SEQ ID NO: 394 - protein, 115 aa, Artificial Sequence; identical to SEQ ID NO: 293
  Description of Artificial Sequence: Synthetic polypeptide
  cl_VUBBABABA_1_115; 16 6 HC humanized 200

SEQ ID NO: 395 - protein, 115 aa, Artificial Sequence; identical to SEQ ID NO: 294
  Description of Artificial Sequence: Synthetic polypeptide
  cl_WUBBABABA_1_115; 16 6 HC humanized 1977

SEQ ID NO: 396 - protein, 115 aa, Artificial Sequence; identical to SEQ ID NO: 295
  Description of Artificial Sequence: Synthetic polypeptide
  cl_XUBBABABA_1_115; 16 6 HC humanized 2027

SEQ ID NO: 397 - protein, 115 aa, Artificial Sequence; identical to SEQ ID NO: 296
  Description of Artificial Sequence: Synthetic polypeptide
  cl_YUBBABABA_1_115; 16 6 HC humanized 1958

SEQ ID NO: 398 - protein, 115 aa, Artificial Sequence
  Description of Artificial Sequence: Synthetic polypeptide
  cl_ZUBBABABA_1_115; 16 6 HC humanized 1949
QSLEESGGRLVTPGTPLTLTCTVSGSDISSYHMGWVRQAPGKGLEYVSIIVSSGSAYYATWAKGRFTISRDNSTLYLQMSSLRAEDTAVYYCVKNQYSGYGFSFWGPGTLVTVSS

SEQ ID NO: 399 - protein, 115 aa, Artificial Sequence; identical to SEQ ID NO: 297
  Description of Artificial Sequence: Synthetic polypeptide
  cl_BACBABABA_1_115; 16 6 HC humanized 1905

SEQ ID NO: 400 - protein, 110 aa, Artificial Sequence; identical to SEQ ID NO: 298
  Description of Artificial Sequence: Synthetic polypeptide
  cl_CACBABABA_1_110; 16 6 LC humanized 586

SEQ ID NO: 401 - protein, 110 aa, Artificial Sequence
  Description of Artificial Sequence: Synthetic polypeptide
  cl_DACBABABA_1_110; 16 6 LC humanized 411
IVLTQSPSSLSASVGDRVTITCQSSHSVYYGDWLAWYQQKPGKAPNLLIYRASNLASGVPSRFSGSGSATDFTLTISSLQPEDFATYYCLGGYDDDGETAFGGGTRVEIK

SEQ ID NO: 402 - protein, 110 aa, Artificial Sequence
  Description of Artificial Sequence: Synthetic polypeptide
  cl_FACBABABA_1_110; 16 6 LC humanized 372
IQLTQSPSTLSASVGDRVTITCQSSHSVYYGDWLAWYQQKAGKAPTLLIYRASNLASGVPSRFSGSGSGTEFTLTISSLQPDDFATYYCLGGYDDDGETAFGQGTKVDIK

SEQ ID NO: 403 - protein, 110 aa, Artificial Sequence; identical to SEQ ID NO: 301
  Description of Artificial Sequence: Synthetic polypeptide
  cl_GACBABABA_1_110; 16 6 LC humanized 1996

SEQ ID NO: 404 - protein, 110 aa, Artificial Sequence; identical to SEQ ID NO: 302
  Description of Artificial Sequence: Synthetic polypeptide
  cl_HACBABABA_2_110; 16 6 LC humanized 1907; 16 6 LC humanized 716

SEQ ID NO: 405 - protein, 110 aa, Artificial Sequence; identical to SEQ ID NO: 303
  Description of Artificial Sequence: Synthetic polypeptide
  cl_LACBABABA_2_110; 16 6 LC humanized 1945; 16 6 LC humanized 1451

SEQ ID NO: 406 - protein, 110 aa, Artificial Sequence
  Description of Artificial Sequence: Synthetic polypeptide
  cl_NACBABABA_2_110; 16 6 LC humanized 1004; 16 6 LC humanized 283
IQLTQSPSSVSASVGDRVTITCQSSHSVYYGDWLAWYQQKPGKAPKLLIYRASNLASGVPSRFSGSGSGTDFALTISSLQPEDFATYYCLGGYDDDGETAFGQGTRLEIK

SEQ ID NO: 407 - protein, 110 aa, Artificial Sequence
  Description of Artificial Sequence: Synthetic polypeptide
  cl_PACBABABA_1_110; 16 6 LC humanized 1971
VVLTQTPSPVSTAVGGTVTITCQSSHSVYYGDWLAWYQQKSGKAPKLLIYRASNLASGVPSRFSGSGSGTDFTLTISSLQPEDFATYYCLGGYDDDGETAFGGGTEVVVK

SEQ ID NO: 408 - protein, 110 aa, Artificial Sequence
  Description of Artificial Sequence: Synthetic polypeptide
  cl_QACBABABA_1_110; 16 6 LC humanized 802
IRMTQSPSSFSASTGDRVTITCQSSHSVYYGDWLAWYQQKPGKAPKLLIYRASNLASGVPSRFSGSGSGTDFTLTISCLQSEDFATYYCLGGYDDDGETAFGGGTKVEIK

SEQ ID NO: 409 - protein, 110 aa, Artificial Sequence
  Description of Artificial Sequence: Synthetic polypeptide
  cl_RACBABABA_1_110; 16 6 LC humanized 609
IRLTQSPSFLSASVGDRVTITCQSSHSVYYGDWLAWYQQKPGKAPKLLIYRASNLASGVPSRFSGSGSGTDFTLTISTLQPEDFATYYCLGGYDDDGETAFGQGTKLEIK

SEQ ID NO: 410 - protein, 110 aa, Artificial Sequence
  Description of Artificial Sequence: Synthetic polypeptide
  cl_SACBABABA_1_110; 16 6 LC humanized 587
VVMTQSPSSLSASVGDRVTITCQSSHSVYYGDWLAWFQQKPGKAPNLLIYRASNLASGVPSRFSGSGSGTEFTLTISSLQPEDFATYYCLGGYDDDGETAFGQGTKVEIK

SEQ ID NO: 411 - protein, 110 aa, Artificial Sequence
  Description of Artificial Sequence: Synthetic polypeptide
  cl_TACBABABA_1_110; 16 6 LC humanized 305
IQLTQSPSSLSASVGDRVTITCQSSHSVYYGDWLAWFQQKPGKAPKSLIYRASNLASGVPSRFSGSGSGTDFTLTISSLQPEDSATYYCLGGYDDDGETAFGGGTKVEIK

SEQ ID NO: 412 - protein, 110 aa, Artificial Sequence
  Description of Artificial Sequence: Synthetic polypeptide
  cl_VACBABABA_12_110; 16 6 LC humanized 1877; 16 6 LC humanized 860; 16 6 LC humanized 213; 16 6 LC humanized 902; 16 6 LC humanized 334
IQLTQSPSSLSASVGDRVTITCQSSHSVYYGDWLAWYQQKPGKAPKLLIYRASNLASGVPSRFSGSGSGTDFTLTISSLQPEDFATYYCLGGYDDDGETAFGGGTKVEIK

SEQ ID NO: 413 - protein, 110 aa, Artificial Sequence
  Description of Artificial Sequence: Synthetic polypeptide
  cl_WACBABABA_2_110; 16 6 LC humanized 1012; 16 6 LC humanized 65
IQLTQSPSTLSASVGDRVTITCQSSHSVYYGDWLAWYQQKPGKAPKLLIYRASNLASGVPSRFSGSGSGTEFTLTISSLQPDDFATYYCLGGYDDDGETAFGQGTKLEIK

SEQ ID NO: 414 - protein, 110 aa, Artificial Sequence
  Description of Artificial Sequence: Synthetic polypeptide
  cl_XACBABABA_6_110; 16 6 LC humanized 988; 16 6 LC humanized 910; 16 6 LC humanized 956; 16 6 LC humanized 2056; 16 6 LC humanized 672
IVLTQSPSSLSASVGDRVTITCQSSHSVYYGDWLAWYQQKPGKAPKLLIYRASNLASGVPSRFSGSGSGTDFTLTISSLQPEDFATYYCLGGYDDDGETAFGQGTRLEIK

SEQ ID NO: 415 - protein, 110 aa, Artificial Sequence
  Description of Artificial Sequence: Synthetic polypeptide
  cl_CECBABABA_1_110; 16 6 LC humanized 253
IVLTQSPSAMSASVGDRVTITCQSSHSVYYGDWLAWFQQKPGKAPKLLIYRASNLASGVPSRFSGSGSGTEFTLTISSLQPEDSATYYCLGGYDDDGETAFGQGTKVDIK

SEQ ID NO: 416 - protein, 110 aa, Artificial Sequence
  Description of Artificial Sequence: Synthetic polypeptide
  cl_DECBABABA_1_110; 16 6 LC humanized 218
IVMTQSPSSLSASVGDRVTITCQSSHSVYYGDWLAWYQQKPGKVPKLLIYRASNLASGVPSRFSGSGSGTDFTLTISSLQPEDVATYYCLGGYDDDGETAFGPGTKVEIK

SEQ ID NO: 417 - protein, 110 aa, Artificial Sequence
  Description of Artificial Sequence: Synthetic polypeptide
  cl_GECBABABA_1_110; 16 6 LC humanized 136
VVMTQSPSTLSASVGDRVTITCQSSHSVYYGDWLAWYQQKPGKAPKVLIYRASNLASGVPSRFSGSGSGTEFTLTISSLQPDDFASYYCLGGYDDDGETAFGPGTKVDIK

SEQ ID NO: 418 - protein, 110 aa, Artificial Sequence
  Description of Artificial Sequence: Synthetic polypeptide
  cl_HECBABABA_1_110; 16 6 LC humanized 129
IVMTQSPSSLSASVGDRVTITCQSSHSVYYGDWLAWYQHKPGKAPRLLIYRASNLASGVPSRFSGSGSGTDFTLTISSLQPDDFATYYCLGGYDDDGETAFGQGTKVEVK

SEQ ID NO: 419 - protein, 110 aa, Artificial Sequence
  Description of Artificial Sequence: Synthetic polypeptide
  cl_KECBABABA_1_110; 16 6 LC humanized 109
IQLTQSPSSVSASVGDTITITCQSSHSVYYGDWLAWYQQKPGKAPKLLIYRASNLASGVPSRFSGSRSGTDFTLTISSLQPEDFATYYCLGGYDDDGETAFGQGTKVEIK

SEQ ID NO: 420 - protein, 110 aa, Artificial Sequence
  Description of Artificial Sequence: Synthetic polypeptide
  cl_LECBABABA_1_110; 16 6 LC humanized 103
IVLTQSPSTLSASVGDRVTITCQSSHSVYYGDWLAWYQQKPGQAPKLLIYRASNLASGVPSRFSGSGSGTEFTLSINSLQPDDSATYFCLGGYDDDGETAFGQGTKVEIK

SEQ ID NO: 421 - protein, 110 aa, Artificial Sequence
  Description of Artificial Sequence: Synthetic polypeptide
  cl_MECBABABA_1_110; 16 6 LC humanized 954
IVLTQSPSTLSASVGDRVTITCQSSHSVYYGDWLAWYQQKPGKAPKLLIYRASNLASGVPSRFSGSGSGTEFTLTISSLQPDDFATYYCLGGYDDDGETAFGQGTKAEIK

SEQ ID NO: 422 - protein, 110 aa, Artificial Sequence; identical to SEQ ID NO: 305
  Description of Artificial Sequence: Synthetic polypeptide
  cl_PECBABABA_3_110; 16 6 LC humanized 851; 16 6 LC humanized 908; 16 6 LC humanized 912

SEQ ID NO: 423 - protein, 110 aa, Artificial Sequence
  Description of Artificial Sequence: Synthetic polypeptide
  cl_RECBABABA_1_110; 16 6 LC humanized 17
IQLTQSPSSLSAAVGDRVTIACQSSHSVYYGDWLAWYQQKPGKAPKLLIYRASNLASGVPSRFSGSGSGTDFTLSISSLQPGDFATYYCLGGYDDDGETAFGGGTKVQMK

SEQ ID NO: 424 - protein, 110 aa, Artificial Sequence
  Description of Artificial Sequence: Synthetic polypeptide
  cl_XECBABABA_2_110; 16 6 LC humanized 108; 16 6 LC humanized 946
IVLTQSPSSVSASVGDRVTITCQSSHSVYYGDWLAWYQQKPGKAPKLLIYRASNLASGVPSRFSGSGSGTDFTLTISSLQPEDFATYYCLGGYDDDGETAFGGGTKVEIK

SEQ ID NO: 425 - protein, 110 aa, Artificial Sequence
  Description of Artificial Sequence: Synthetic polypeptide
  cl_ZECBABABA_1_110; 16 6 LC humanized 882
VVLTQSPSSLSASVGDRVTITCQSSHSVYYGDWLAWYQQKPGKAPKLLIYRASNLASGVPSRFSGSGFGTDFTFTISSLQPEDSATYYCLGGYDDDGETAFGQGTKLEIK

SEQ ID NO: 426 - protein, 110 aa, Artificial Sequence
  Description of Artificial Sequence: Synthetic polypeptide
  cl_BICBABABA_1_110; 16 6 LC humanized 186
IQLTQSPSTLSASVGDRVTITCQSSHSVYYGDWLAWYQQKPGKAPKLLIYRASNLASGVPSRFSGSGSGTEFTLTISSLQPDDFATYYCLGGYDDDGETAFGQGTKVVVK

SEQ ID NO: 427 - protein, 110 aa, Artificial Sequence
  Description of Artificial Sequence: Synthetic polypeptide
  cl_CICBABABA_1_110; 16 6 LC humanized 2041
VVLTQTPSPVSTAVGGTVTITCQSSHSVYYGDWLAWYQQKPGKAPKLLIYRASNLASGVPSRFSGSGSGTDFTLTISCLQSEDFATYYCLGGYDDDGETAFGGGTEVVVK

SEQ ID NO: 428 - protein, 110 aa, Artificial Sequence; identical to SEQ ID NO: 309
  Description of Artificial Sequence: Synthetic polypeptide
  cl_DICBABABA_1_110; 16 6 LC humanized 202

SEQ ID NO: 429 - protein, 110 aa, Artificial Sequence
  Description of Artificial Sequence: Synthetic polypeptide
  cl_FICBABABA_1_110; 16 6 LC humanized 192
VVMTQSPSSLSASVGDRVTITCQSSHSVYYGDWLAWYQQKPGKAPKLLIYRASNLASGVPSRFSGSGSGTDFTLTISSLQAEDFTTYYCLGGYDDDGETAFGQGTKVEFK

SEQ ID NO: 430 - protein, 110 aa, Artificial Sequence
  Description of Artificial Sequence: Synthetic polypeptide
  cl_GICBABABA_2_110; 16 6 LC humanized 1982; 16 6 LC humanized 734
VELTQSPSSVSASVGDRVTITCQSSHSVYYGDWLAWYQQKPGKAPKLLIYRASNLASGVPSRFSGSGSGTDFSLTISSLQPEDSATYYCLGGYDDDGETAFGQGTKVEIK

SEQ ID NO: 431 - protein, 110 aa, Artificial Sequence
  Description of Artificial Sequence: Synthetic polypeptide
  cl_KICBABABA_2_110; 16 6 LC humanized 1944; 16 6 LC humanized 1895
IELTQSPSTLSASVGDRVIISCQSSHSVYYGDWLAWYQQKPGKAPKLLIYRASNLASGVPSRFSGSGSGTEFSLTINSLQPDDFATYYCLGGYDDDGETAFGPGTKVDIK

SEQ ID NO: 432 - protein, 110 aa, Artificial Sequence; identical to SEQ ID NO: 311
  Description of Artificial Sequence: Synthetic polypeptide
  cl_NICBABABA_2_110; 16 6 LC humanized 1938; 16 6 LC humanized 762

SEQ ID NO: 433 - protein, 110 aa, Artificial Sequence
  Description of Artificial Sequence: Synthetic polypeptide
  cl_QICBABABA_2_110; 16 6 LC humanized 2031; 16 6 LC humanized 621
VELTQSPSSLSASVGDRVTITCQSSHSVYYGDWLAWYQQKPGKAPKLLIYRASNLASGVPSRFSGSGSGTDFTLTISSLQPEDFATYYCLGGYDDDGETAFGQGTKVEIK

SEQ ID NO: 434 - protein, 110 aa, Artificial Sequence
  Description of Artificial Sequence: Synthetic polypeptide
  cl_SICBABABA_4_110; 16 6 LC humanized 993; 16 6 LC humanized 880; 16 6 LC humanized 23; 16 6 LC humanized 917
VVLTQSPSSLSASVGDRVTITCQSSHSVYYGDWLAWYQQKPGKAPKLLIYRASNLASGVPSRFSGSGSGTDFTLTISSLQPEDFATYYCLGGYDDDGETAFGPGTKVDIK

SEQ ID NO: 435 - protein, 110 aa, Artificial Sequence
  Description of Artificial Sequence: Synthetic polypeptide
  cl_VICBABABA_1_110; 16 6 LC humanized 920
IVMTQSPSSLSASVGDRVTITCQSSHSVYYGDWLAWYQQKPGKAPKLLIYRASNLASGVPSRFSGSGSGTDFTLTISSLQPEDIATYYCLGGYDDDGETAFGQGTKVEIK

SEQ ID NO: 436 - protein, 110 aa, Artificial Sequence; identical to SEQ ID NO: 312
  Description of Artificial Sequence: Synthetic polypeptide
  cl_WICBABABA_1_110; 16 6 LC humanized 278

SEQ ID NO: 437 - protein, 110 aa, Artificial Sequence; identical to SEQ ID NO: 313
  Description of Artificial Sequence: Synthetic polypeptide
  cl_YICBABABA_1_110; 16 6 LC humanized 169

SEQ ID NO: 438 - protein, 110 aa, Artificial Sequence
  Description of Artificial Sequence: Synthetic polypeptide
  cl_ZICBABABA_1_110; 16 6 LC humanized 994
IVLTQSPSSLSASVGDRVTITCQSSHSVYYGDWLAWYQQKPGKVPKLLIYRASNLASGVPSRFSGSGSGTDFTLTISSLQPEDVATYYCLGGYDDDGETAFGQGTKVEIK

SEQ ID NO: 439 - protein, 110 aa, Artificial Sequence
  Description of Artificial Sequence: Synthetic polypeptide
  cl_BOCBABABA_1_110; 16 6 LC humanized 975
IVLTQSPSTQSASVGDRVTITCQSSHSVYYGDWLAWYQQKPGKAPKLLIYRASNLASGVPSRFSGSGSGTEFTLTISSLQPDDFATYYCLGGYDDDGETAFGQGTKLEIK

SEQ ID NO: 440 - protein, 110 aa, Artificial Sequence
  Description of Artificial Sequence: Synthetic polypeptide
  cl_DOCBABABA_1_110; 16 6 LC humanized 230
VVLTQTPSPVSASVGDRVTITCQSSHSVYYGDWLAWYQQKPGKAPKVLIYRASNLASGVPSRFSGSGSGTDFTLTISTLQPEDFATYYCLGGYDDDGETAFGQGTKLEIK

SEQ ID NO: 441 - protein, 110 aa, Artificial Sequence; identical to SEQ ID NO: 314
  Description of Artificial Sequence: Synthetic polypeptide
  cl_GOCBABABA_1_110; 16 6 LC humanized 1894

SEQ ID NO: 442 - protein, 110 aa, Artificial Sequence; identical to SEQ ID NO: 315
  Description of Artificial Sequence: Synthetic polypeptide
  cl_LOCBABABA_1_110; 16 6 LC humanized 657

SEQ ID NO: 443 - protein, 110 aa, Artificial Sequence
  Description of Artificial Sequence: Synthetic polypeptide
  cl_MOCBABABA_2_110; 16 6 LC humanized 1917; 16 6 LC humanized 677
VVLTQSPSFLSASVGDRVTITCQSSHSVYYGDWLAWYQQKPGKAPKLLIYRASNLASGVPSRFSGSGSGTEFTLTISSLQPEDFATYYCLGGYDDDGETAFGQGTRLEIK

SEQ ID NO: 444 - protein, 110 aa, Artificial Sequence
  Description of Artificial Sequence: Synthetic polypeptide
  cl_POCBABABA_1_110; 16 6 LC humanized 2038
VVLTQTPSPVSTAVGGRVTITCQSSHSVYYGDWLAWYQQKPGKAPKLLIYRASNLASGVPSRFSGSGSGTEFTLTISSLQDKPFATYYCLGGYDDDGETAFGGGTEVVVK

SEQ ID NO: 445 - protein, 110 aa, Artificial Sequence
  Description of Artificial Sequence: Synthetic polypeptide
  cl_ROCBABABA_1_110; 16 6 LC humanized 21
IQMTQSPSSLSASVGDRVTITCQSSHSVYYGDWLAWYQQKPGKAPKVLIYRASNLASGVPSRFSGSGSGTDFTLTISSLQPEDFATYYCLGGYDDDGETAFGPGTKVEVK

SEQ ID NO: 446 - protein, 110 aa, Artificial Sequence
  Description of Artificial Sequence: Synthetic polypeptide
  cl_SOCBABABA_1_110; 16 6 LC humanized 469
IVLTQSPSLLSASIGDRVTIPCQSSHSVYYGDWLAWYQQKPGKAPKLLIYRASNLASGVPSRFSGSGSGTEFTLTISSLQPEDFATYYCLGGYDDDGETAFGGGTKVDIK

SEQ ID NO: 447 - protein, 110 aa, Artificial Sequence
  Description of Artificial Sequence: Synthetic polypeptide
  cl_TOCBABABA_1_110; 16 6 LC humanized 2008
VVLTQTPSPVSTAVGGRVTITCQSSHSVYYGDWLAWYQQKPGKAPKLLIYRASNLASGVPSRFSGSGSGTDFTLTIGSLQPEDFAAYFCLGGYDDDGETAFGGGTKVEIK

SEQ ID NO: 448 - protein, 110 aa, Artificial Sequence
  Description of Artificial Sequence: Synthetic polypeptide
  cl_WOCBABABA_1_110; 16 6 LC humanized 168
IVMTQSPSTLSASVGDRVTITCQSSHSVYYGDWLAWYQQKPGKAPKLLIYRASNLASGVPSRFSGSGSGTEFTLTISGLQPEDFATYYCLGGYDDDGETAFGGGTKLEIK

SEQ ID NO: 449 - protein, 110 aa, Artificial Sequence
  Description of Artificial Sequence: Synthetic polypeptide
  cl_XOCBABABA_1_110; 16 6 LC humanized 149
IVLTQSPSSLSASVGDRVTITCQSSHSVYYGDWLAWYQQKPGKAPKRLIYRASNLASGVPSRFSGSGSGTEFTLTISGLQPEDIATYYCLGGYDDDGETAFGQGTKVEIK

SEQ ID NO: 450 - protein, 110 aa, Artificial Sequence; identical to SEQ ID NO: 316
  Description of Artificial Sequence: Synthetic polypeptide
  cl_YOCBABABA_1_110; 16 6 LC humanized 113

SEQ ID NO: 451 - protein, 110 aa, Artificial Sequence; identical to SEQ ID NO: 299
  Description of Artificial Sequence: Synthetic polypeptide
  cl_ZOCBABABA_4_110; 16 6 LC humanized 978; 16 6 LC humanized 965; 16 6 LC humanized 924; 16 6 LC humanized 879

SEQ ID NO: 452 - protein, 110 aa, Artificial Sequence
  Description of Artificial Sequence: Synthetic polypeptide
  cl_GUCBABABA_1_110; 16 6 LC humanized 818
VVLTQTPSSVSASVGDRVTITCQSSHSVYYGDWLAWYQQKPGKAPKLLIYRASNLASGVPSRFSGSGSGTDFTLTISSLQPEDFATYYCLGGYDDDGETAFGQGTKVEIK

SEQ ID NO: 453 - protein, 110 aa, Artificial Sequence
  Description of Artificial Sequence: Synthetic polypeptide
  cl_HUCBABABA_1_110; 16 6 LC humanized 12
VVMTQSPSTVSASVGDRVTLTCQSSHSVYYGDWLAWYQQKPGQPPKLLIYRASNLASGVPDRFSGSGSGTDFTLTISSLQADDFATYYCLGGYDDDGETAFGQGTKVEIK

SEQ ID NO: 454 - protein, 110 aa, Artificial Sequence
  Description of Artificial Sequence: Synthetic polypeptide
  cl_LUCBABABA_1_110; 16 6 LC humanized 273
LVMTQSPSSLSASVGDRVTITCQSSHSVYYGDWLAWYQQKPGEAPKLLIYRASNLASGVPSRFSGSGSGTDFTLTISGLQSEDFATYYCLGGYDDDGETAFGQGTKVEIK

SEQ ID NO: 455 - protein, 110 aa, Artificial Sequence
  Description of Artificial Sequence: Synthetic polypeptide
  cl_MUCBABABA_1_110; 16 6 LC humanized 2032
VVLTQTPSPVSTAVGGTGPINCQSSHSVYYGDWLAWYQQKPGQPPKLLIYRASNLASGVPDRFSGSGSGTDFTLTISSLQAEDVAVYYCLGGYDDDGETAFGGGTKLEIK

SEQ ID NO: 456 - protein, 110 aa, Artificial Sequence
  Description of Artificial Sequence: Synthetic polypeptide
  cl_PUCBABABA_1_110; 16 6 LC humanized 267
VVLTQSPSTLAASVGDRVTITCQSSHSVYYGDWLAWYQQKPGKAPKLLIYRASNLASGVPSRFSGSGSGTEFTLTISSLQPDDFATYYCLGGYDDDGETAFGQGTKVEVK

SEQ ID NO: 457 - protein, 110 aa, Artificial Sequence
  Description of Artificial Sequence: Synthetic polypeptide
  cl_QUCBABABA_1_110; 16 6 LC humanized 1992
VVLTQTPSPVSTAVGDRVTITCQSSHSVYYGDWLAWYQQKPGKAPKLLIYRASNLASGVPSRFSGSGSGTDFTLTISSLQPEDFATYYCLGGYDDDGETAFGGGTEVVVK

SEQ ID NO: 458 - protein, 110 aa, Artificial Sequence; identical to SEQ ID NO: 318
  Description of Artificial Sequence: Synthetic polypeptide
  cl_RUCBABABA_1_110; 16 6 LC humanized 1995
  MOD_RES (45)..(45): Any amino acid

SEQ ID NO: 459 - protein, 110 aa, Artificial Sequence
  Description of Artificial Sequence: Synthetic polypeptide
  cl_TUCBABABA_2_110; 16 6 LC humanized 1934; 16 6 LC humanized 1977
VVLTQTPSPVSTAVGGTVTITCQSSHSVYYGDWLAWYQQKPGKAPKLLIYRASNLASGVPSRFSGSGSGTDFTFTISSLQPEDIATYYCLGGYDDDGETAFGGGTEVVVK

SEQ ID NO: 460 - protein, 110 aa, Artificial Sequence
  Description of Artificial Sequence: Synthetic polypeptide
  cl_VUCBABABA_1_110; 16 6 LC humanized 200
VVLTQTPSPVSTAVGERATINCQSSHSVYYGDWLAWYQQKPGQPPKLLIYRASNLASGVPDRFSGTGSGTDFTLTISSLQAEDVAVYYCLGGYDDDGETAFGGGTKVVVK

SEQ ID NO: 461 - protein, 110 aa, Artificial Sequence
  Description of Artificial Sequence: Synthetic polypeptide
  cl_XUCBABABA_1_110; 16 6 LC humanized 2027
  MOD_RES (89)..(89): Any amino acid
VVLTQTPSPVSTAVGGTVTITCQSSHSVYYGDWLAWYQQKPGKAPKRLIYRASNLASGVPSRFSGSGSGTEFTLTISSLQPEDFATYYXLGGYDDDGETAFGGGTEVVVK

SEQ ID NO: 462 - protein, 110 aa, Artificial Sequence
  Description of Artificial Sequence: Synthetic polypeptide
  cl_YUCBABABA_2_110; 16 6 LC humanized 1958; 16 6 LC humanized 1949
VVLTQTPSPVSTAVGGTVTIPCQSSHSVYYGDWLAWYQQKPGKAPKLLIYRASNLASGVPSRFSGSGSGTEFTLTISSLQPDDFATYYCLGGYDDDGETAFGGGTEVVVK

SEQ ID NO: 463 - protein, 110 aa, Artificial Sequence
  Description of Artificial Sequence: Synthetic polypeptide
  cl_BADBABABA_1_110; 16 6 LC humanized 1905
VVLTQTPSPVSTAVGGTVTINCQSSHSVYYGDWLAWYQQKPGQPPKLLIYRASNLASGVPDRFSGSGSGTDFTLTISSLQAEDVAVYYCLGGYDDDGETAFGGGTEVVVK

SEQ ID NO: 464 - protein, 115 aa, Artificial Sequence
  Description of Artificial Sequence: Synthetic polypeptide
  cl_CABBABABA_43_115; 16 6 HC humanized 775; 16 6 HC humanized 722; 16 6 HC humanized 563; 16 6 HC humanized 139; 16 6 HC humanized 988
VQLVESGGGLVQPGGSLRLSCAASGSDISSYHMGWVRQAPGKGLEWVSIIVSSGSAYYATWAKGRFTISRDNSTLYLQMNSLRAEDTAVYYCARNQYSGYGFSFWGPGTLVTVSS

SEQ ID NO: 465 - protein, 115 aa, Artificial Sequence
  Description of Artificial Sequence: Synthetic polypeptide
  cl_DABBABABA_39_115; 16 6 HC humanized 724; 16 6 HC humanized 565; 16 6 HC humanized 141; 16 6 HC humanized 990; 16 6 HC humanized 985
VQLVESGGGLVQPGGSLRLSCAASGSDISSYHMGWVRQAPGKGLEWVGIIVSSGSAYYATWAKGRFTISRSKNTLYLQMNSLKTEDTAVYYCTRNQYSGYGFSFWGPGTLVTVSS

SEQ ID NO: 466 - protein, 115 aa, Artificial Sequence
  Description of Artificial Sequence: Synthetic polypeptide
  cl_REBBABABA_18_115; 16 6 HC humanized 365; 16 6 HC humanized 364; 16 6 HC humanized 363; 16 6 HC humanized 360; 16 6 HC humanized 359
VQLQESGPGLVKPSETLSLTCTVSGSDISSYHMGWIRQPPGKGLEWIGIIVSSGSAYYATWAKSRVTISTSKNQFSLKLSSVTAADTAVYYCARNQYSGYGFSFWGPGTLVTVSS

SEQ ID NO: 467 - protein, 110 aa, Artificial Sequence
  Description of Artificial Sequence: Synthetic polypeptide
  cl_CACBABABA_100_110; 16 6 LC humanized 775; 16 6 LC humanized 724; 16 6 LC humanized 722; 16 6 LC humanized 565; 16 6 LC humanized 563
VVLTQSPSSLSASVGDRVTITCQSSHSVYYGDWLAWYQQKPGKAPKLLIYRASNLASGVPSRFSGSGSGTDFTLTISSLQPEDFATYYCLGGYDDDGETAFGGGTEVVVK

SEQ ID NO: 468 - protein, 115 aa, Artificial Sequence
  Description of Artificial Sequence: Synthetic polypeptide
  cl_CABBABABA_13_115; 16 6 HC humanized 775; 16 6 HC humanized 722; 16 6 HC humanized 563; 16 6 HC humanized 139; 16 6 HC humanized 987
VQLVESGGGLVQPGGSLRLSCAASGSDISSYHMGWVRQAPGKGLEYVSIIVSSGSAYYATWAKGRFTISRDNSTLYLQMGSLRAEDMAVYYCARNQYSGYGFSFWGPGTLVTVSS

SEQ ID NO: 469 - protein, 115 aa, Artificial Sequence
  Description of Artificial Sequence: Synthetic polypeptide
  cl_DABBABABA_12_115; 16 6 HC humanized 724; 16 6 HC humanized 565; 16 6 HC humanized 141; 16 6 HC humanized 989; 16 6 HC humanized 936
VQLVESGGGLVQPGGSLRLSCAASGSDISSYHMGWVRQAPGKGLEWVGIIVSSGSAYYATWAKGRFTISRSKNSLYLQMNSLKTEDTAVYYCARNQYSGYGFSFWGPGTLVTVSS

SEQ ID NO: 470 - protein, 115 aa, Artificial Sequence
  Description of Artificial Sequence: Synthetic polypeptide
  cl_MABBABABA_9_115; 16 6 HC humanized 990; 16 6 HC humanized 937; 16 6 HC humanized 672; 16 6 HC humanized 407; 16 6 HC humanized 248
VQLVESGGGLVQPGGSLKLSCAASGSDISSYHMGWVRQASGKGLEWVGIIVSSGSAYYATWAKGRFTISRSKNTAYLQMNSLKTEDTAVYYCTRNQYSGYGFSFWGPGTLVTVSS

SEQ ID NO: 471 - protein, 115 aa, Artificial Sequence; identical to SEQ ID NO: 464
  Description of Artificial Sequence: Synthetic polypeptide
  cl_NABBABABA_27_115; 16 6 HC humanized 988; 16 6 HC humanized 935; 16 6 HC humanized 670; 16 6 HC humanized 405; 16 6 HC humanized 246

SEQ ID NO: 472 - protein, 115 aa, Artificial Sequence
  Description of Artificial Sequence: Synthetic polypeptide
  cl_PABBABABA_9_115; 16 6 HC humanized 985; 16 6 HC humanized 932; 16 6 HC humanized 667; 16 6 HC humanized 402; 16 6 HC humanized 243
VQLVESGGGLVQPGRSLRLSCTASGSDISSYHMGWFRQAPGKGLEWVGIIVSSGSAYYATWAKGRFTISRSKSIAYLQMNSLKTEDTAVYYCTRNQYSGYGFSFWGPGTLVTVSS

SEQ ID NO: 473 - protein, 115 aa, Artificial Sequence
  Description of Artificial Sequence: Synthetic polypeptide
  cl_QABBABABA_9_115; 16 6 HC humanized 973; 16 6 HC humanized 920; 16 6 HC humanized 655; 16 6 HC humanized 390; 16 6 HC humanized 231
VQLVESGGGLVKPGGSLRLSCAASGSDISSYHMGWVRQAPGKGLEWVGIIVSSGSAYYATWAKGRFTISRSKNTLYLQMNSLKTEDTAVYYCTTNQYSGYGFSFWGPGTLVTVSS

SEQ ID NO: 474 - protein, 115 aa, Artificial Sequence; identical to SEQ ID NO: 466
  Description of Artificial Sequence: Synthetic polypeptide
  cl_REBBABABA_12_115; 16 6 HC humanized 365; 16 6 HC humanized 364; 16 6 HC humanized 363; 16 6 HC humanized 360; 16 6 HC humanized 312

SEQ ID NO: 475 - protein, 115 aa, Artificial Sequence
  Description of Artificial Sequence: Synthetic polypeptide
  cl_WEBBABABA_3_115; 16 6 HC humanized 359; 16 6 HC humanized 306; 16 6 HC humanized 41
LQLQESGSGLVKPSQTLSLTCAVSGSDISSYHMGWIRQPPGKGLEWIGIIVSSGSAYYATWAKSRVTISRSKNQFSLKLSSVTAADTAVYYCARNQYSGYGFSFWGPGTLVTVSS

SEQ ID NO: 476 - protein, 115 aa, Artificial Sequence
  Description of Artificial Sequence: Synthetic polypeptide
  cl_XEBBABABA_3_115; 16 6 HC humanized 357; 16 6 HC humanized 304; 16 6 HC humanized 39
VQLQESGPGLVKPPGTLSLTCAVSGSDISSYHMGWVRQPPGKGLEWIGIIVSSGSAYYATWAKSRVTISKSKNQFSLKLSSVTAADTAVYCCARNQYSGYGFSFWGPGTLVTVSS

SEQ ID NO: 477 - protein, 115 aa, Artificial Sequence
  Description of Artificial Sequence: Synthetic polypeptide
  cl_CIBBABABA_3_115; 16 6 HC humanized 343; 16 6 HC humanized 290; 16 6 HC humanized 25
VQLVESGGGVVQPGRSLRLSCAASGSDISSYHMGWVRQAPGKGLEWVAIIVSSGSAYYATWAKGRFTISRDNSTLYLQMNSLRAEDTAVYYCARNQYSGYGFSFWGPGTLVTVSS

SEQ ID NO: 478 - protein, 110 aa, Artificial Sequence
  Description of Artificial Sequence: Synthetic polypeptide
  cl_CACBABABA_3_110; 16 6 LC humanized 775; 16 6 LC humanized 724;  16 6 LC humanized 722
VVLTQSPSSLSASVGDRVTITCQSSHSVYYGDWLAWYQQKPGKAPKLLIYRASNLASGVPSRFSGSGSGTDFTFTISSLQPEDIATYYCLGGYDDDGETAFGGGTEVVVK

SEQ ID NO: 479 - protein, 110 aa, Artificial Sequence
  Description of Artificial Sequence: Synthetic polypeptide
  cl_GACBABABA_2_110; 16 6 LC humanized 565; 16 6 LC humanized 563
VVLTQSPSSLSASVGDRVTITCQSSHSVYYGDWLAWYQQKPGKAPKRLIYRASNLASGVPSRFSGSGSGTEFTLTISSLQPEDFATYYCLGGYDDDGETAFGGGTEVVVK

SEQ ID NO: 480 - protein, 110 aa, Artificial Sequence
  Description of Artificial Sequence: Synthetic polypeptide
  cl_KACBABABA_2_110; 16 6 LC humanized 141; 16 6 LC humanized 139
VVLTQSPSSFSASTGDRVTITCQSSHSVYYGDWLAWYQQKPGKAPKLLIYRASNLASGVPSRFSGSGSGTDFTLTISCLQSEDFATYYCLGGYDDDGETAFGGGTEVVVK

SEQ ID NO: 481 - protein, 110 aa, Artificial Sequence
  Description of Artificial Sequence: Synthetic polypeptide
  cl_MACBABABA_62_110; 16 6 LC humanized 990; 16 6 LC humanized 988; 16 6 LC humanized 985; 16 6 LC humanized 973; 16 6 LC humanized 937
VVLTQSPSSVSASVGDRVTITCQSSHSVYYGDWLAWYQQKPGKAPKLLIYRASNLASGVPSRFSGSGSGTDFTLTISSLQPEDFATYYCLGGYDDDGETAFGGGTEVVVK

SEQ ID NO: 482 - protein, 110 aa, Artificial Sequence
  Description of Artificial Sequence: Synthetic polypeptide
  cl_WACBABABA_6_110; 16 6 LC humanized 672; 16 6 LC humanized 670;  16 6 LC humanized 667; 16 6 LC humanized 655; 16 6 LC humanized 671
VVLTQSPSSLSASVGDRVTITCQSSHSVYYGDWLAWYQQKPGKVPKLLIYRASNLASGVPSRFSGSGSGTDFTLTISSLQPEDVATYYCLGGYDDDGETAFGGGTEVVVK

SEQ ID NO: 483 - protein, 110 aa, Artificial Sequence
  Description of Artificial Sequence: Synthetic polypeptide
  cl_GECBABABA_6_110; 16 6 LC humanized 248; 16 6 LC humanized 246;  16 6 LC humanized 243; 16 6 LC humanized 231; 16 6 LC humanized 247
VVLTQSPSFLSASVGDRVTITCQSSHSVYYGDWLAWYQQKPGKAPKLLIYRASNLASGVPSRFSGSGSGTEFTLTISSLQPEDFATYYCLGGYDDDGETAFGGGTEVVVK

SEQ ID NO: 484 - protein, 110 aa, Artificial Sequence
  Description of Artificial Sequence: Synthetic polypeptide
  cl_YICBABABA_19_110; 16 6 LC humanized 47; 16 6 LC humanized 46; 16 6 LC humanized 45; 16 6 LC humanized 42; 16 6 LC humanized 41
VVLTQSPSTLSASVGDRVTITCQSSHSVYYGDWLAWYQQKPGKAPKLLIYRASNLASGVPSRFSGSGSGTEFTLTISSLQPDDFATYYCLGGYDDDGETAFGGGTEVVVK

SEQ ID NO: 485 - protein, 16 aa, Artificial Sequence
  Description of Artificial Sequence: Synthetic peptide
  Clone 8 and Clone 16 epitope
GSTSGSGKPGSGEGST

SEQ ID NO: 486 - protein, 14 aa, Artificial Sequence
  Description of Artificial Sequence: Synthetic peptide
  Clone 8 and Clone 16 epitope
GSTSGSGKPGSGEG

SEQ ID NO: 487 - protein, 12 aa, Artificial Sequence
  Description of Artificial Sequence: Synthetic peptide
  Clone 8 and Clone 16 epitope
GSTSGSGKPGSG

SEQ ID NO: 488 - protein, 10 aa, Artificial Sequence
  Description of Artificial Sequence: Synthetic peptide
  Clone 8 and Clone 16 epitope
GSTSGSGKPG

SEQ ID NO: 489 - protein, 14 aa, Artificial Sequence
  Description of Artificial Sequence: Synthetic peptide
  Clone 8 and Clone 16 epitope
GSGKPGSGEGSTKG

SEQ ID NO: 490 - protein, 12 aa, Artificial Sequence
  Description of Artificial Sequence: Synthetic peptide
  Clone 8 and Clone 16 epitope
GKPGSGEGSTKG

SEQ ID NO: 491 - protein, 10 aa, Artificial Sequence
  Description of Artificial Sequence: Synthetic peptide
  Clone 8 and Clone 16 epitope
PGSGEGSTKG

SEQ ID NO: 492 - protein, 5 aa, Artificial Sequence
  Description of Artificial Sequence: Synthetic peptide
  Clone 8 HC CDR1 (Kabat)
NLAII

SEQ ID NO: 493 - protein, 5 aa, Artificial Sequence
  Description of Artificial Sequence: Synthetic peptide
  Clone 16 HC CDR1 (Kabat)
SYHMG

SEQ ID NO: 494 - protein, 10 aa, Artificial Sequence
  Description of Artificial Sequence: Synthetic peptide
  Clone 8 HC CDR1 (IMGT)
GFTISNLAII

SEQ ID NO: 495 - protein, 10 aa, Artificial Sequence
  Description of Artificial Sequence: Synthetic peptide
  Clone 16 HC CDR1 (IMGT)
GSDISSYHMG

SEQ ID NO: 496 - protein, 13 aa, Artificial Sequence
  Description of Artificial Sequence: Synthetic peptide
  Clone 8 and Clone 16 epitope
GSTSGSGKPGSGE

SEQ ID NO: 497 - protein, 13 aa, Artificial Sequence
  Description of Artificial Sequence: Synthetic peptide
  Clone 8 and Clone 16 epitope
SGKPGSGEGSTKG

SEQ ID NO: 498 - protein, 11 aa, Artificial Sequence
  Description of Artificial Sequence: Synthetic peptide
  Clone 8 and Clone 16 epitope
KPGSGEGSTKG

SEQ ID NO: 499 - protein, 8 aa, Artificial Sequence
  Description of Artificial Sequence: Synthetic peptide
  Clone 8 epitope
SGKPGSGE

SEQ ID NO: 500 - protein, 5 aa, Artificial Sequence
  Description of Artificial Sequence: Synthetic peptide
  Clone 16 epitope
KPGSG